European Patent Specification EP 3 497 214 B1, published June 28, 2023. Title: PROGRAMMABLE CAS9-RECOMBINASE FUSION PROTEINS AND USES THEREOF. Applicant: President and Fellows of Harvard College. Application Not Yet Assigned. The sequence listing filed with the application follows.

SEQUENCE LISTING (775 sequences)

SEQ ID NO: 1 - protein, 1368 aa, Artificial Sequence
  Synthetic Polypeptide
MDKKYSIGLAIGTNSVGWAVITDEYKVPSKKFKVLGNTDRHSIKKNLIGALLFDSGETAEATRLKRTARRRYTRRKNRICYLQEIFSNEMAKVDDSFFHRLEESFLVEEDKKHERHPIFGNIVDEVAYHEKYPTIYHLRKKLVDSTDKADLRLIYLALAHMIKFRGHFLIEGDLNPDNSDVDKLFIQLVQTYNQLFEENPINASGVDAKAILSARLSKSRRLENLIAQLPGEKKNGLFGNLIALSLGLTPNFKSNFDLAEDAKLQLSKDTYDDDLDNLLAQIGDQYADLFLAAKNLSDAILLSDILRVNTEITKAPLSASMIKRYDEHHQDLTLLKALVRQQLPEKYKEIFFDQSKNGYAGYIDGGASQEEFYKFIKPILEKMDGTEELLVKLNREDLLRKQRTFDNGSIPHQIHLGELHAILRRQEDFYPFLKDNREKIEKILTFRIPYYVGPLARGNSRFAWMTRKSEETITPWNFEEVVDKGASAQSFIERMTNFDKNLPNEKVLPKHSLLYEYFTVYNELTKVKYVTEGMRKPAFLSGEQKKAIVDLLFKTNRKVTVKQLKEDYFKKIECFDSVEISGVEDRFNASLGTYHDLLKIIKDKDFLDNEENEDILEDIVLTLTLFEDREMIEERLKTYAHLFDDKVMKQLKRRRYTGWGRLSRKLINGIRDKQSGKTILDFLKSDGFANRNFMQLIHDDSLTFKEDIQKAQVSGQGDSLHEHIANLAGSPAIKKGILQTVKVVDELVKVMGRHKPENIVIEMARENQTTQKGQKNSRERMKRIEEGIKELGSQILKEHPVENTQLQNEKLYLYYLQNGRDMYVDQELDINRLSDYDVDAIVPQSFLKDDSIDNKVLTRSDKNRGKSDNVPSEEVVKKMKNYWRQLLNAKLITQRKFDNLTKAERGGLSELDKAGFIKRQLVETRQITKHVAQILDSRMNTKYDENDKLIREVKVITLKSKLVSDFRKDFQFYKVREINNYHHAHDAYLNAVVGTALIKKYPKLESEFVYGDYKVYDVRKMIAKSEQEIGKATAKYFFYSNIMNFFKTEITLANGEIRKRPLIETNGETGEIVWDKGRDFATVRKVLSMPQVNIVKKTEVQTGGFSKESILPKRNSDKLIARKKDWDPKKYGGFDSPTVAYSVLVVAKVEKGKSKKLKSVKELLGITIMERSSFEKNPIDFLEAKGYKEVKKDLIIKLPKYSLFELENGRKRMLASAGELQKGNELALPSKYVNFLYLASHYEKLKGSPEDNEQKQLFVEQHKHYLDEIIEQISEFSKRVILADANLDKVLSAYNKHRDKPIREQAENIIHLFTLTNLGAPAAFKYFDTTIDRKRYTSTKEVLDATLIHQSITGLYETRIDLSQLGGD

SEQ ID NO: 2 - DNA, 4104 bp, Streptococcus pyogenes
atggataagaaatactcaataggcttagatatcggcacaaatagcgtcggatgggcggtgatcactgatgattataaggttccgtctaaaaagttcaaggttctgggaaatacagaccgccacagtatcaaaaaaaatcttataggggctcttttatttggcagtggagagacagcggaagcgactcgtctcaaacggacagctcgtagaaggtatacacgtcggaagaatcgtatttgttatctacaggagattttttcaaatgagatggcgaaagtagatgatagtttctttcatcgacttgaagagtcttttttggtggaagaagacaagaagcatgaacgtcatcctatttttggaaatatagtagatgaagttgcttatcatgagaaatatccaactatctatcatctgcgaaaaaaattggcagattctactgataaagcggatttgcgcttaatctatttggccttagcgcatatgattaagtttcgtggtcattttttgattgagggagatttaaatcctgataatagtgatgtggacaaactatttatccagttggtacaaatctacaatcaattatttgaagaaaaccctattaacgcaagtagagtagatgctaaagcgattctttctgcacgattgagtaaatcaagacgattagaaaatctcattgctcagctccccggtgagaagagaaatggcttgtttgggaatctcattgctttgtcattgggattgacccctaattttaaatcaaattttgatttggcagaagatgctaaattacagctttcaaaagatacttacgatgatgatttagataatttattggcgcaaattggagatcaatatgctgatttgtttttggcagctaagaatttatcagatgctattttactttcagatatcctaagagtaaatagtgaaataactaaggctcccctatcagcttcaatgattaagcgctacgatgaacatcatcaagacttgactcttttaaaagctttagttcgacaacaacttccagaaaagtataaagaaatcttttttgatcaatcaaaaaacggatatgcaggttatattgatgggggagctagccaagaagaattttataaatttatcaaaccaattttagaaaaaatggatggtactgaggaattattggtgaaactaaatcgtgaagatttgctgcgcaagcaacggacctttgacaacggctctattccccatcaaattcacttgggtgagctgcatgctattttgagaagacaagaagacttttatccatttttaaaagacaatcgtgagaagattgaaaaaatcttgacttttcgaattccttattatgttggtccattggcgcgtggcaatagtcgttttgcatggatgactcggaagtctgaagaaacaattaccccatggaattttgaagaagttgtcgataaaggtgcttcagctcaatcatttattgaacgcatgacaaactttgataaaaatcttccaaatgaaaaagtactaccaaaacatagtttgctttatgagtattttacggtttataacgaattgacaaaggtcaaatatgttactgagggaatgcgaaaaccagcatttctttcaggtgaacagaagaaagccattgttgatttactcttcaaaacaaatcgaaaagtaaccgttaagcaattaaaagaagattatttcaaaaaaatagaatgttttgatagtgttgaaatttcaggagttgaagatagatttaatgcttcattaggcgcctaccatgatttgctaaaaattattaaagataaagattttttggataatgaagaaaatgaagatatcttagaggatattgttttaacattgaccttatttgaagatagggggatgattgaggaaagacttaaaacatatgctcacctctttgatgataaggtgatgaaacagcttaaacgtcgccgttatactggttggggacgtttgtctcgaaaattgattaatggtattagggataagcaatctggcaaaacaatattagattttttgaaatcagatggttttgccaatcgcaattttatgcagctgatccatgatgatagtttgacatttaaagaagatattcaaaaagcacaggtgtctggacaaggccatagtttacatgaacagattgctaacttagctggcagtcctgctattaaaaaaggtattttacagactgtaaaaattgttgatgaactggtcaaagtaatggggcataagccagaaaatatcgttattgaaatggcacgtgaaaatcagacaactcaaaagggccagaaaaattcgcgagagcgtatgaaacgaatcgaagaaggtatcaaagaattaggaagtcagattcttaaagagcatcctgttgaaaatactcaattgcaaaatgaaaagctctatctctattatctacaaaatggaagagacatgtatgtggaccaagaattagatattaatcgtttaagtgattatgatgtcgatcacattgttccacaaagtttcattaaagacgattcaatagacaataaggtactaacgcgttctgataaaaatcgtggtaaatcggataacgttccaagtgaagaagtagtcaaaaagatgaaaaactattggagacaacttctaaacgccaagttaatcactcaacgtaagtttgataatttaacgaaagctgaacgtggaggtttgagtgaacttgataaagctggttttatcaaacgccaattggttgaaactcgccaaatcactaagcatgtggcacaaattttggatagtcgcatgaatactaaatacgatgaaaatgataaacttattcgagaggttaaagtgattaccttaaaatctaaattagtttctgacttccgaaaagatttccaattctataaagtacgtgagattaacaattaccatcatgcccatgatgcgtatctaaatgccgtcgttggaactgctttgattaagaaatatccaaaacttgaatcggagtttgtctatggtgattataaagtttatgatgttcgtaaaatgattgctaagtctgagcaagaaataggcaaagcaaccgcaaaatatttcttttactctaatatcatgaacttcttcaaaacagaaattacacttgcaaatggagagattcgcaaacgccctctaatcgaaactaatggggaaactggagaaattgtctgggataaagggcgagattttgccacagtgcgcaaagtattgtccatgccccaagtcaatattgtcaagaaaacagaagtacagacaggcggattctccaaggagtcaattttaccaaaaagaaattcggacaagcttattgctcgtaaaaaagactgggatccaaaaaaatatggtggttttgatagtccaacggtagcttattcagtcctagtggttgctaaggtggaaaaagggaaatcgaagaagttaaaatccgttaaagagttactagggatcacaattatggaaagaagttcctttgaaaaaaatccgattgactttttagaagctaaaggatataaggaagttaaaaaagacttaatcattaaactacctaaatatagtctttttgagttagaaaacggtcgtaaacggatgctggctagtgccggagaattacaaaaaggaaatgagctggctctgccaagcaaatatgtgaattttttatatttagctagtcattatgaaaagttgaagggtagtccagaagataacgaacaaaaacaattgtttgtggagcagcataagcattatttagatgagattattgagcaaatcagtgaattttctaagcgtgttattttagcagatgccaatttagataaagttcttagtgcatataacaaacatagagacaaaccaatacgtgaacaagcagaaaatattattcatttatttacgttgacgaatcttggagctcccgctgcttttaaatattttgatacaacaattgatcgtaaacgatatacgtctacaaaagaagttttagatgccactcttatccatcaatccatcactggtctttatgaaacacgcattgatttgagtcagctaggaggtgactga

SEQ ID NO: 3 - protein, 1367 aa, Streptococcus pyogenes
MDKKYSIGLDIGTNSVGWAVITDDYKVPSKKFKVLGNTDRHSIKKNLIGALLFGSGETAEATRLKRTARRRYTRRKNRICYLQEIFSNEMAKVDDSFFHRLEESFLVEEDKKHERHPIFGNIVDEVAYHEKYPTIYHLRKKLADSTDKADLRLIYLALAHMIKFRGHFLIEGDLNPDNSDVDKLFIQLVQIYNQLFEENPINASRVDAKAILSARLSKSRRLENLIAQLPGEKRNGLFGNLIALSLGLTPNFKSNFDLAEDAKLQLSKDTYDDDLDNLLAQIGDQYADLFLAAKNLSDAILLSDILRVNSEITKAPLSASMIKRYDEHHQDLTLLKALVRQQLPEKYKEIFFDQSKNGYAGYIDGGASQEEFYKFIKPILEKMDGTEELLVKLNREDLLRKQRTFDNGSIPHQIHLGELHAILRRQEDFYPFLKDNREKIEKILTFRIPYYVGPLARGNSRFAWMTRKSEETITPWNFEEVVDKGASAQSFIERMTNFDKNLPNEKVLPKHSLLYEYFTVYNELTKVKYVTEGMRKPAFLSGEQKKAIVDLLFKTNRKVTVKQLKEDYFKKIECFDSVEISGVEDRFNASLGAYHDLLKIIKDKDFLDNEENEDILEDIVLTLTLFEDRGMIEERLKTYAHLFDDKVMKQLKRRRYTGWGRLSRKLINGIRDKQSGKTILDFLKSDGFANRNFMQLIHDDSLTFKEDIQKAQVSGQGHSLHEQIANLAGSPAIKKGILQTVKIVDELVKVMGHKPENIVIEMARENQTTQKGQKNSRERMKRIEEGIKELGSQILKEHPVENTQLQNEKLYLYYLQNGRDMYVDQELDINRLSDYDVDHIVPQSFIKDDSIDNKVLTRSDKNRGKSDNVPSEEVVKKMKNYWRQLLNAKLITQRKFDNLTKAERGGLSELDKAGFIKRQLVETRQITKHVAQILDSRMNTKYDENDKLIREVKVITLKSKLVSDFRKDFQFYKVREINNYHHAHDAYLNAVVGTALIKKYPKLESEFVYGDYKVYDVRKMIAKSEQEIGKATAKYFFYSNIMNFFKTEITLANGEIRKRPLIETNGETGEIVWDKGRDFATVRKVLSMPQVNIVKKTEVQTGGFSKESILPKRNSDKLIARKKDWDPKKYGGFDSPTVAYSVLVVAKVEKGKSKKLKSVKELLGITIMERSSFEKNPIDFLEAKGYKEVKKDLIIKLPKYSLFELENGRKRMLASAGELQKGNELALPSKYVNFLYLASHYEKLKGSPEDNEQKQLFVEQHKHYLDEIIEQISEFSKRVILADANLDKVLSAYNKHRDKPIREQAENIIHLFTLTNLGAPAAFKYFDTTIDRKRYTSTKEVLDATLIHQSITGLYETRIDLSQLGGD

SEQ ID NO: 4 - DNA, 4212 bp, Artificial Sequence
  Synthetic Polynucleotide
atggataaaaagtattctattggtttagacatcggcactaattccgttggatgggctgtcataaccgatgaatacaaagtaccttcaaagaaatttaaggtgttggggaacacagaccgtcattcgattaaaaagaatcttatcggtgccctcctattcgatagtggcgaaacggcagaggcgactcgcctgaaacgaaccgctcggagaaggtatacacgtcgcaagaaccgaatatgttacttacaagaaatttttagcaatgagatggccaaagttgacgattctttctttcaccgtttggaagagtccttccttgtcgaagaggacaagaaacatgaacggcaccccatctttggaaacatagtagatgaggtggcatatcatgaaaagtacccaacgatttatcacctcagaaaaaagctagttgactcaactgataaagcggacctgaggttaatctacttggctcttgcccatatgataaagttccgtgggcactttctcattgagggtgatctaaatccggacaactcggatgtcgacaaactgttcatccagttagtacaaacctataatcagttgtttgaagagaaccctataaatgcaagtggcgtggatgcgaaggctattcttagcgcccgcctctctaaatcccgacggctagaaaacctgatcgcacaattacccggagagaagaaaaatgggttgttcggtaaccttatagcgctctcactaggcctgacaccaaattttaagtcgaacttcgacttagctgaagatgccaaattgcagcttagtaaggacacgtacgatgacgatctcgacaatctactggcacaaattggagatcagtatgcggacttatttttggctgccaaaaaccttagcgatgcaatcctcctatctgacatactgagagttaatactgagattaccaaggcgccgttatccgcttcaatgatcaaaaggtacgatgaacatcaccaagacttgacacttctcaaggccctagtccgtcagcaactgcctgagaaatataaggaaatattctttgatcagtcgaaaaacgggtacgcaggttatattgacggcggagcgagtcaagaggaattctacaagtttatcaaacccatattagagaagatggatgggacggaagagttgcttgtaaaactcaatcgcgaagatctactgcgaaagcagcggactttcgacaacggtagcattccacatcaaatccacttaggcgaattgcatgctatacttagaaggcaggaggatttttatccgttcctcaaagacaatcgtgaaaagattgagaaaatcctaacctttcgcataccttactatgtgggacccctggcccgagggaactctcggttcgcatggatgacaagaaagtccgaagaaacgattactccatggaattttgaggaagttgtcgataaaggtgcgtcagctcaatcgttcatcgagaggatgaccaactttgacaagaatttaccgaacgaaaaagtattgcctaagcacagtttactttacgagtatttcacagtgtacaatgaactcacgaaagttaagtatgtcactgagggcatgcgtaaacccgcctttctaagcggagaacagaagaaagcaatagtagatctgttattcaagaccaaccgcaaagtgacagttaagcaattgaaagaggactactttaagaaaattgaatgcttcgattctgtcgagatctccggggtagaagatcgatttaatgcgtcacttggtacgtatcatgacctcctaaagataattaaagataaggacttcctggataacgaagagaatgaagatatcttagaagatatagtgttgactcttaccctctttgaagatcgggaaatgattgaggaaagactaaaaacatacgctcacctgttcgacgataaggttatgaaacagttaaagaggcgtcgctatacgggctggggacgattgtcgcggaaacttatcaacgggataagagacaagcaaagtggtaaaactattctcgattttctaaagagcgacggcttcgccaataggaactttatgcagctgatccatgatgactctttaaccttcaaagaggatatacaaaaggcacaggtttccggacaaggggactcattgcacgaacatattgcgaatcttgctggttcgccagccatcaaaaagggcatactccagacagtcaaagtagtggatgagctagttaaggtcatgggacgtcacaaaccggaaaacattgtaatcgagatggcacgcgaaaatcaaacgactcagaaggggcaaaaaaacagtcgagagcggatgaagagaatagaagagggtattaaagaactgggcagccagatcttaaaggagcatcctgtggaaaatacccaattgcagaacgagaaactttacctctattacctacaaaatggaagggacatgtatgttgatcaggaactggacataaaccgtttatctgattacgacgtcgatcacattgtaccccaatcctttttgaaggacgattcaatcgacaataaagtgcttacacgctcggataagaaccgagggaaaagtgacaatgttccaagcgaggaagtcgtaaagaaaatgaagaactattggcggcagctcctaaatgcgaaactgataacgcaaagaaagttcgataacttaactaaagctgagaggggtggcttgtctgaacttgacaaggccggatttattaaacgtcagctcgtggaaacccgccaaatcacaaagcatgttgcacagatactagattcccgaatgaatacgaaatacgacgagaacgataagctgattcgggaagtcaaagtaatcactttaaagtcaaaattggtgtcggacttcagaaaggattttcaattctataaagttagggagataaataactaccaccatgcgcacgacgcttatcttaatgccgtcgtagggaccgcactcattaagaaatacccgaagctagaaagtgagtttgtgtatggtgattacaaagtttatgacgtccgtaagatgatcgcgaaaagcgaacaggagataggcaaggctacagccaaatacttcttttattctaacattatgaatttctttaagacggaaatcactctggcaaacggagagatacgcaaacgacctttaattgaaaccaatggggagacaggtgaaatcgtatgggataagggccgggacttcgcgacggtgagaaaagttttgtccatgccccaagtcaacatagtaaagaaaactgaggtgcagaccggagggttttcaaaggaatcgattcttccaaaaaggaatagtgataagctcatcgctcgtaaaaaggactgggacccgaaaaagtacggtggcttcgatagccctacagttgcctattctgtcctagtagtggcaaaagttgagaagggaaaatccaagaaactgaagtcagtcaaagaattattggggataacgattatggagcgctcgtcttttgaaaagaaccccatcgacttccttgaggcgaaaggttacaaggaagtaaaaaaggatctcataattaaactaccaaagtatagtctgtttgagttagaaaatggccgaaaacggatgttggctagcgccggagagcttcaaaaggggaacgaactcgcactaccgtctaaatacgtgaatttcctgtatttagcgtcccattacgagaagttgaaaggttcacctgaagataacgaacagaagcaactttttgttgagcagcacaaacattatctcgacgaaatcatagagcaaatttcggaattcagtaagagagtcatcctagctgatgccaatctggacaaagtattaagcgcatacaacaagcacagggataaacccatacgtgagcaggcggaaaatattatccatttgtttactcttaccaacctcggcgctccagccgcattcaagtattttgacacaacgatagatcgcaaacgatacacttctaccaaggaggtgctagacgcgacactgattcaccaatccatcacgggattatatgaaactcggatagatttgtcacagcttgggggtgacggatcccccaagaagaagaggaaagtctcgagcgactacaaagaccatgacggtgattataaagatcatgacatcgattacaaggatgacgatgacaaggctgcagga

SEQ ID NO: 5 - protein, 1368 aa, Artificial Sequence
  Synthetic Polypeptide
MDKKYSIGLAIGTNSVGWAVITDEYKVPSKKFKVLGNTDRHSIKKNLIGALLFDSGETAEATRLKRTARRRYTRRKNRICYLQEIFSNEMAKVDDSFFHRLEESFLVEEDKKHERHPIFGNIVDEVAYHEKYPTIYHLRKKLVDSTDKADLRLIYLALAHMIKFRGHFLIEGDLNPDNSDVDKLFIQLVQTYNQLFEENPINASGVDAKAILSARLSKSRRLENLIAQLPGEKKNGLFGNLIALSLGLTPNFKSNFDLAEDAKLQLSKDTYDDDLDNLLAQIGDQYADLFLAAKNLSDAILLSDILRVNTEITKAPLSASMIKRYDEHHQDLTLLKALVRQQLPEKYKEIFFDQSKNGYAGYIDGGASQEEFYKFIKPILEKMDGTEELLVKLNREDLLRKQRTFDNGSIPHQIHLGELHAILRRQEDFYPFLKDNREKIEKILTFRIPYYVGPLARGNSRFAWMTRKSEETITPWNFEEVVDKGASAQSFIERMTNFDKNLPNEKVLPKHSLLYEYFTVYNELTKVKYVTEGMRKPAFLSGEQKKAIVDLLFKTNRKVTVKQLKEDYFKKIECFDSVEISGVEDRFNASLGTYHDLLKIIKDKDFLDNEENEDILEDIVLTLTLFEDREMIEERLKTYAHLFDDKVMKQLKRRRYTGWGRLSRKLINGIRDKQSGKTILDFLKSDGFANRNFMQLIHDDSLTFKEDIQKAQVSGQGDSLHEHIANLAGSPAIKKGILQTVKVVDELVKVMGRHKPENIVIEMARENQTTQKGQKNSRERMKRIEEGIKELGSQILKEHPVENTQLQNEKLYLYYLQNGRDMYVDQELDINRLSDYDVDHIVPQSFLKDDSIDNKVLTRSDKNRGKSDNVPSEEVVKKMKNYWRQLLNAKLITQRKFDNLTKAERGGLSELDKAGFIKRQLVETRQITKHVAQILDSRMNTKYDENDKLIREVKVITLKSKLVSDFRKDFQFYKVREINNYHHAHDAYLNAVVGTALIKKYPKLESEFVYGDYKVYDVRKMIAKSEQEIGKATAKYFFYSNIMNFFKTEITLANGEIRKRPLIETNGETGEIVWDKGRDFATVRKVLSMPQVNIVKKTEVQTGGFSKESILPKRNSDKLIARKKDWDPKKYGGFDSPTVAYSVLVVAKVEKGKSKKLKSVKELLGITIMERSSFEKNPIDFLEAKGYKEVKKDLIIKLPKYSLFELENGRKRMLASAGELQKGNELALPSKYVNFLYLASHYEKLKGSPEDNEQKQLFVEQHKHYLDEIIEQISEFSKRVILADANLDKVLSAYNKHRDKPIREQAENIIHLFTLTNLGAPAAFKYFDTTIDRKRYTSTKEVLDATLIHQSITGLYETRIDLSQLGGD

SEQ ID NO: 6 - protein, 18 aa, Artificial Sequence
  Synthetic Polypeptide
GGSGGSGGSGGSGGSGGS

SEQ ID NO: 7 - protein, 16 aa, Artificial Sequence
  Synthetic Polypeptide
SGSETPGTSESATPES

SEQ ID NO: 8 - protein, 12 aa, Artificial Sequence
  Synthetic Polypeptide
SGSETPGTSESA

SEQ ID NO: 9 - protein, 21 aa, Artificial Sequence
  Synthetic Polypeptide
SGSETPGTSESATPEGGSGGS

SEQ ID NO: 10 - protein, 15 aa, Artificial Sequence
  Synthetic Polypeptide
VPFLLEPDNINGKTC

SEQ ID NO: 11 - protein, 12 aa, Artificial Sequence
  Synthetic Polypeptide
GSAGSAAGSGEF

SEQ ID NO: 12 - protein, 12 aa, Artificial Sequence
  Synthetic Polypeptide
SIVAQLSRPDPA

SEQ ID NO: 13 - protein, 10 aa, Artificial Sequence
  Synthetic Polypeptide
MKIIEQLPSA

SEQ ID NO: 14 - protein, 10 aa, Artificial Sequence
  Synthetic Polypeptide
VRHKLKRVGS

SEQ ID NO: 15 - protein, 12 aa, Artificial Sequence
  Synthetic Polypeptide
GHGTGSTGSGSS

SEQ ID NO: 16 - protein, 7 aa, Artificial Sequence
  Synthetic Polypeptide
MSRPDPA

SEQ ID NO: 17 - protein, 4 aa, Artificial Sequence
  Synthetic Polypeptide
GGSM

SEQ ID NO: 18 - skipped

SEQ ID NO: 19 - RNA, 17 nt, Artificial Sequence
  Synthetic Polynucleotide
  misc_feature (1)..(4): n is a, c, g, or u
  misc_feature (8)..(9): s is g or c
  misc_feature (10)..(11): w is a, t or u
  misc_feature (12)..(13): s is g or c
  misc_feature (14)..(17): n is a, c, g, or u
nnnnaaasswwssnnnn

SEQ ID NO: 20 - DNA, 22 bp, Artificial Sequence
  Synthetic Polynucleotide
ggtgtttcgtcctttccacaag

SEQ ID NO: 21 - DNA, 41 bp, Artificial Sequence
  Synthetic Polynucleotide
gcacactagttagggataacagttttagagctagaaatagc

SEQ ID NO: 22 - DNA, 40 bp, Artificial Sequence
  Synthetic Polynucleotide
gcccatgacccttctcctctgttttagagctagaaatagc

SEQ ID NO: 23 - DNA, 41 bp, Artificial Sequence
  Synthetic Polynucleotide
gctcagggcctgtgatgggaggttttagagctagaaatagc

SEQ ID NO: 24 - DNA, 40 bp, Artificial Sequence
  Synthetic Polynucleotide
ggcccatgacccttctcctcgttttagagctagaaatagc

SEQ ID NO: 25 - DNA, 41 bp, Artificial Sequence
  Synthetic Polynucleotide
gcctcagggcctgtgatgggagttttagagctagaaatagc

SEQ ID NO: 26 - DNA, 40 bp, Artificial Sequence
  Synthetic Polynucleotide
gacttgaaacactctttttcgttttagagctagaaatagc

SEQ ID NO: 27 - DNA, 41 bp, Artificial Sequence
  Synthetic Polynucleotide
gagttgaagacacacaacacagttttagagctagaaatagc

SEQ ID NO: 28 - DNA, 40 bp, Artificial Sequence
  Synthetic Polynucleotide
ggaactcatgtgattaactggttttagagctagaaatagc

SEQ ID NO: 29 - DNA, 41 bp, Artificial Sequence
  Synthetic Polynucleotide
gtctacctctcatgagccggtgttttagagctagaaatagc

SEQ ID NO: 30 - DNA, 41 bp, Artificial Sequence
  Synthetic Polynucleotide
gtttcccgcaggatgtgggatgttttagagctagaaatagc

SEQ ID NO: 31 - DNA, 41 bp, Artificial Sequence
  Synthetic Polynucleotide
gcctggggatttatgttcttagttttagagctagaaatagc

SEQ ID NO: 32 - DNA, 41 bp, Artificial Sequence
  Synthetic Polynucleotide
gaaatagcacaatgaatggaagttttagagctagaaatagc

SEQ ID NO: 33 - DNA, 41 bp, Artificial Sequence
  Synthetic Polynucleotide
gactttttgggggagagggaggttttagagctagaaatagc

SEQ ID NO: 34 - DNA, 40 bp, Artificial Sequence
  Synthetic Polynucleotide
ggagacttaagtccaaaaccgttttagagctagaaatagc

SEQ ID NO: 35 - DNA, 41 bp, Artificial Sequence
  Synthetic Polynucleotide
gtcagctatgatcacttccctgttttagagctagaaatagc

SEQ ID NO: 36 - DNA, 56 bp, Artificial Sequence
  Synthetic Polynucleotide
tcgtctcggcgtccccaattttcccaaacagaggtctgtaaaccgaggtgagacgg

SEQ ID NO: 37 - DNA, 56 bp, Artificial Sequence
  Synthetic Polynucleotide
ccgtctcacctcggtttacagacctctgtttgggaaaattggggacgccgagacga

SEQ ID NO: 38 - DNA, 57 bp, Artificial Sequence
  Synthetic Polynucleotide
tcgtctcggcgtccccaattttcccaaacagaggttctgtaaaccgaggtgagacgg

SEQ ID NO: 39 - DNA, 57 bp, Artificial Sequence
  Synthetic Polynucleotide
ccgtctcacctcggtttacagaacctctgtttgggaaaattggggacgccgagacga

SEQ ID NO: 40 - DNA, 58 bp, Artificial Sequence
  Synthetic Polynucleotide
tcgtctcggcgtccccaattttcccaaacagaggtatctgtaaaccgaggtgagacgg

SEQ ID NO: 41 - DNA, 58 bp, Artificial Sequence
  Synthetic Polynucleotide
ccgtctcacctcggtttacagatacctctgtttgggaaaattggggacgccgagacga

SEQ ID NO: 42 - DNA, 59 bp, Artificial Sequence
  Synthetic Polynucleotide
tcgtctcggcgtccccaattttcccaaacagaggtaatctgtaaaccgaggtgagacgg

SEQ ID NO: 43 - DNA, 59 bp, Artificial Sequence
  Synthetic Polynucleotide
ccgtctcacctcggtttacagattacctctgtttgggaaaattggggacgccgagacga

SEQ ID NO: 44 - DNA, 60 bp, Artificial Sequence
  Synthetic Polynucleotide
tcgtctcggcgtccccaattttcccaaacagaggtaaatctgtaaaccgaggtgagacgg

SEQ ID NO: 45 - DNA, 60 bp, Artificial Sequence
  Synthetic Polynucleotide
ccgtctcacctcggtttacagatttacctctgtttgggaaaattggggacgccgagacga

SEQ ID NO: 46 - DNA, 61 bp, Artificial Sequence
  Synthetic Polynucleotide
tcgtctcggcgtccccaattttcccaaacagaggtgaaatctgtaaaccgaggtgagacgg

SEQ ID NO: 47 - DNA, 61 bp, Artificial Sequence
  Synthetic Polynucleotide
ccgtctcacctcggtttacagatttcacctctgtttgggaaaattggggacgccgagacga

SEQ ID NO: 48 - DNA, 62 bp, Artificial Sequence
  Synthetic Polynucleotide
tcgtctcggcgtccccaattttcccaaacagaggtcgaaatctgtaaaccgaggtgagacgg

SEQ ID NO: 49 - DNA, 62 bp, Artificial Sequence
  Synthetic Polynucleotide
ccgtctcacctcggtttacagatttcgacctctgtttgggaaaattggggacgccgagacga

SEQ ID NO: 50 - DNA, 63 bp, Artificial Sequence
  Synthetic Polynucleotide
tcgtctcggcgtccccaattttcccaaacagaggttcgaaatctgtaaaccgaggtgagacgg

SEQ ID NO: 51 - DNA, 63 bp, Artificial Sequence
  Synthetic Polynucleotide
ccgtctcacctcggtttacagatttcgaacctctgtttgggaaaattggggacgccgagacga

SEQ ID NO: 52 - DNA, 54 bp, Artificial Sequence
  Synthetic Polynucleotide
tcgtctcggaggttttggaacctctgtttgggaaaattggggagtctgagacgg

SEQ ID NO: 53 - DNA, 54 bp, Artificial Sequence
  Synthetic Polynucleotide
ccgtctcagactccccaattttcccaaacagaggttccaaaacctccgagacga

SEQ ID NO: 54 - DNA, 55 bp, Artificial Sequence
  Synthetic Polynucleotide
tcgtctcggaggttttggacacctctgtttgggaaaattggggagtctgagacgg

SEQ ID NO: 55 - DNA, 55 bp, Artificial Sequence
  Synthetic Polynucleotide
ccgtctcagactccccaattttcccaaacagaggtgtccaaaacctccgagacga

SEQ ID NO: 56 - DNA, 56 bp, Artificial Sequence
  Synthetic Polynucleotide
tcgtctcggaggttttggactacctctgtttgggaaaattggggagtctgagacgg

SEQ ID NO: 57 - DNA, 56 bp, Artificial Sequence
  Synthetic Polynucleotide
ccgtctcagactccccaattttcccaaacagaggtagtccaaaacctccgagacga

SEQ ID NO: 58 - DNA, 57 bp, Artificial Sequence
  Synthetic Polynucleotide
tcgtctcggaggttttggacttacctctgtttgggaaaattggggagtctgagacgg

SEQ ID NO: 59 - DNA, 57 bp, Artificial Sequence
  Synthetic Polynucleotide
ccgtctcagactccccaattttcccaaacagaggtaagtccaaaacctccgagacga

SEQ ID NO: 60 - DNA, 58 bp, Artificial Sequence
  Synthetic Polynucleotide
tcgtctcggaggttttggacttaacctctgtttgggaaaattggggagtctgagacgg

SEQ ID NO: 61 - DNA, 58 bp, Artificial Sequence
  Synthetic Polynucleotide
ccgtctcagactccccaattttcccaaacagaggttaagtccaaaacctccgagacga

SEQ ID NO: 62 - DNA, 59 bp, Artificial Sequence
  Synthetic Polynucleotide
tcgtctcggaggttttggacttagacctctgtttgggaaaattggggagtctgagacgg

SEQ ID NO: 63 - DNA, 59 bp, Artificial Sequence
  Synthetic Polynucleotide
ccgtctcagactccccaattttcccaaacagaggtctaagtccaaaacctccgagacga

SEQ ID NO: 64 - DNA, 60 bp, Artificial Sequence
  Synthetic Polynucleotide
tcgtctcggaggttttggacttagcacctctgtttgggaaaattggggagtctgagacgg

SEQ ID NO: 65 - DNA, 60 bp, Artificial Sequence
  Synthetic Polynucleotide
ccgtctcagactccccaattttcccaaacagaggtgctaagtccaaaacctccgagacga

SEQ ID NO: 66 - DNA, 61 bp, Artificial Sequence
  Synthetic Polynucleotide
tcgtctcggaggttttggacttagctacctctgtttgggaaaattggggagtctgagacgg

SEQ ID NO: 67 - DNA, 61 bp, Artificial Sequence
  Synthetic Polynucleotide
ccgtctcagactccccaattttcccaaacagaggtagctaagtccaaaacctccgagacga

SEQ ID NO: 68 - DNA, 54 bp, Artificial Sequence
  Synthetic Polynucleotide
tcgtctctgcacccccaattttcccaaacagaggtctgtaaaccgatgagacgg

SEQ ID NO: 69 - DNA, 54 bp, Artificial Sequence
  Synthetic Polynucleotide
ccgtctcatcggtttacagacctctgtttgggaaaattgggggtgcagagacga

SEQ ID NO: 70 - DNA, 55 bp, Artificial Sequence
  Synthetic Polynucleotide
tcgtctctgcacccccaattttcccaaacagaggttctgtaaaccgatgagacgg

SEQ ID NO: 71 - DNA, 55 bp, Artificial Sequence
  Synthetic Polynucleotide
ccgtctcatcggtttacagaacctctgtttgggaaaattgggggtgcagagacga

SEQ ID NO: 72 - DNA, 56 bp, Artificial Sequence
  Synthetic Polynucleotide
tcgtctctgcacccccaattttcccaaacagaggtatctgtaaaccgatgagacgg

SEQ ID NO: 73 - DNA, 56 bp, Artificial Sequence
  Synthetic Polynucleotide
ccgtctcatcggtttacagatacctctgtttgggaaaattgggggtgcagagacga

SEQ ID NO: 74 - DNA, 57 bp, Artificial Sequence
  Synthetic Polynucleotide
tcgtctctgcacccccaattttcccaaacagaggtaatctgtaaaccgatgagacgg

SEQ ID NO: 75 - DNA, 57 bp, Artificial Sequence
  Synthetic Polynucleotide
ccgtctcatcggtttacagattacctctgtttgggaaaattgggggtgcagagacga

SEQ ID NO: 76 - DNA, 58 bp, Artificial Sequence
  Synthetic Polynucleotide
tcgtctctgcacccccaattttcccaaacagaggtaaatctgtaaaccgatgagacgg

SEQ ID NO: 77 - DNA, 58 bp, Artificial Sequence
  Synthetic Polynucleotide
ccgtctcatcggtttacagatttacctctgtttgggaaaattgggggtgcagagacga

SEQ ID NO: 78 - DNA, 59 bp, Artificial Sequence
  Synthetic Polynucleotide
tcgtctctgcacccccaattttcccaaacagaggtgaaatctgtaaaccgatgagacgg

SEQ ID NO: 79 - DNA, 59 bp, Artificial Sequence
  Synthetic Polynucleotide
ccgtctcatcggtttacagatttcacctctgtttgggaaaattgggggtgcagagacga

SEQ ID NO: 80 - DNA, 60 bp, Artificial Sequence
  Synthetic Polynucleotide
tcgtctctgcacccccaattttcccaaacagaggtcgaaatctgtaaaccgatgagacgg

SEQ ID NO: 81 - DNA, 60 bp, Artificial Sequence
  Synthetic Polynucleotide
ccgtctcatcggtttacagatttcgacctctgtttgggaaaattgggggtgcagagacga

SEQ ID NO: 82 - DNA, 61 bp, Artificial Sequence
  Synthetic Polynucleotide
tcgtctctgcacccccaattttcccaaacagaggttcgaaatctgtaaaccgatgagacgg

SEQ ID NO: 83 - DNA, 61 bp, Artificial Sequence
  Synthetic Polynucleotide
ccgtctcatcggtttacagatttcgaacctctgtttgggaaaattgggggtgcagagacga

SEQ ID NO: 84 - DNA, 56 bp, Artificial Sequence
  Synthetic Polynucleotide
tcgtctcgccgaggttttggaacctctgtttgggaaaattggggctcgtgagacgg

SEQ ID NO: 85 - DNA, 56 bp, Artificial Sequence
  Synthetic Polynucleotide
ccgtctcacgagccccaattttcccaaacagaggttccaaaacctcggcgagacga

SEQ ID NO: 86 - DNA, 57 bp, Artificial Sequence
  Synthetic Polynucleotide
tcgtctcgccgaggttttggacacctctgtttgggaaaattggggctcgtgagacgg

SEQ ID NO: 87 - DNA, 57 bp, Artificial Sequence
  Synthetic Polynucleotide
ccgtctcacgagccccaattttcccaaacagaggtgtccaaaacctcggcgagacga

SEQ ID NO: 88 - DNA, 58 bp, Artificial Sequence
  Synthetic Polynucleotide
tcgtctcgccgaggttttggactacctctgtttgggaaaattggggctcgtgagacgg

SEQ ID NO: 89 - DNA, 58 bp, Artificial Sequence
  Synthetic Polynucleotide
ccgtctcacgagccccaattttcccaaacagaggtagtccaaaacctcggcgagacga

SEQ ID NO: 90 - DNA, 59 bp, Artificial Sequence
  Synthetic Polynucleotide
tcgtctcgccgaggttttggacttacctctgtttgggaaaattggggctcgtgagacgg

SEQ ID NO: 91 - DNA, 59 bp, Artificial Sequence
  Synthetic Polynucleotide
ccgtctcacgagccccaattttcccaaacagaggtaagtccaaaacctcggcgagacga

SEQ ID NO: 92 - DNA, 60 bp, Artificial Sequence
  Synthetic Polynucleotide
tcgtctcgccgaggttttggacttaacctctgtttgggaaaattggggctcgtgagacgg

SEQ ID NO: 93 - DNA, 60 bp, Artificial Sequence
  Synthetic Polynucleotide
ccgtctcacgagccccaattttcccaaacagaggttaagtccaaaacctcggcgagacga

SEQ ID NO: 94 - DNA, 61 bp, Artificial Sequence
  Synthetic Polynucleotide
tcgtctcgccgaggttttggacttagacctctgtttgggaaaattggggctcgtgagacgg

SEQ ID NO: 95 - DNA, 61 bp, Artificial Sequence
  Synthetic Polynucleotide
ccgtctcacgagccccaattttcccaaacagaggtctaagtccaaaacctcggcgagacga

SEQ ID NO: 96 - DNA, 62 bp, Artificial Sequence
  Synthetic Polynucleotide
tcgtctcgccgaggttttggacttagcacctctgtttgggaaaattggggctcgtgagacgg

SEQ ID NO: 97 - DNA, 62 bp, Artificial Sequence
  Synthetic Polynucleotide
ccgtctcacgagccccaattttcccaaacagaggtgctaagtccaaaacctcggcgagacga

SEQ ID NO: 98 - DNA, 63 bp, Artificial Sequence
  Synthetic Polynucleotide
tcgtctcgccgaggttttggacttagctacctctgtttgggaaaattggggctcgtgagacgg

SEQ ID NO: 99 - DNA, 63 bp, Artificial Sequence
  Synthetic Polynucleotide
ccgtctcacgagccccaattttcccaaacagaggtagctaagtccaaaacctcggcgagacga

SEQ ID NO: 100 - DNA, 58 bp, Artificial Sequence
  Synthetic Polynucleotide
tcgtctcggcgtcccctcccatcacaggccctgaggtttaagagaaaacctgagacgg

SEQ ID NO: 101 - DNA, 58 bp, Artificial Sequence
  Synthetic Polynucleotide
ccgtctcaggttttctcttaaacctcagggcctgtgatgggaggggacgccgagacga

SEQ ID NO: 102 - DNA, 64 bp, Artificial Sequence
  Synthetic Polynucleotide
tcgtctcgaaccatggttttgtgggccaggcccatgacccttctcctctgggagtctgagacgg

SEQ ID NO: 103 - DNA, 64 bp, Artificial Sequence
  Synthetic Polynucleotide
ccgtctcagactcccagaggagaagggtcatgggcctggcccacaaaaccatggttcgagacga

SEQ ID NO: 104 - DNA, 60 bp, Artificial Sequence
  Synthetic Polynucleotide
tcgtctctgcaccccctcccatcacaggccctgaggtttaagagaaaaccattgagacgg

SEQ ID NO: 105 - DNA, 60 bp, Artificial Sequence
  Synthetic Polynucleotide
ccgtctcaatggttttctcttaaacctcagggcctgtgatgggagggggtgcagagacga

SEQ ID NO: 106 - DNA, 62 bp, Artificial Sequence
  Synthetic Polynucleotide
tcgtctcgccatggttttgtgggccaggcccatgacccttctcctctgggctcgtgagacgg

SEQ ID NO: 107 - DNA, 62 bp, Artificial Sequence
  Synthetic Polynucleotide
ccgtctcacgagcccagaggagaagggtcatgggcctggcccacaaaaccatggcgagacga

SEQ ID NO: 108 - DNA, 43 bp, Artificial Sequence
  Synthetic Polynucleotide
atccgtctccagtcgagtcggatttgatctgatcaagagacag

SEQ ID NO: 109 - DNA, 45 bp, Artificial Sequence
  Synthetic Polynucleotide
aaccgtctcggtgcgttcggatttgatccagacatgataagatac

SEQ ID NO: 110 - DNA, 30 bp, Artificial Sequence
  Synthetic Polynucleotide
hscgcgttgagacgctgccatccgtctcgc

SEQ ID NO: 111 - DNA, 30 bp, Artificial Sequence
  Synthetic Polynucleotide
hstcgagcgagacggatggcagcgtctcaa

SEQ ID NO: 112 - DNA, 130 bp, Artificial Sequence
  Synthetic Polynucleotide
gttgttcgtctcggcgtccttgtgttgtgtgtcttcaactcacagagttaaacgatgctttacacagagtagacttgaaacactctttttctggagtctgagacggttctgttttggtgtgattagttat

SEQ ID NO: 113 - DNA, 130 bp, Artificial Sequence
  Synthetic Polynucleotide
gttggtcgtctctgcacccttgtgttgtgtgtcttcaactcacagagttaaacgatgctttacacagagtagacttgaaacactctttttctggctcgtgagacggttctgttttggtgtgattagttat

SEQ ID NO: 114 - DNA, 131 bp, Artificial Sequence
  Synthetic Polynucleotide
gttgttcgtctcggcgtcccaccggctcatgagaggtagagctaaggtccaaacctaggtttatctgagaccggaactcatgtgattaactgtggagtctgagacggttctgttttggtgtgattagttat

SEQ ID NO: 115 - DNA, 131 bp, Artificial Sequence
  Synthetic Polynucleotide
gttggtcgtctctgcaccccaccggctcatgagaggtagagctaaggtccaaacctaggtttatctgagaccggaactcatgtgattaactgtggctcgtgagacggttctgttttggtgtgattagttat

SEQ ID NO: 116 - DNA, 130 bp, Artificial Sequence
  Synthetic Polynucleotide
gttgttcgtctcggcgtccttaagaacataaatccccaggaattcacagaaaccttggtttgagctttggatttcccgcaggatgtgggataggagtctgagacggttctgttttggtgtgattagttat

SEQ ID NO: 117 - DNA, 130 bp, Artificial Sequence
  Synthetic Polynucleotide
gttggtcgtctctgcacccttaagaacataaatccccaggaattcacagaaaccttggtttgagctttggatttcccgcaggatgtgggataggctcgtgagacggttctgttttggtgtgattagttat

SEQ ID NO: 118 - DNA, 129 bp, Artificial Sequence
  Synthetic Polynucleotide
gttgttcgtctcggcgtccactccctctcccccaaaaagtaaaggtagaaaaccaaggtttacaggcaacaaatagcacaatgaatggaatggagtctgagacggttctgttttggtgtgattagttat

SEQ ID NO: 119 - DNA, 129 bp, Artificial Sequence
  Synthetic Polynucleotide
gttggtcgtctctgcacccactccctctcccccaaaaagtaaaggtagaaaaccaaggtttacaggcaacaaatagcacaatgaatggaatggctcgtgagacggttctgttttggtgtgattagttat

SEQ ID NO: 120 - DNA, 130 bp, Artificial Sequence
  Synthetic Polynucleotide
gttgttcgtctcggcgtcctagggaagtgatcatagctgagtttctggaaaaacctaggttttaaagttgaggagacttaagtccaaaacctggagtctgagacggttctgttttggtgtgattagttat

SEQ ID NO: 121 - DNA, 130 bp, Artificial Sequence
  Synthetic Polynucleotide
gttggtcgtctctgcaccctagggaagtgatcatagctgagtttctggaaaaacctaggttttaaagttgaggagacttaagtccaaaacctggctcgtgagacggttctgttttggtgtgattagttat

SEQ ID NO: 122 - DNA, 47 bp, Artificial Sequence
  Synthetic Polynucleotide
ttcatcggatccgataaaaagtattctattggtttagctatcggcac

SEQ ID NO: 123 - DNA, 34 bp, Artificial Sequence
  Synthetic Polynucleotide
ttcatcggatccggtggttcaggtggcagcggag

SEQ ID NO: 124 - DNA, 61 bp, Artificial Sequence
  Synthetic Polynucleotide
ttcatcggatccggagggtccggaggtagtggcggcagcggtggttcaggtggcagcggag

SEQ ID NO: 125 - DNA, 100 bp, Artificial Sequence
  Synthetic Polynucleotide
aataaccggttcagaccttccttttcttctttggggaacctcccttgtcgtcatcatccttataatcggagccaccgtcacccccaagctgtgacaaatc

SEQ ID NO: 126 - DNA, 38 bp, Artificial Sequence
  Synthetic Polynucleotide
tgataaggatccaccctttggtggtcttccaaaccgcc

SEQ ID NO: 127 - DNA, 38 bp, Artificial Sequence
  Synthetic Polynucleotide
tgataaggatccaccgctaccaccctttggtggtcttc

SEQ ID NO: 128 - DNA, 20 bp, Artificial Sequence
  Synthetic Polynucleotide
agatccgcggccgctaatac

SEQ ID NO: 129 - DNA, 54 bp, Artificial Sequence
  Synthetic Polynucleotide
ttgagtcgtctctatactcttcctttttcaatattattgaagcatttatcaggg

SEQ ID NO: 130 - DNA, 50 bp, Artificial Sequence
  Synthetic Polynucleotide
ctggaacgtctcactgtcagaccaagtttactcatatatactttagattg

SEQ ID NO: 131 - DNA, 46 bp, Artificial Sequence
  Synthetic Polynucleotide
ggtgtgcgtctctacagttatttgccgactaccttggtgatctcgc

SEQ ID NO: 132 - DNA, 36 bp, Artificial Sequence
  Synthetic Polynucleotide
acaccacgtctctgtatgagggaagcggtgatcgcc

SEQ ID NO: 133 - DNA, 42 bp, Artificial Sequence
  Synthetic Polynucleotide
catactcttcctttttcaatattattgaagcatttatcaggg

SEQ ID NO: 134 - DNA, 37 bp, Artificial Sequence
  Synthetic Polynucleotide
ctgtcagaccaagtttactcatatatactttagattg

SEQ ID NO: 135 - DNA, 62 bp, Artificial Sequence
  Synthetic Polynucleotide
caatctaaagtatatatgagtaaacttggtctgacagtttgccgactaccttggtgatctcg

SEQ ID NO: 136 - DNA, 65 bp, Artificial Sequence
  Synthetic Polynucleotide
caatctaaagtatatatgagtaaacttggtctgacagttatttgccgactaccttggtgatctcg

SEQ ID NO: 137 - DNA, 42 bp, Artificial Sequence
  Synthetic Polynucleotide
ccctgataaatgcttcaataatattgaaaaaggaagagtatg

SEQ ID NO: 138 - DNA, 21 bp, Artificial Sequence
  Synthetic Polynucleotide
cgcaaatgggcggtaggcgtg

SEQ ID NO: 139 - DNA, 20 bp, Artificial Sequence
  Synthetic Polynucleotide
ccgtgatggattggtgaatc

SEQ ID NO: 140 - DNA, 20 bp, Artificial Sequence
  Synthetic Polynucleotide
cccatacgatttcacctgtc

SEQ ID NO: 141 - DNA, 20 bp, Artificial Sequence
  Synthetic Polynucleotide
gggtattttccacaggatgc

SEQ ID NO: 142 - DNA, 20 bp, Artificial Sequence
  Synthetic Polynucleotide
cttagaaaggcgggtttacg

SEQ ID NO: 143 - DNA, 20 bp, Artificial Sequence
  Synthetic Polynucleotide
cttactaagctgcaatttgg

SEQ ID NO: 144 - DNA, 21 bp, Artificial Sequence
  Synthetic Polynucleotide
tgtattcatcggttatgacag

SEQ ID NO: 145 - DNA, 19 bp, Artificial Sequence
  Synthetic Polynucleotide
cagggtcaaggaaggcacg

SEQ ID NO: 146 - DNA, 17 bp, Artificial Sequence
  Synthetic Polynucleotide
gttccgcgcacatttcc

SEQ ID NO: 147 - DNA, 19 bp, Artificial Sequence
  Synthetic Polynucleotide
gcggagcctatggaaaaac

SEQ ID NO: 148 - DNA, 22 bp, Artificial Sequence
  Synthetic Polynucleotide
gccttcttctttttcctacagc

SEQ ID NO: 149 - DNA, 16 bp, Artificial Sequence
  Synthetic Polynucleotide
cgcatcgagcgagcac

SEQ ID NO: 150 - DNA, 27 bp, Artificial Sequence
  Synthetic Polynucleotide
tcaagtagcaaaagaagtaggagtcag

SEQ ID NO: 151 - DNA, 22 bp, Artificial Sequence
  Synthetic Polynucleotide
ttagatgcattcgtgcttgaag

SEQ ID NO: 152 - DNA, 29 bp, Artificial Sequence
  Synthetic Polynucleotide
ttaatttctgctgctagaactaaatctgg

SEQ ID NO: 153 - DNA, 24 bp, Artificial Sequence
  Synthetic Polynucleotide
gggaagaaaactggatggagaatg

SEQ ID NO: 154 - DNA, 22 bp, Artificial Sequence
  Synthetic Polynucleotide
cataaatgacctagtggagctg

SEQ ID NO: 155 - DNA, 26 bp, Artificial Sequence
  Synthetic Polynucleotide
tggttattttgcccattagttgatgc

SEQ ID NO: 156 - DNA, 1318 bp, Artificial Sequence
  Synthetic Polynucleotide
acgcgtccccaattttcccaaacagaggtctgtaaaccgaggttttggaacctctgtttgggaaaattggggagtcgagtcggatttgatctgatcaagagacaggatgaggatcgtttcgcatgattgaacaagatggattgcacgcaggttctccggccgcttgggtggagaggctattcggctatgactgggcacaacagacaatcggctgctctgatgccgccgtgttccggctgtcagtcgcaggggcgcccggttctttttgtcaagaccgacctgtccggtgccctgaatgaactgcaggacgaggcagcgcggctatcgtggctggccacgacgggcgttccttgcgcagctgtgctcgacgttgtcactgaagcgggaagggactggctgctattgggcgaagtgccggggcaggatctcctgtcatctcaccttgctcctgccgagaaagtatccatcatggctgatgcaatgcggcggctgcatacgcttgatccggctacctgcccattcgaccaccaagcgaaacatcgcatcgagcgagcacgtactcggatggaagccggtcttgtcgatcaggatgatctggacgaagagcatcaggggctcgcgccagccgaactgttcgccaggctcaaggcgcgcatgcccgacggcgaggatctcgtcgtgacccatggcgatgcctgcttgccgaatatcatggtggaaaatggccgcttttctggattcatcgactgtggccggctgggtgtggcggaccgctatcaggacatagcgttggctacccgtgatattgctgaagagcttggcggcgaatgggctgaccgcttcctcgtgctttacggtatcgccgctcccgattcgcagcgcatcgccttctatcgccttcttgacgagttcttctgagcgggactctggggttcgaaatgaccgaccaagcgacgcccaacctgccatcacgagatttcgattccaccgccgccttctatgaaaggttgggcttcggaatcgttttccgggacgccggctggatgatcctccagcgcggggatctcatgctggagttcttcgcccaccccatcgataacttgtttattgcagcttataatggttacaaataaagcaatagcatcacaaatttcacaaataaagcatttttttcactgcattctagttgtggtttgtccaaactcatcaatgtatcttatcatgtctggatcaaatccgaacgcacccccaattttcccaaacagaggtctgtaaaccgaggttttggaacctctgtttgggaaaattggggctcgag

SEQ ID NO: 157 - DNA, 67 bp, Artificial Sequence
  Synthetic Polynucleotide
ccccaattttcccaaacagaggttctgtaaaccgaggttttggaacctctgtttgggaaaattgggg

SEQ ID NO: 158 - DNA, 68 bp, Artificial Sequence
  Synthetic Polynucleotide
ccccaattttcccaaacagaggttctgtaaaccgaggttttggcaacctctgtttgggaaaattgggg

SEQ ID NO: 159 - DNA, 70 bp, Artificial Sequence
  Synthetic Polynucleotide
ccccaattttcccaaacagaggtatctgtaaaccgaggttttggctaacctctgtttgggaaaattgggg

SEQ ID NO: 160 - DNA, 72 bp, Artificial Sequence
  Synthetic Polynucleotide
ccccaattttcccaaacagaggtaatctgtaaaccgaggttttggcttaacctctgtttgggaaaattgggg

SEQ ID NO: 161 - DNA, 74 bp, Artificial Sequence
  Synthetic Polynucleotide
ccccaattttcccaaacagaggtaaatctgtaaaccgaggttttggcttaaacctctgtttgggaaaattgggg

SEQ ID NO: 162 - DNA, 76 bp, Artificial Sequence
  Synthetic Polynucleotide
ccccaattttcccaaacagaggtgaaatctgtaaaccgaggttttggcttagaacctctgtttgggaaaattgggg

SEQ ID NO: 163 - DNA, 78 bp, Artificial Sequence
  Synthetic Polynucleotide
ccccaattttcccaaacagaggtcgaaatctgtaaaccgaggttttggcttagcaacctctgtttgggaaaattgggg

SEQ ID NO: 164 - DNA, 80 bp, Artificial Sequence
  Synthetic Polynucleotide
ccccaattttcccaaacagaggttcgaaatctgtaaaccgaggttttggcttagctaacctctgtttgggaaaattgggg

SEQ ID NO: 165 - DNA, 73 bp, Artificial Sequence
  Synthetic Polynucleotide
ccccaattttcccaaacagaggttcgaaatctgtaaaccgaggttttggaacctctgtttgggaaaattgggg

SEQ ID NO: 166 - DNA, 74 bp, Artificial Sequence
  Synthetic Polynucleotide
ccccaattttcccaaacagaggttcgaaatctgtaaaccgaggttttggcaacctctgtttgggaaaattgggg

SEQ ID NO: 167 - DNA, 74 bp, Artificial Sequence
  Synthetic Polynucleotide
ccccaattttcccaaacagaggtcgaaatctgtaaaccgaggttttggctaacctctgtttgggaaaattgggg

SEQ ID NO: 168 - DNA, 76 bp, Artificial Sequence
  Synthetic Polynucleotide
ccccaattttcccaaacagaggtcgaaatctgtaaaccgaggttttggcttaaacctctgtttgggaaaattgggg

SEQ ID NO: 169 - DNA, 77 bp, Artificial Sequence
  Synthetic Polynucleotide
ccccaattttcccaaacagaggtcgaaatctgtaaaccgaggttttggcttagaacctctgtttgggaaaattgggg

SEQ ID NO: 170 - DNA, 72 bp, Artificial Sequence
  Synthetic Polynucleotide
ccccaattttcccaaacagaggtctgtaaaccgaggttttggcttagcaacctctgtttgggaaaattgggg

SEQ ID NO: 171 - DNA, 73 bp, Artificial Sequence
  Synthetic Polynucleotide
ccccaattttcccaaacagaggttctgtaaaccgaggttttggcttagcaacctctgtttgggaaaattgggg

SEQ ID NO: 172 - DNA, 74 bp, Artificial Sequence
  Synthetic Polynucleotide
ccccaattttcccaaacagaggtatctgtaaaccgaggttttggcttagcaacctctgtttgggaaaattgggg

SEQ ID NO: 173 - DNA, 75 bp, Artificial Sequence
  Synthetic Polynucleotide
ccccaattttcccaaacagaggtaatctgtaaaccgaggttttggcttagcaacctctgtttgggaaaattgggg

SEQ ID NO: 174 - DNA, 76 bp, Artificial Sequence
  Synthetic Polynucleotide
ccccaattttcccaaacagaggtaaatctgtaaaccgaggttttggcttagcaacctctgtttgggaaaattgggg

SEQ ID NO: 175 - DNA, 77 bp, Artificial Sequence
  Synthetic Polynucleotide
ccccaattttcccaaacagaggtgaaatctgtaaaccgaggttttggcttagcaacctctgtttgggaaaattgggg

SEQ ID NO: 176 - DNA, 78 bp, Artificial Sequence
  Synthetic Polynucleotide
cccctcccatcacaggccctgaggtttaagagaaaaccatggttttgtgggccaggcccatgacccttctcctctggg

SEQ ID NO: 177 - DNA, 77 bp, Artificial Sequence
  Synthetic Polynucleotide
ccttgtgttgtgtgtcttcaactcacagagttaaacgatgctttacacagagtagacttgaaacactctttttctgg

SEQ ID NO: 178 - DNA, 77 bp, Artificial Sequence
  Synthetic Polynucleotide
ccaccggctcatgagaggtagagctaaggtccaaacctaggtttatctgagaccggaactcatgtgattaactgtgg

SEQ ID NO: 179 - DNA, 77 bp, Artificial Sequence
  Synthetic Polynucleotide
ccttaagaacataaatccccaggaattcacagaaaccttggtttgagctttggatttcccgcaggatgtgggatagg

SEQ ID NO: 180 - DNA, 76 bp, Artificial Sequence
  Synthetic Polynucleotide
ccactccctctcccccaaaaagtaaaggtagaaaaccaaggtttacaggcaacaaatagcacaatgaatggaatgg

SEQ ID NO: 181 - DNA, 77 bp, Artificial Sequence
  Synthetic Polynucleotide
cctagggaagtgatcatagctgagtttctggaaaaacctaggttttaaagttgaggagacttaagtccaaaacctgg

SEQ ID NO: 182 - protein, 6 aa, Artificial Sequence
  Synthetic Polypeptide
GGSGGS

SEQ ID NO: 183 - protein, 24 aa, Artificial Sequence
  Synthetic Polypeptide
GGSGGSGGSGGSGGSGGSGGSGGS

SEQ ID NO: 184 - DNA, 4665 bp, Artificial Sequence
  Synthetic Polynucleotide
atgctcattggctacgtgcgcgtctcaactaacgaccagaataccgatcttcagaggaacgcactggtttgtgcaggctgcgaacagattttcgaggacaaactcagcgggacacggacggacagacctggcctcaagcgagcactcaagaggctgcagaaaggagacactctggtggtctggaaattggaccgcctgggtcgaagcatgaagcatctcatttctctggttggcgaactgcgagaaagggggatcaactttcgaagtctgacggattccatagatacaagcagccccatgggccggttcttcttctacgtgatgggtgcactggctgaaatggaaagagaactcattatagagcgaaccatggcagggcttgcggctgccaggaataaaggcaggcggtttggaagaccaccaaagggtggatccggagggtccggaggtagtggcggcagcggtggttcaggtggcagcggagggtcaggaggctctgataaaaagtattctattggtttagctatcggcactaattccgttggatgggctgtcataaccgatgaatacaaagtaccttcaaagaaatttaaggtgttggggaacacagaccgtcattcgattaaaaagaatcttatcggtgccctcctattcgatagtggcgaaacggcagaggcgactcgcctgaaacgaaccgctcggagaaggtatacacgtcgcaagaaccgaatatgttacttacaagaaatttttagcaatgagatggccaaagttgacgattctttctttcaccgtttggaagagtccttccttgtcgaagaggacaagaaacatgaacggcaccccatctttggaaacatagtagatgaggtggcatatcatgaaaagtacccaacgatttatcacctcagaaaaaagctagttgactcaactgataaagcggacctgaggttaatctacttggctcttgcccatatgataaagttccgtgggcactttctcattgagggtgatctaaatccggacaactcggatgtcgacaaactgttcatccagttagtacaaacctataatcagttgtttgaagagaaccctataaatgcaagtggcgtggatgcgaaggctattcttagcgcccgcctctctaaatcccgacggctagaaaacctgatcgcacaattacccggagagaagaaaaatgggttgttcggtaaccttatagcgctctcactaggcctgacaccaaattttaagtcgaacttcgacttagctgaagatgccaaattgcagcttagtaaggacacgtacgatgacgatctcgacaatctactggcacaaattggagatcagtatgcggacttatttttggctgccaaaaaccttagcgatgcaatcctcctatctgacatactgagagttaatactgagattaccaaggcgccgttatccgcttcaatgatcaaaaggtacgatgaacatcaccaagacttgacacttctcaaggccctagtccgtcagcaactgcctgagaaatataaggaaatattctttgatcagtcgaaaaacgggtacgcaggttatattgacggcggagcgagtcaagaggaattctacaagtttatcaaacccatattagagaagatggatgggacggaagagttgcttgtaaaactcaatcgcgaagatctactgcgaaagcagcggactttcgacaacggtagcattccacatcaaatccacttaggcgaattgcatgctatacttagaaggcaggaggatttttatccgttcctcaaagacaatcgtgaaaagattgagaaaatcctaacctttcgcataccttactatgtgggacccctggcccgagggaactctcggttcgcatggatgacaagaaagtccgaagaaacgattactccatggaattttgaggaagttgtcgataaaggtgcgtcagctcaatcgttcatcgagaggatgaccaactttgacaagaatttaccgaacgaaaaagtattgcctaagcacagtttactttacgagtatttcacagtgtacaatgaactcacgaaagttaagtatgtcactgagggcatgcgtaaacccgcctttctaagcggagaacagaagaaagcaatagtagatctgttattcaagaccaaccgcaaagtgacagttaagcaattgaaagaggactactttaagaaaattgaatgcttcgattctgtcgagatctccggggtagaagatcgatttaatgcgtcacttggtacgtatcatgacctcctaaagataattaaagataaggacttcctggataacgaagagaatgaagatatcttagaagatatagtgttgactcttaccctctttgaagatcgggaaatgattgaggaaagactaaaaacatacgctcacctgttcgacgataaggttatgaaacagttaaagaggcgtcgctatacgggctggggacgattgtcgcggaaacttatcaacgggataagagacaagcaaagtggtaaaactattctcgattttctaaagagcgacggcttcgccaataggaactttatgcagctgatccatgatgactctttaaccttcaaagaggatatacaaaaggcacaggtttccggacaaggggactcattgcacgaacatattgcgaatcttgctggttcgccagccatcaaaaagggcatactccagacagtcaaagtagtggatgagctagttaaggtcatgggacgtcacaaaccggaaaacattgtaatcgagatggcacgcgaaaatcaaacgactcagaaggggcaaaaaaacagtcgagagcggatgaagagaatagaagagggtattaaagaactgggcagccagatcttaaaggagcatcctgtggaaaatacccaattgcagaacgagaaactttacctctattacctacaaaatggaagggacatgtatgttgatcaggaactggacataaaccgtttatctgattacgacgtcgatgccattgtaccccaatcctttttgaaggacgattcaatcgacaataaagtgcttacacgctcggataagaaccgagggaaaagtgacaatgttccaagcgaggaagtcgtaaagaaaatgaagaactattggcggcagctcctaaatgcgaaactgataacgcaaagaaagttcgataacttaactaaagctgagaggggtggcttgtctgaacttgacaaggccggatttattaaacgtcagctcgtggaaacccgccaaatcacaaagcatgttgcacagatactagattcccgaatgaatacgaaatacgacgagaacgataagctgattcgggaagtcaaagtaatcactttaaagtcaaaattggtgtcggacttcagaaaggattttcaattctataaagttagggagataaataactaccaccatgcgcacgacgcttatcttaatgccgtcgtagggaccgcactcattaagaaatacccgaagctagaaagtgagtttgtgtatggtgattacaaagtttatgacgtccgtaagatgatcgcgaaaagcgaacaggagataggcaaggctacagccaaatacttcttttattctaacattatgaatttctttaagacggaaatcactctggcaaacggagagatacgcaaacgacctttaattgaaaccaatggggagacaggtgaaatcgtatgggataagggccgggacttcgcgacggtgagaaaagttttgtccatgccccaagtcaacatagtaaagaaaactgaggtgcagaccggagggttttcaaaggaatcgattcttccaaaaaggaatagtgataagctcatcgctcgtaaaaaggactgggacccgaaaaagtacggtggcttcgatagccctacagttgcctattctgtcctagtagtggcaaaagttgagaagggaaaatccaagaaactgaagtcagtcaaagaattattggggataacgattatggagcgctcgtcttttgaaaagaaccccatcgacttccttgaggcgaaaggttacaaggaagtaaaaaaggatctcataattaaactaccaaagtatagtctgtttgagttagaaaatggccgaaaacggatgttggctagcgccggagagcttcaaaaggggaacgaactcgcactaccgtctaaatacgtgaatttcctgtatttagcgtcccattacgagaagttgaaaggttcacctgaagataacgaacagaagcaactttttgttgagcagcacaaacattatctcgacgaaatcatagagcaaatttcggaattcagtaagagagtcatcctagctgatgccaatctggacaaagtattaagcgcatacaacaagcacagggataaacccatacgtgagcaggcggaaaatattatccatttgtttactcttaccaacctcggcgctccagccgcattcaagtattttgacacaacgatagatcgcaaacgatacacttctaccaaggaggtgctagacgcgacactgattcaccaatccatcacgggattatatgaaactcggatagatttgtcacagcttgggggtgacggtggctccgattataaggatgatgacgacaagggaggttccccaaagaagaaaaggaaggtctga

SEQ ID NO: 185 - protein, 1554 aa, Artificial Sequence
  Synthetic Polypeptide
MLIGYVRVSTNDQNTDLQRNALVCAGCEQIFEDKLSGTRTDRPGLKRALKRLQKGDTLVVWKLDRLGRSMKHLISLVGELRERGINFRSLTDSIDTSSPMGRFFFYVMGALAEMERELIIERTMAGLAAARNKGRRFGRPPKGGSGGSGGSGGSGGSGGSGGSGGSDKKYSIGLAIGTNSVGWAVITDEYKVPSKKFKVLGNTDRHSIKKNLIGALLFDSGETAEATRLKRTARRRYTRRKNRICYLQEIFSNEMAKVDDSFFHRLEESFLVEEDKKHERHPIFGNIVDEVAYHEKYPTIYHLRKKLVDSTDKADLRLIYLALAHMIKFRGHFLIEGDLNPDNSDVDKLFIQLVQTYNQLFEENPINASGVDAKAILSARLSKSRRLENLIAQLPGEKKNGLFGNLIALSLGLTPNFKSNFDLAEDAKLQLSKDTYDDDLDNLLAQIGDQYADLFLAAKNLSDAILLSDILRVNTEITKAPLSASMIKRYDEHHQDLTLLKALVRQQLPEKYKEIFFDQSKNGYAGYIDGGASQEEFYKFIKPILEKMDGTEELLVKLNREDLLRKQRTFDNGSIPHQIHLGELHAILRRQEDFYPFLKDNREKIEKILTFRIPYYVGPLARGNSRFAWMTRKSEETITPWNFEEVVDKGASAQSFIERMTNFDKNLPNEKVLPKHSLLYEYFTVYNELTKVKYVTEGMRKPAFLSGEQKKAIVDLLFKTNRKVTVKQLKEDYFKKIECFDSVEISGVEDRFNASLGTYHDLLKIIKDKDFLDNEENEDILEDIVLTLTLFEDREMIEERLKTYAHLFDDKVMKQLKRRRYTGWGRLSRKLINGIRDKQSGKTILDFLKSDGFANRNFMQLIHDDSLTFKEDIQKAQVSGQGDSLHEHIANLAGSPAIKKGILQTVKVVDELVKVMGRHKPENIVIEMARENQTTQKGQKNSRERMKRIEEGIKELGSQILKEHPVENTQLQNEKLYLYYLQNGRDMYVDQELDINRLSDYDVDAIVPQSFLKDDSIDNKVLTRSDKNRGKSDNVPSEEVVKKMKNYWRQLLNAKLITQRKFDNLTKAERGGLSELDKAGFIKRQLVETRQITKHVAQILDSRMNTKYDENDKLIREVKVITLKSKLVSDFRKDFQFYKVREINNYHHAHDAYLNAVVGTALIKKYPKLESEFVYGDYKVYDVRKMIAKSEQEIGKATAKYFFYSNIMNFFKTEITLANGEIRKRPLIETNGETGEIVWDKGRDFATVRKVLSMPQVNIVKKTEVQTGGFSKESILPKRNSDKLIARKKDWDPKKYGGFDSPTVAYSVLVVAKVEKGKSKKLKSVKELLGITIMERSSFEKNPIDFLEAKGYKEVKKDLIIKLPKYSLFELENGRKRMLASAGELQKGNELALPSKYVNFLYLASHYEKLKGSPEDNEQKQLFVEQHKHYLDEIIEQISEFSKRVILADANLDKVLSAYNKHRDKPIREQAENIIHLFTLTNLGAPAAFKYFDTTIDRKRYTSTKEVLDATLIHQSITGLYETRIDLSQLGGDGGSDYKDDDDKGGSPKKKRKV

SEQ ID NO: 186 - DNA, 18 bp, Artificial Sequence
  Synthetic Polynucleotide
ggtggtagcggtggatcc

SEQ ID NO: 187 - DNA, 45 bp, Artificial Sequence
  Synthetic Polynucleotide
ggtggatccggtggttcaggtggcagcggagggtcaggaggctct

SEQ ID NO: 188 - DNA, 72 bp, Artificial Sequence
  Synthetic Polynucleotide
ggtggatccggagggtccggaggtagtggcggcagcggtggttcaggtggcagcggagggtcaggaggctct

SEQ ID NO: 189 - DNA, 20 bp, Artificial Sequence
  Synthetic Polynucleotide
acctctgtttgggaaaattg

SEQ ID NO: 190 - DNA, 21 bp, Artificial Sequence
  Synthetic Polynucleotide
gcacactagttagggataaca

SEQ ID NO: 191 - DNA, 21 bp, Artificial Sequence
  Synthetic Polynucleotide
gcctcagggcctgtgatggga

SEQ ID NO: 192 - DNA, 21 bp, Artificial Sequence
  Synthetic Polynucleotide
gctcagggcctgtgatgggag

SEQ ID NO: 193 - DNA, 20 bp, Artificial Sequence
  Synthetic Polynucleotide
ggcccatgacccttctcctc

SEQ ID NO: 194 - DNA, 20 bp, Artificial Sequence
  Synthetic Polynucleotide
gcccatgacccttctcctct

SEQ ID NO: 195 - DNA, 20 bp, Artificial Sequence
  Synthetic Polynucleotide
gacttgaaacactctttttc

SEQ ID NO: 196 - DNA, 21 bp, Artificial Sequence
  Synthetic Polynucleotide
gagttgaagacacacaacaca

SEQ ID NO: 197 - DNA, 20 bp, Artificial Sequence
  Synthetic Polynucleotide
ggaactcatgtgattaactg

SEQ ID NO: 198 - DNA, 21 bp, Artificial Sequence
  Synthetic Polynucleotide
gtctacctctcatgagccggt

SEQ ID NO: 199 - DNA, 21 bp, Artificial Sequence
  Synthetic Polynucleotide
gtttcccgcaggatgtgggat

SEQ ID NO: 200 - DNA, 21 bp, Artificial Sequence
  Synthetic Polynucleotide
gcctggggatttatgttctta

SEQ ID NO: 201 - DNA, 21 bp, Artificial Sequence
  Synthetic Polynucleotide
gaaatagcacaatgaatggaa

SEQ ID NO: 202 - DNA, 21 bp, Artificial Sequence
  Synthetic Polynucleotide
gactttttgggggagagggag

SEQ ID NO: 203 - DNA, 20 bp, Artificial Sequence
  Synthetic Polynucleotide
ggagacttaagtccaaaacc

SEQ ID NO: 204 - DNA, 21 bp, Artificial Sequence
  Synthetic Polynucleotide
gtcagctatgatcacttccct

SEQ ID NO: 205 - DNA, 20 bp, Artificial Sequence
  Synthetic Polynucleotide
gcagatgtagtgtttccaca

SEQ ID NO: 206 - DNA, 20 bp, Artificial Sequence
  Synthetic Polynucleotide
gggtggggggagtttgctcc

SEQ ID NO: 207 - DNA, 21 bp, Artificial Sequence
  Synthetic Polynucleotide
gatatccgtttatcagtgtca

SEQ ID NO: 208 - DNA, 21 bp, Artificial Sequence
  Synthetic Polynucleotide
gttcctaagcttgggctgcag

SEQ ID NO: 209 - DNA, 21 bp, Artificial Sequence
  Synthetic Polynucleotide
gcctaaaagtgactgggagaa

SEQ ID NO: 210 - DNA, 21 bp, Artificial Sequence
  Synthetic Polynucleotide
gcacagtcccatatttcttgg

SEQ ID NO: 211 - DNA, 77 bp, Artificial Sequence
  Synthetic Polynucleotide
cctttagtgaaaagtagacagctctgaatatgaaaggtaggttttcatttctgggaaagagacgccaagtgatgtgg

SEQ ID NO: 212 - DNA, 78 bp, Artificial Sequence
  Synthetic Polynucleotide
cctccaataaatatgggactatgtggaaagaccaaacctacgtttgattggtgtacctgaaagtgacgggaagaatgg

SEQ ID NO: 213 - DNA, 78 bp, Artificial Sequence
  Synthetic Polynucleotide
ccattctgcccgtcactttcaggtacaccaatcaaacgtaggtttagtcttttcacatagtcccatatttcttggagg

SEQ ID NO: 214 - DNA, 78 bp, Artificial Sequence
  Synthetic Polynucleotide
ccattctccccgtcactttcaggtacaacaatcaaacgtaggtttggtcttttcacatagtcccatatttcttggagg

SEQ ID NO: 215 - DNA, 77 bp, Artificial Sequence
  Synthetic Polynucleotide
ccttgtagtgtgtgtattcaactcacagagttaaacgatcctttacacagagcagacttgaaacactcttgttgtgg

SEQ ID NO: 216 - DNA, 77 bp, Artificial Sequence
  Synthetic Polynucleotide
ccttgtagtgtgtgtattcaactcacagagttaaacgatcctttacacagagcatacttgaaacactctttttgtgg

SEQ ID NO: 217 - DNA, 77 bp, Artificial Sequence
  Synthetic Polynucleotide
ccttgtgttgtgtgtattcaactcacagagttaaacgatcctttacacagagcagacttgaaacactctttttgtgg

SEQ ID NO: 218 - DNA, 77 bp, Artificial Sequence
  Synthetic Polynucleotide
ccttgtgttgtgtttattcaactcacagagttaaacgatcctttacacagagcagacttgaaatactctttttgtgg

SEQ ID NO: 219 - DNA, 77 bp, Artificial Sequence; identical to SEQ ID NO: 216
  Synthetic Polynucleotide

SEQ ID NO: 220 - DNA, 77 bp, Artificial Sequence
  Synthetic Polynucleotide
ccttgtattgtgagtattcaactcacagagttaaacgatcctttacacagagcagacttgaaacactctttttgtgg

SEQ ID NO: 221 - DNA, 77 bp, Artificial Sequence; identical to SEQ ID NO: 177
  Synthetic Polynucleotide

SEQ ID NO: 222 - DNA, 77 bp, Artificial Sequence
  Synthetic Polynucleotide
ccttgtgttgtgtgtattcaactcacagagttaaacgatcctttacacagagcagacttgtaacactctttttgtgg

SEQ ID NO: 223 - DNA, 77 bp, Artificial Sequence
  Synthetic Polynucleotide
ccttgtgttgtgtgtattcaactcacagagttaaacgatcctttacacagagcagacgtgaaacactctttttgtgg

SEQ ID NO: 224 - DNA, 77 bp, Artificial Sequence; identical to SEQ ID NO: 217
  Synthetic Polynucleotide

SEQ ID NO: 225 - DNA, 77 bp, Artificial Sequence
  Synthetic Polynucleotide
ccttgtgttgtgtgtattcaactcacagagttaaacgatcctttacacagaggagacttgtaacactctttttgtgg

SEQ ID NO: 226 - DNA, 77 bp, Artificial Sequence
  Synthetic Polynucleotide
cctgaggttttccaggttttaaaaggaaacctaaaggtaggtttagcattaagtgtcttgaagtttattttaaaagg

SEQ ID NO: 227 - DNA, 76 bp, Artificial Sequence
  Synthetic Polynucleotide
ccaaaattcccacaaaaccgaatgcatcagtcaaagcaaggtttgaagaaaagatttaccacttcagggagcttgg

SEQ ID NO: 228 - DNA, 77 bp, Artificial Sequence
  Synthetic Polynucleotide
ccttttctggatatcgttgatgctctgtatgcaaaaggtaggtttttgggttatgttgttaaacagtgattgaatgg

SEQ ID NO: 229 - DNA, 78 bp, Artificial Sequence
  Synthetic Polynucleotide
cctccaagaaatatggaactatgtgaaaagaccaaacctacgtttgattggtgtacctgaaagtgacagagagaatgg

SEQ ID NO: 230 - DNA, 78 bp, Artificial Sequence
  Synthetic Polynucleotide
cctccaagaaatatgggactatgtgagaagaccaaacctacgtttgattggtgtacctgaaagtgatggggagaatgg

SEQ ID NO: 231 - DNA, 78 bp, Artificial Sequence
  Synthetic Polynucleotide
ccattctccccatcgctttcaggtacaccaatcaaacgtaggtttggtcttttcacatagttccatattctttggagg

SEQ ID NO: 232 - DNA, 78 bp, Artificial Sequence
  Synthetic Polynucleotide
ccattctccccatcactttcaggtgtaccgatcaaacgtaggtttggtcttttcacatagtcccatatttcttggagg

SEQ ID NO: 233 - DNA, 78 bp, Artificial Sequence
  Synthetic Polynucleotide
cctccaagaaatatgggactatgtgaaaagaccaaacctacgtttgattggtgtacctgaaagtgacggggagaatgg

SEQ ID NO: 234 - DNA, 76 bp, Artificial Sequence
  Synthetic Polynucleotide
ccttcagggcagaaacagctctactagcagagaaagcaagctttcaatattgtgcaatacaaaaacgagagcaggg

SEQ ID NO: 235 - DNA, 78 bp, Artificial Sequence
  Synthetic Polynucleotide
ccattctcctcatctccttctggtactccaatcaaacgtaggtttggtcttttctcatagtctcatatttcttggagg

SEQ ID NO: 236 - DNA, 78 bp, Artificial Sequence
  Synthetic Polynucleotide
cctccaagacatataggactatgtgaaaataccaaacctacgtttgattggtgtacctgaaagtgacagggagtatgg

SEQ ID NO: 237 - DNA, 76 bp, Artificial Sequence
  Synthetic Polynucleotide
cctgccagataccagtagtcactgtgaattacaaagctacgtttcttccatagggaaagtttggagtccagccagg

SEQ ID NO: 238 - DNA, 78 bp, Artificial Sequence
  Synthetic Polynucleotide
ccattctccctgtcactttcaggtacaccaatcaaacgtaggtttggtcttttcacatagtcccatatttcttggagg

SEQ ID NO: 239 - DNA, 78 bp, Artificial Sequence
  Synthetic Polynucleotide
ccattctccccaccactttcaggtacaccaatcaaacgtaggtttggtcttttcacatagtcccatatttcttgtagg

SEQ ID NO: 240 - DNA, 78 bp, Artificial Sequence
  Synthetic Polynucleotide
cctaaccagaaactaactaatagatatgggcagaaagcatcctttcacttttgttctgggagagggaagaagcaaagg

SEQ ID NO: 241 - DNA, 77 bp, Artificial Sequence
  Synthetic Polynucleotide
ccattttggggaggccttgatgggaagctggaaaaggaagctttcctcccagtcctgctgaaggccttgccagctgg

SEQ ID NO: 242 - DNA, 78 bp, Artificial Sequence
  Synthetic Polynucleotide
cctccaagaaacacaggactatgtgaaaagatcaaacctacgtttgattggtgttcctgaaagtgatggggagaatgg

SEQ ID NO: 243 - DNA, 78 bp, Artificial Sequence
  Synthetic Polynucleotide
ccattctcttcatgactttcaggtacaccattgaaacgtaggtttggtcttttcacattgtcccatatttcttggagg

SEQ ID NO: 244 - DNA, 78 bp, Artificial Sequence
  Synthetic Polynucleotide
ccattctccccatcactttcaggtacaccaatcaaacgtaggtttggtcttttcacatagtcccgtatttcttggtgg

SEQ ID NO: 245 - DNA, 78 bp, Artificial Sequence
  Synthetic Polynucleotide
ccattctccctgtcactttcaggtacaccaatcaaacgtaggtttggtcttttcacatagtcccatatttcttggggg

SEQ ID NO: 246 - DNA, 77 bp, Artificial Sequence
  Synthetic Polynucleotide
ccattctccctgtcactttcaggtacaccaatcaaacgtaggtttggtcttttcacatagtcccatatttcttgggg

SEQ ID NO: 247 - DNA, 78 bp, Artificial Sequence
  Synthetic Polynucleotide
cctccaagaaatatgagattatatgaaaagaccaaacctacgtttgattggtgtactttaaagtgacggggagaatgg

SEQ ID NO: 248 - DNA, 78 bp, Artificial Sequence
  Synthetic Polynucleotide
ccattctccccgtcattttcaggtacaccaatcaaacgtaggtttggtcttttcacatagtcccaaatttcttggagg

SEQ ID NO: 249 - DNA, 78 bp, Artificial Sequence
  Synthetic Polynucleotide
cccccaagaaatgtgggactatatgaaaagaccaaacctacgtttgactggtgtacctaaaagtgatggggagaatgg

SEQ ID NO: 250 - DNA, 77 bp, Artificial Sequence
  Synthetic Polynucleotide
ccccaagaaatgtgggactatatgaaaagaccaaacctacgtttgactggtgtacctaaaagtgatggggagaatgg

SEQ ID NO: 251 - DNA, 77 bp, Artificial Sequence
  Synthetic Polynucleotide
cccattggtgctgaccagatggtgaaggaggcaaaggttgctttgaatgactgtgctctggggtgagccaggcctgg

SEQ ID NO: 252 - DNA, 76 bp, Artificial Sequence
  Synthetic Polynucleotide
ccctttacagaggtgagctttgttattagtaaaaaggtaggtttccctgtttttctgaagaaaagctgtgagtggg

SEQ ID NO: 253 - DNA, 78 bp, Artificial Sequence
  Synthetic Polynucleotide
ccactgcccattgacagagtggcgaggtgggtgaaaccttgctttcctcctggcccatgggcagggtggggctgtggg

SEQ ID NO: 254 - DNA, 77 bp, Artificial Sequence
  Synthetic Polynucleotide
ccactgcccattgacagagtggcgaggtgggtgaaaccttgctttcctcctggcccatgggcagggtggggctgtgg

SEQ ID NO: 255 - DNA, 78 bp, Artificial Sequence
  Synthetic Polynucleotide
ccattctccctgtcacttttagatacaccaatcaaacgtaggtttggtcttttcacatagtcccatgtttcttggagg

SEQ ID NO: 256 - DNA, 77 bp, Artificial Sequence
  Synthetic Polynucleotide
cctccaagaaatatcaactgtgtgaaaagacgaaacctacgtttgattaatgtacctgaaagtgacagggagaatgg

SEQ ID NO: 257 - DNA, 78 bp, Artificial Sequence
  Synthetic Polynucleotide
ccattctcccattaactttcaagtacaccaatcaaaggtaggtttggtgttttcccatagtcccgtatttcttggagg

SEQ ID NO: 258 - DNA, 78 bp, Artificial Sequence
  Synthetic Polynucleotide
ccttttcatcatgcccctttcactttaaggtgaaaaccttgctttacatgtcagagaaaagaagagccctcagctggg

SEQ ID NO: 259 - DNA, 77 bp, Artificial Sequence
  Synthetic Polynucleotide
ccttttcatcatgcccctttcactttaaggtgaaaaccttgctttacatgtcagagaaaagaagagccctcagctgg

SEQ ID NO: 260 - DNA, 78 bp, Artificial Sequence
  Synthetic Polynucleotide
ccattcaccccgtcactttcaggtacaccaatcaaacgtaggtttggtcttttcacatagtcccatatttcttggagg

SEQ ID NO: 261 - DNA, 77 bp, Artificial Sequence
  Synthetic Polynucleotide
cctccaagaaatatgggactatgtgaaaagaccaaacctacgtttgatggtgtacccgaaagtgacagggagaatgg

SEQ ID NO: 262 - DNA, 78 bp, Artificial Sequence
  Synthetic Polynucleotide
ccaccaagaaatatgggactatgtgaaaagaccaaacctacgtttgataggtatacctgaaagtgacagggagaatgg

SEQ ID NO: 263 - DNA, 78 bp, Artificial Sequence
  Synthetic Polynucleotide
ccattctccccatcactttcaggtgcaccaatcaaacgtaggtttggtcttttcacatagtcccatatttcttggagg

SEQ ID NO: 264 - DNA, 78 bp, Artificial Sequence
  Synthetic Polynucleotide
ccctcaagaaatatgagactatgtgaaaagaccaaacctacgtttgactggtatacctgaaagtgacagggagaatgg

SEQ ID NO: 265 - DNA, 77 bp, Artificial Sequence
  Synthetic Polynucleotide
cctcaagaaatatgagactatgtgaaaagaccaaacctacgtttgactggtatacctgaaagtgacagggagaatgg

SEQ ID NO: 266 - DNA, 78 bp, Artificial Sequence
  Synthetic Polynucleotide
cctccaacaaatatgggactatgtgaaaagaccaaacctacgtttgattggtgtacctgaaagtgacggggataatgg

SEQ ID NO: 267 - DNA, 78 bp, Artificial Sequence
  Synthetic Polynucleotide
ccattctctccctcactttcaagtacaccaatcaaacgtaggtttggtcttttcacatagtcttatatttcttggcgg

SEQ ID NO: 268 - DNA, 77 bp, Artificial Sequence
  Synthetic Polynucleotide
ccattctccctgtcactgtcagtacaccaatcaaacgtaggtttggtctcttcacatagtcccatatttcttggagg

SEQ ID NO: 269 - DNA, 77 bp, Artificial Sequence
  Synthetic Polynucleotide
cctccaagaaatatgggactatgtgaacagaccaaacctacgtttgattggtgtacctgaaagtgatggcagaatgg

SEQ ID NO: 270 - DNA, 77 bp, Artificial Sequence
  Synthetic Polynucleotide
ccaccatgcctggccaccacacatttttttctaaagcttggttttggccacagtgagagtttcttgggctgtcaggg

SEQ ID NO: 271 - DNA, 76 bp, Artificial Sequence
  Synthetic Polynucleotide
ccaccatgcctggccaccacacatttttttctaaagcttggttttggccacagtgagagtttcttgggctgtcagg

SEQ ID NO: 272 - DNA, 77 bp, Artificial Sequence
  Synthetic Polynucleotide
cccactaggtggcgatatctgagggtccaatgaaaccatgctttttactcagatcttccactaaccacctcccccgg

SEQ ID NO: 273 - DNA, 78 bp, Artificial Sequence
  Synthetic Polynucleotide
cctctaagaaatatgggactatgtgaaaagaccaaacctacgtttgactggtgtacctgaaagtgacggggagaatgg

SEQ ID NO: 274 - DNA, 78 bp, Artificial Sequence
  Synthetic Polynucleotide
cctccaagaaatatgggactatgtgaaaagaccaaacctacgtttgattagtgtacctgaaagtgacggggagaatgg

SEQ ID NO: 275 - DNA, 78 bp, Artificial Sequence
  Synthetic Polynucleotide
ccattctccctgtcactttcaggtacatcaatcaaacgtaggtttggtcttttcacatagtcccatatttcttggagg

SEQ ID NO: 276 - DNA, 78 bp, Artificial Sequence
  Synthetic Polynucleotide
cctccaagaaatatgggactatgtgaaaagaccaaacctacgtttgactggtgtacctgaaagggatggggagaatgg

SEQ ID NO: 277 - DNA, 78 bp, Artificial Sequence
  Synthetic Polynucleotide
cccccaagaaatatgagactatgtgaaaagaccaaacctacgtttgattggtgtacctgaaagtgacagggagaatgg

SEQ ID NO: 278 - DNA, 77 bp, Artificial Sequence
  Synthetic Polynucleotide
ccccaagaaatatgagactatgtgaaaagaccaaacctacgtttgattggtgtacctgaaagtgacagggagaatgg

SEQ ID NO: 279 - DNA, 78 bp, Artificial Sequence
  Synthetic Polynucleotide
cctctaagaaatatgggactatgtgaaaagaccaaacctacgtttgattggtgtaactgaaagtgacagggagaatgg

SEQ ID NO: 280 - DNA, 78 bp, Artificial Sequence
  Synthetic Polynucleotide
cctccaagaaatatgcgcctatgtgaaaagaccaaacctacgtttgattggtatacctgaaagtgatggagagaatgg

SEQ ID NO: 281 - DNA, 78 bp, Artificial Sequence
  Synthetic Polynucleotide
ccattctccctgtcactttgaggtacaccaatcaaacgtaggtttggtcttttcacatattcgcatatttcttggagg

SEQ ID NO: 282 - DNA, 78 bp, Artificial Sequence
  Synthetic Polynucleotide
ccattctccccgtcactttcaggtacaccaaccaaacgttggtttggtcttttcacatagtcccatatttcttggagg

SEQ ID NO: 283 - DNA, 78 bp, Artificial Sequence
  Synthetic Polynucleotide
ccattctccctgtcactttccagtacaccagtcaaacgtaggtttggtcttttcacatactcccatatttcttggagg

SEQ ID NO: 284 - DNA, 77 bp, Artificial Sequence
  Synthetic Polynucleotide
cctggcctaatttttaattcttagtttgacttaaaccttgcttttagtgtgatggcgacaaaagctgagctgaaagg

SEQ ID NO: 285 - DNA, 76 bp, Artificial Sequence
  Synthetic Polynucleotide
ccagtgctttttggttttaaaggcaagcctccaaaccttcctttctcctggatgctgtggtggttgccatgcatgg

SEQ ID NO: 286 - DNA, 76 bp, Artificial Sequence
  Synthetic Polynucleotide
cccaactcctgcgagaagtagctcaccatgacaaagctacctttgcttttatcgttttgcaaaacaaaaaaggggg

SEQ ID NO: 287 - DNA, 78 bp, Artificial Sequence
  Synthetic Polynucleotide
ccattctccccgtcactttgaggtgtgccaatcaaacgtaggtttggtcttttcacatagtcctatatttcttggagg

SEQ ID NO: 288 - DNA, 78 bp, Artificial Sequence
  Synthetic Polynucleotide
cctccaaaaaatatgggactacgtaaaaagaccaaacctacgtttgattggtgtacctgaaactgacagggagaatgg

SEQ ID NO: 289 - DNA, 78 bp, Artificial Sequence
  Synthetic Polynucleotide
ccattctccccgtcactttcaggtacaccaatcaaacgtaggtttggtcttttcacatagttccatatttcttggagg

SEQ ID NO: 290 - DNA, 78 bp, Artificial Sequence
  Synthetic Polynucleotide
cctacaagatatatgggactatgtgaaaagaccaaacctacgttttactggtgtgcctgaaactgacggggagaatgg

SEQ ID NO: 291 - DNA, 78 bp, Artificial Sequence
  Synthetic Polynucleotide
ccattctctctgtcactttcaggtacaccaatcaaacgtaggtttggtcttttcacatagtcccatatttcttggagg

SEQ ID NO: 292 - DNA, 78 bp, Artificial Sequence
  Synthetic Polynucleotide
cctccaagaaatatgggactatgtgaaaagaccaaacctacgtttcattggtgtacctgaaagtgatagggagaatgg

SEQ ID NO: 293 - DNA, 78 bp, Artificial Sequence
  Synthetic Polynucleotide
cctccaaaaaatatgggatgatgtgaaaagaccaaacctaggtttgactggtgtacctgaaaatgatggggagaatgg

SEQ ID NO: 294 - DNA, 78 bp, Artificial Sequence
  Synthetic Polynucleotide
cctccaagaaatatgagactatgtgaaaagaccaaacctacgtttgattggtgtacctgaaagtgacagggagaatgg

SEQ ID NO: 295 - DNA, 78 bp, Artificial Sequence
  Synthetic Polynucleotide
cctccaagaaatatgggactacgtgaaaagatcaaacctacgtttgattgttgtacctgaaagtgatggggagaatgg

SEQ ID NO: 296 - DNA, 78 bp, Artificial Sequence
  Synthetic Polynucleotide
cctccaagaaatatgggactatgtgaaaagaccaaacctacgtttgattgttgtacctgaaagtgatggggagaatgg

SEQ ID NO: 297 - DNA, 78 bp, Artificial Sequence
  Synthetic Polynucleotide
cctcaaaagtgttctggttttgttttgttttttaaaccatggttttacctctggcttagtgggactaaaaataggagg

SEQ ID NO: 298 - DNA, 78 bp, Artificial Sequence
  Synthetic Polynucleotide
cctccaagaaatatgggactatgtgaaaagaccaaacctacgtttgactggtgtacctgaaagtgatggggaaaatgg

SEQ ID NO: 299 - DNA, 78 bp, Artificial Sequence
  Synthetic Polynucleotide
cctccaagaaatatgggactgtgtgtaaagaccaaacctacgtttgattggtgtacctcaaagtgatggggagaatgg

SEQ ID NO: 300 - DNA, 78 bp, Artificial Sequence
  Synthetic Polynucleotide
ccattctccccatcacattcaggtacaccaatcaaacgtaggtttggtcttttcacatagtcccatatttcttggagg

SEQ ID NO: 301 - DNA, 77 bp, Artificial Sequence
  Synthetic Polynucleotide
cccctggaaaagttggagcatcacaggaaaagcaaaccaaccttttttctcccctaggtaaactggggagccagggg

SEQ ID NO: 302 - DNA, 76 bp, Artificial Sequence
  Synthetic Polynucleotide
ccctggaaaagttggagcatcacaggaaaagcaaaccaaccttttttctcccctaggtaaactggggagccagggg

SEQ ID NO: 303 - DNA, 77 bp, Artificial Sequence
  Synthetic Polynucleotide
ccttccccagttgcagcagacaagagtctcgaaaagcttgctttggttgctgcagtggatgggttggtaggcacagg

SEQ ID NO: 304 - DNA, 76 bp, Artificial Sequence
  Synthetic Polynucleotide
cccccacctcccaagctgctggcttctcgaataaagctacctttccttttaccaaaacttgtctctcgaatgtcgg

SEQ ID NO: 305 - DNA, 77 bp, Artificial Sequence
  Synthetic Polynucleotide
ccttggccctggacagctgcttttccttccctaaaccttggtttccccctttgtgcaggtgggtgggtttgggctgg

SEQ ID NO: 306 - DNA, 78 bp, Artificial Sequence
  Synthetic Polynucleotide
cctcttctagtgaacccatggggttaccaagggaaagcaaccttttgataaatattcccatctttttatgttgtctgg

SEQ ID NO: 307 - DNA, 78 bp, Artificial Sequence
  Synthetic Polynucleotide
ccacttgaaagggttaccaaggataagatttttaaagcttgctttcacaaacaactcatgctccaggcttgtcagtgg

SEQ ID NO: 308 - DNA, 78 bp, Artificial Sequence
  Synthetic Polynucleotide
cctttctccccatcactttcaggtacaccaatcaaacgtaggtttgatcttttcacatagtcccatatttcttggagg

SEQ ID NO: 309 - DNA, 78 bp, Artificial Sequence
  Synthetic Polynucleotide
ccattctccccatcaatttcagttacaccaatgaaacgtaggtttggccttttcacatagtcccatatttcttagagg

SEQ ID NO: 310 - DNA, 78 bp, Artificial Sequence
  Synthetic Polynucleotide
ccattctccctgtcactctcaggtacaccaatcaaacgtaggtttggtcttttcatatagtcccatatttcttggagg

SEQ ID NO: 311 - DNA, 77 bp, Artificial Sequence
  Synthetic Polynucleotide
cctccaagaaaattgggactatgtgaaaaaaccaaacctacgtttgattgatgtacctgaaagtgacaggagaatgg

SEQ ID NO: 312 - DNA, 78 bp, Artificial Sequence
  Synthetic Polynucleotide
ccttcaagaaatatgggactatgtgaaaggacaaaacctacgttttattggtgtacctgaaagtgacagggagaatgg

SEQ ID NO: 313 - DNA, 78 bp, Artificial Sequence
  Synthetic Polynucleotide
ccattctccccatcactttcaggtacgctaatcaaacgtaggtttgatcttttcacatagtcttatatttcttggagg

SEQ ID NO: 314 - DNA, 78 bp, Artificial Sequence
  Synthetic Polynucleotide
cctccaagaaatatgggactatgtgaaaagaccaaacctacgtttgactggtgtacctcaatgtgacagggagaatgg

SEQ ID NO: 315 - DNA, 78 bp, Artificial Sequence
  Synthetic Polynucleotide
ccattctccctgtcacttttaggtacaccaatcaaacgtacgtttggtcttttcacatagacccatatttcttggagg

SEQ ID NO: 316 - DNA, 78 bp, Artificial Sequence
  Synthetic Polynucleotide
ccttcaagaaatatgggactgtgtgaaaagaccaaagctaggtttgattggtgtacctgaaagtgatggggagaatgg

SEQ ID NO: 317 - DNA, 76 bp, Artificial Sequence
  Synthetic Polynucleotide
cctactattcacagagtaatgcagtttgctgaaaaggttggtttttgctgacctctgagagctcacattacagtgg

SEQ ID NO: 318 - DNA, 78 bp, Artificial Sequence
  Synthetic Polynucleotide
ccattctctctgtcactttctggtacaccaatcaaacgtaggtttgctcttttcacataatcccatatttattgaagg

SEQ ID NO: 319 - DNA, 77 bp, Artificial Sequence
  Synthetic Polynucleotide
ccataacatgtatttgctggtgctagactctccaaagctaggtttctttctacaacaatggctggaagtcttcttgg

SEQ ID NO: 320 - DNA, 78 bp, Artificial Sequence
  Synthetic Polynucleotide
ccattctccccatcactttcaggtacaccaatcaaacgtaggtttggtcttctcacacagtcccatatttcttggagg

SEQ ID NO: 321 - DNA, 78 bp, Artificial Sequence
  Synthetic Polynucleotide
ccattcttcccattactttcaggtacaccaatcaaacgtaggtttggtcttttcacatagtcccacatttcttggagg

SEQ ID NO: 322 - DNA, 78 bp, Artificial Sequence
  Synthetic Polynucleotide
ccattctccccctcactttcaggtacaccaatcaaacgtaggtttggtcttttcacattgtcccatatttcttggagg

SEQ ID NO: 323 - DNA, 78 bp, Artificial Sequence
  Synthetic Polynucleotide
ccattctccccagcacttacaggtacaccaatcaaacgtaggtttggtcatttcacatagtcccatatttcttggagg

SEQ ID NO: 324 - DNA, 78 bp, Artificial Sequence
  Synthetic Polynucleotide
ccattctccctgtcactttcaggtacagcaatcaaacgtaggtttggtcttttcacatggtcccatatttcttggagg

SEQ ID NO: 325 - DNA, 78 bp, Artificial Sequence
  Synthetic Polynucleotide
cctccaagaaatatgagactatgtgaaaagaccaaacctacgtttgattggtgtacctgaaagtgacggggaagatgg

SEQ ID NO: 326 - DNA, 78 bp, Artificial Sequence; identical to SEQ ID NO: 294
  Synthetic Polynucleotide

SEQ ID NO: 327 - DNA, 78 bp, Artificial Sequence
  Synthetic Polynucleotide
cctccaagagatatgagactatgtaaatagaccaaacctacctttgattggtgtacgtgaaagtgacaggaagaatgg

SEQ ID NO: 328 - DNA, 78 bp, Artificial Sequence
  Synthetic Polynucleotide
ccattctccccatcactttcaggtacaccaaccaaacgtaggtttggtcttttcacatagtctcatatttcttggagg

SEQ ID NO: 329 - DNA, 76 bp, Artificial Sequence
  Synthetic Polynucleotide
cctccattgactactccttatcattggctagaaaacctacctttcaaccagtttctaaggccaagaaacttggagg

SEQ ID NO: 330 - DNA, 78 bp, Artificial Sequence
  Synthetic Polynucleotide
ccaccaagaaatatgggactacgtgaaaagaccaaacctacgtttgatgggtgtgcctgaaagtgacgggaagaatgg

SEQ ID NO: 331 - DNA, 78 bp, Artificial Sequence
  Synthetic Polynucleotide
cctccaagaaataagggactatgtgaaaagaccaaacctacgtttgattggtgtacctgaaggtgacagggagaatgg

SEQ ID NO: 332 - DNA, 77 bp, Artificial Sequence
  Synthetic Polynucleotide
ccaaagggcctttgtgattctactttgtaatataaaggatggtttcttactacggttggtgtccttgcaggagtggg

SEQ ID NO: 333 - DNA, 78 bp, Artificial Sequence
  Synthetic Polynucleotide
cctccaagaaatatgggactatgtgaaaagaccaaacctacgtttgattggtgtacctgaaagtgatggggagaatgg

SEQ ID NO: 334 - DNA, 78 bp, Artificial Sequence
  Synthetic Polynucleotide
ccattctccccgttactttcaggtacaccaataaaacctaggtttggtcttttcacatagtcccatatttcttggagg

SEQ ID NO: 335 - DNA, 76 bp, Artificial Sequence
  Synthetic Polynucleotide
cccatatctctggcaagggcagctctctggctaaaccaagctttcctgtagagcttgagttccaaggcagcgttgg

SEQ ID NO: 336 - DNA, 77 bp, Artificial Sequence; identical to SEQ ID NO: 215
  Synthetic Polynucleotide

SEQ ID NO: 337 - DNA, 77 bp, Artificial Sequence; identical to SEQ ID NO: 216
  Synthetic Polynucleotide

SEQ ID NO: 338 - DNA, 77 bp, Artificial Sequence; identical to SEQ ID NO: 217
  Synthetic Polynucleotide

SEQ ID NO: 339 - DNA, 77 bp, Artificial Sequence; identical to SEQ ID NO: 218
  Synthetic Polynucleotide

SEQ ID NO: 340 - DNA, 77 bp, Artificial Sequence; identical to SEQ ID NO: 216
  Synthetic Polynucleotide

SEQ ID NO: 341 - DNA, 77 bp, Artificial Sequence; identical to SEQ ID NO: 220
  Synthetic Polynucleotide

SEQ ID NO: 342 - DNA, 77 bp, Artificial Sequence; identical to SEQ ID NO: 177
  Synthetic Polynucleotide

SEQ ID NO: 343 - DNA, 77 bp, Artificial Sequence; identical to SEQ ID NO: 222
  Synthetic Polynucleotide

SEQ ID NO: 344 - DNA, 77 bp, Artificial Sequence; identical to SEQ ID NO: 223
  Synthetic Polynucleotide

SEQ ID NO: 345 - DNA, 77 bp, Artificial Sequence; identical to SEQ ID NO: 217
  Synthetic Polynucleotide

SEQ ID NO: 346 - DNA, 77 bp, Artificial Sequence; identical to SEQ ID NO: 225
  Synthetic Polynucleotide

SEQ ID NO: 347 - DNA, 77 bp, Artificial Sequence
  Synthetic Polynucleotide
ccttttcataagaagaaaatcgactcatcattgaaaccaagctttggtacaatttcattgatgtttccagaagcagg

SEQ ID NO: 348 - DNA, 76 bp, Artificial Sequence
  Synthetic Polynucleotide
cccatagactatgatagaaacaaaataacccaaaagctagctttctgattgagtttccataaatgcaatgtgaagg

SEQ ID NO: 349 - DNA, 77 bp, Artificial Sequence
  Synthetic Polynucleotide
ccattcacttgtcactttctggtacaccaatcaaacgtaggtttggtcttttcacatagtctcatatttcttggagg

SEQ ID NO: 350 - DNA, 78 bp, Artificial Sequence
  Synthetic Polynucleotide
cctccaagaaatatgggactctgtaaagagaccaaacctacgtttgattggtgtacctgaaagtgaaggggagaatgg

SEQ ID NO: 351 - DNA, 78 bp, Artificial Sequence
  Synthetic Polynucleotide
ccattctccccgtcattttcaggtacaccaatcaaacctaggtttggtctttttacatagtcccatatttcttggagg

SEQ ID NO: 352 - DNA, 78 bp, Artificial Sequence
  Synthetic Polynucleotide
cctccacgaaacatgggactatgtgaaaagaccaaacctacgtttgattggtgtacctgaaagtgacagggagaatgg

SEQ ID NO: 353 - DNA, 78 bp, Artificial Sequence
  Synthetic Polynucleotide
ccaatttccccctcactttcagatacaccaatcaaacgtaggtttggtcttttcacatagttccatatttcctggagg

SEQ ID NO: 354 - DNA, 78 bp, Artificial Sequence
  Synthetic Polynucleotide
ccattctccccatcactttcaggtacaccaatcaaacgtaggtttggtcttttcacatattcccatatgtcttggagg

SEQ ID NO: 355 - DNA, 78 bp, Artificial Sequence
  Synthetic Polynucleotide
cccaccggctcatgagaggtagagctaaggtccaaacctaggtttatctgagaccggaactcatgtgattaactgtgg

SEQ ID NO: 356 - DNA, 77 bp, Artificial Sequence; identical to SEQ ID NO: 178
  Synthetic Polynucleotide

SEQ ID NO: 357 - DNA, 78 bp, Artificial Sequence
  Synthetic Polynucleotide
ccttcaagaaatatgggactatgtgaagagaccaaacctacgtttgattggtgtagccaaaagtgatggggaaaatgg

SEQ ID NO: 358 - DNA, 78 bp, Artificial Sequence
  Synthetic Polynucleotide
cctcagattagatttacttgcaaagagacatttaaaggatcgttttgatactattttgaaagtactatacaaagatgg

SEQ ID NO: 359 - DNA, 77 bp, Artificial Sequence; identical to SEQ ID NO: 179
  Synthetic Polynucleotide

SEQ ID NO: 360 - DNA, 78 bp, Artificial Sequence
  Synthetic Polynucleotide
ccattctctctgtcactttcaggtacaccaatcaaacgtaggtttggtcttttctcatagtcccatatttcttggagg

SEQ ID NO: 361 - DNA, 76 bp, Artificial Sequence
  Synthetic Polynucleotide
ccatttaccatcattctctgtcatggcaggtgaaagcaagcttttatatagacaatgttctacttagtttacaggg

SEQ ID NO: 362 - DNA, 77 bp, Artificial Sequence
  Synthetic Polynucleotide
cccaaagttaattttactctttttctgaatcaaaaggaacctttcctccatgagaagaatcctgccatatttctagg

SEQ ID NO: 363 - DNA, 78 bp, Artificial Sequence
  Synthetic Polynucleotide
cctccaagaaatatgggactatgtgaaaagaccaaacctacgtttgattgctatacatgaaagtgacggggagaatgg

SEQ ID NO: 364 - DNA, 78 bp, Artificial Sequence
  Synthetic Polynucleotide
ccttcaagaaatatgggactatgtgaaaagaccaaacctacctttgattggtgtacctgaaagtgatgggaagaatgg

SEQ ID NO: 365 - DNA, 78 bp, Artificial Sequence
  Synthetic Polynucleotide
ccattctccccatcactttcaggtacaccaatcaaacgtaggtttggtcttttcacatagtcccatagttcttggagg

SEQ ID NO: 366 - DNA, 78 bp, Artificial Sequence
  Synthetic Polynucleotide
ccattctccccgtcactttcagggacaacaatcaaacgtaggtttggcctttgcacatagtcttatatttcttggagg

SEQ ID NO: 367 - DNA, 78 bp, Artificial Sequence
  Synthetic Polynucleotide
ccattctccccatcactttcaggtacaccaatcaaacgtaggtttggtcttttcacatagtcccatatttcttggagg

SEQ ID NO: 368 - DNA, 78 bp, Artificial Sequence
  Synthetic Polynucleotide
cctccaaaaaatatgggactatgtgagaagaccaaacctacgttttattagtgtacctcaaagtgacagggaggatgg

SEQ ID NO: 369 - DNA, 78 bp, Artificial Sequence
  Synthetic Polynucleotide
ccattctccccatcactttcaggtacaccaatgaaacgtaggtttggccttttcacatagtttcatatttcttggagg

SEQ ID NO: 370 - DNA, 78 bp, Artificial Sequence; identical to SEQ ID NO: 333
  Synthetic Polynucleotide

SEQ ID NO: 371 - DNA, 77 bp, Artificial Sequence
  Synthetic Polynucleotide
cctacaagaaatatggaacttgtaaaaagaccaaacctacgtttgattggtgtacctgaaagtgacggggagaatgg

SEQ ID NO: 372 - DNA, 78 bp, Artificial Sequence
  Synthetic Polynucleotide
cctccaagaaatatgggacaatgtgaaaaggccaaagctacgtttgattggtgtacctgaaagtgacagggagaatgg

SEQ ID NO: 373 - DNA, 78 bp, Artificial Sequence
  Synthetic Polynucleotide
cctttcaaacttagaggtaaacaaaagtcctgaaaacctaggtttgaccataagttgggaccatacgagcatagaagg

SEQ ID NO: 374 - DNA, 78 bp, Artificial Sequence
  Synthetic Polynucleotide
ccaaaaataaaaaaaaattgacttataagtaagaaaggttcgttttctcacattcagaaagagaacccacatgttggg

SEQ ID NO: 375 - DNA, 77 bp, Artificial Sequence
  Synthetic Polynucleotide
ccaaaaataaaaaaaaattgacttataagtaagaaaggttcgttttctcacattcagaaagagaacccacatgttgg

SEQ ID NO: 376 - DNA, 78 bp, Artificial Sequence; identical to SEQ ID NO: 367
  Synthetic Polynucleotide

SEQ ID NO: 377 - DNA, 78 bp, Artificial Sequence
  Synthetic Polynucleotide
ccattctccccgtcactttcaggtacaccaatcaaacgttggtttagtctattcacatagtcccatatttcttggagg

SEQ ID NO: 378 - DNA, 78 bp, Artificial Sequence
  Synthetic Polynucleotide
ccgaaaagaataagactatcagctgaagtcttaaaacgatcctttggcccccagtactctatatgcaggatagaaagg

SEQ ID NO: 379 - DNA, 77 bp, Artificial Sequence
  Synthetic Polynucleotide
cctacaaaaataggggactatgtgataagaccaaacctacgtttgattggtgtacctgaaagtgatggggagaatgg

SEQ ID NO: 380 - DNA, 78 bp, Artificial Sequence
  Synthetic Polynucleotide
ccattctacccatcactttcaggtacaccaatcaaacgtaggtttggccttttcatatagtctcatatttcttggagg

SEQ ID NO: 381 - DNA, 78 bp, Artificial Sequence
  Synthetic Polynucleotide
ccattctccccatcactttctggtataccaatcaaacgtaggtttggtcttttcacatagtcccatatttcttagagg

SEQ ID NO: 382 - DNA, 78 bp, Artificial Sequence; identical to SEQ ID NO: 367
  Synthetic Polynucleotide

SEQ ID NO: 383 - DNA, 78 bp, Artificial Sequence; identical to SEQ ID NO: 367
  Synthetic Polynucleotide

SEQ ID NO: 384 - DNA, 78 bp, Artificial Sequence; identical to SEQ ID NO: 367
  Synthetic Polynucleotide

SEQ ID NO: 385 - DNA, 78 bp, Artificial Sequence; identical to SEQ ID NO: 367
  Synthetic Polynucleotide

SEQ ID NO: 386 - DNA, 78 bp, Artificial Sequence; identical to SEQ ID NO: 367
  Synthetic Polynucleotide

SEQ ID NO: 387 - DNA, 78 bp, Artificial Sequence; identical to SEQ ID NO: 367
  Synthetic Polynucleotide

SEQ ID NO: 388 - DNA, 77 bp, Artificial Sequence
  Synthetic Polynucleotide
ccaccacacccagccttatgggatggttttcaaaagcatccttttttagaagtggattctgatatataatcggatgg

SEQ ID NO: 389 - DNA, 78 bp, Artificial Sequence
  Synthetic Polynucleotide
ccattctcaatgtcactttcaggtacaccaatcaaacgtaggtttggtcttttcacatagtcccatatttcttggagg

SEQ ID NO: 390 - DNA, 78 bp, Artificial Sequence
  Synthetic Polynucleotide
ccattctctctgtcactttcaggtacaccagtcaaaggtaggtttgttttattcacacgttcacatatttcttggagg

SEQ ID NO: 391 - DNA, 78 bp, Artificial Sequence
  Synthetic Polynucleotide
ccattcgccccatcactttcaggtacactagtaaaacgtaggtttggtcttttcacatagttccatatttcttggagg

SEQ ID NO: 392 - DNA, 78 bp, Artificial Sequence
  Synthetic Polynucleotide
cctccaagaaatatgggactatgtgaagagatcaaacctaggtttgattgttgtacctgaaagtgataagaagaatgg

SEQ ID NO: 393 - DNA, 78 bp, Artificial Sequence
  Synthetic Polynucleotide
cctccaataaatatggggctatgtgaaaagaccaaacctacgtttgattggtgtacctgaaagtgacagggagaatgg

SEQ ID NO: 394 - DNA, 78 bp, Artificial Sequence
  Synthetic Polynucleotide
cccttttccctgtcactttcaggtacaccagtcaaacgtaggtttggtcttttcacatagtcgaatatttcttcaagg

SEQ ID NO: 395 - DNA, 77 bp, Artificial Sequence
  Synthetic Polynucleotide
ccttttccctgtcactttcaggtacaccagtcaaacgtaggtttggtcttttcacatagtcgaatatttcttcaagg

SEQ ID NO: 396 - DNA, 78 bp, Artificial Sequence
  Synthetic Polynucleotide
ccattctccctgtcactttcaggtacactaatcaaacgtaggtttggtgtattcacacagtcccatatttcttggagg

SEQ ID NO: 397 - DNA, 78 bp, Artificial Sequence
  Synthetic Polynucleotide
ccattcttcctgtcactttcaggtataccaatcaaacgtaggtttggtcttttcacatagtcccatgtttcttggagg

SEQ ID NO: 398 - DNA, 78 bp, Artificial Sequence
  Synthetic Polynucleotide
cctccaagaaatatgagactatatgaaaataccaaacctacgtttgattggtgtacctgaaagagacagggagaatgg

SEQ ID NO: 399 - DNA, 78 bp, Artificial Sequence
  Synthetic Polynucleotide
ccattctccctatcactttcaggtacaccaatcaaacgtaggtttggtcttttcatgtagtcccatatttcttggagg

SEQ ID NO: 400 - DNA, 78 bp, Artificial Sequence
  Synthetic Polynucleotide
ccattctgcccgtcactttcaggtacaccaatcaaacgtaggtttggtcttttcacatagtcccatatttcttggagg

SEQ ID NO: 401 - DNA, 77 bp, Artificial Sequence
  Synthetic Polynucleotide
ccgtccgattatatatcagaatctacttctaaaaaaggatgcttttgaaaaccatcccataaggctgggtgtggtgg

SEQ ID NO: 402 - DNA, 78 bp, Artificial Sequence
  Synthetic Polynucleotide
cctacaaggaatataggactatgtgaaaataccaaacctacgtttcactgctgtacctgaaggtgacagggagaatgg

SEQ ID NO: 403 - DNA, 78 bp, Artificial Sequence
  Synthetic Polynucleotide
ccattctccccatcatttccaggtaaaccaatcaaaggtaggtttggtcatttcacatagtcccatatttcttggagg

SEQ ID NO: 404 - DNA, 78 bp, Artificial Sequence
  Synthetic Polynucleotide
ccattctccccgtcactttcaggtacaccagtcaaacgtaggtttggtcttttcacacagtcccatatttcctggagg

SEQ ID NO: 405 - DNA, 78 bp, Artificial Sequence
  Synthetic Polynucleotide
ccattctccccatcactttcaggtacagcaatcaaacgtaggtttggtcttttcacatagtcccatatttcttggagg

SEQ ID NO: 406 - DNA, 76 bp, Artificial Sequence
  Synthetic Polynucleotide
ccactacagattcttgggtcaagatgtgtgcaaaaggatgctttagggtgatggatatgagtgggatgaaatgagg

SEQ ID NO: 407 - DNA, 77 bp, Artificial Sequence
  Synthetic Polynucleotide
cctgaaaaaaaaccctgccagccagcaactctgaaaggatgctttgtgtgagtgagcagtgtctgagatggacaggg

SEQ ID NO: 408 - DNA, 78 bp, Artificial Sequence
  Synthetic Polynucleotide
ccattctccccatcactttcaggtacgccaatcaaacgtaggtttggtcttttgacatagtcccatatttcttggagg

SEQ ID NO: 409 - DNA, 78 bp, Artificial Sequence
  Synthetic Polynucleotide
ccgttctccccatcacttttaggtacaccaatcaaacgtaggtttggtcttttcacatagtctcatatttcttggagg

SEQ ID NO: 410 - DNA, 78 bp, Artificial Sequence
  Synthetic Polynucleotide
ccattctcctggtcactttcaggtataccaatcaaacgtaggtttggtcttttcatgtagtcccatatttcttggagg

SEQ ID NO: 411 - DNA, 78 bp, Artificial Sequence
  Synthetic Polynucleotide
cctccaagaaatatgggactacatgaaaagaccaaacctacgtttgattggtatacctgaaagtgaccaggagaatgg

SEQ ID NO: 412 - DNA, 78 bp, Artificial Sequence
  Synthetic Polynucleotide
cctccaagaactatgggactatgtgaaaagaccaaacctacgtttgattggtgtacctgaaagtgacggggagaatgg

SEQ ID NO: 413 - DNA, 78 bp, Artificial Sequence
  Synthetic Polynucleotide
ccattctccccgtcactttcaggtacaccaatcaaacgtaggtttggtcttttcacatagtcccatagttcttggagg

SEQ ID NO: 414 - DNA, 78 bp, Artificial Sequence
  Synthetic Polynucleotide
ccattctccccgtcactttcaggtacaccaatcaaacgtaggtttggtcttttcacagagtcccatatttcttggagg

SEQ ID NO: 415 - DNA, 78 bp, Artificial Sequence
  Synthetic Polynucleotide
ccattctccccgtcactttcatgtacaccaagcaaacgtaggtttgatctttccacatagtcccgtgtttcttggagg

SEQ ID NO: 416 - DNA, 78 bp, Artificial Sequence
  Synthetic Polynucleotide
cctccaagaaatatgggactatgtgaaaagaccaaacctacgtttgattggtgtacttgaaagtgacagggagaatgg

SEQ ID NO: 417 - DNA, 78 bp, Artificial Sequence
  Synthetic Polynucleotide
cctccaagaaatatgggactatgtgaaaagacaaaacctacgtttcactggtgtacctgaaagtgacagggaggatgg

SEQ ID NO: 418 - DNA, 77 bp, Artificial Sequence
  Synthetic Polynucleotide
cccccaccttttaaaaacatgcatacatacggaaacgttgctttctgcacgatttcattttaatggaacagaacagg

SEQ ID NO: 419 - DNA, 78 bp, Artificial Sequence
  Synthetic Polynucleotide
ccatttcccctgtcactttcaggtacaccaatcaaacgtaggtttggtcttttcacatagtatcatatttcttggagg

SEQ ID NO: 420 - DNA, 77 bp, Artificial Sequence
  Synthetic Polynucleotide
ccattctccccgtcactttcaggtacaccaatcaaacgtaggtttggtcttttcacatagtcccatatttctggagg

SEQ ID NO: 421 - DNA, 77 bp, Artificial Sequence
  Synthetic Polynucleotide
ccttttgttaaagtaatagaattctgcttcttaaaggaacctttcaggcaagatggtggttagagcacctaaatggg

SEQ ID NO: 422 - DNA, 76 bp, Artificial Sequence
  Synthetic Polynucleotide
ccttttgttaaagtaatagaattctgcttcttaaaggaacctttcaggcaagatggtggttagagcacctaaatgg

SEQ ID NO: 423 - DNA, 78 bp, Artificial Sequence; identical to SEQ ID NO: 412
  Synthetic Polynucleotide

SEQ ID NO: 424 - DNA, 78 bp, Artificial Sequence
  Synthetic Polynucleotide
ccattctccccgtcactttcaggtacaccaatcaaacgtaggtttggccttttcacatagtcccatagttcttggagg

SEQ ID NO: 425 - DNA, 77 bp, Artificial Sequence
  Synthetic Polynucleotide
cctccaagaaatatgggactggtgaaaagaccaaacctacgtttgactggtgtacctgaaagtgacggggagactgg

SEQ ID NO: 426 - DNA, 78 bp, Artificial Sequence
  Synthetic Polynucleotide
cctccaagaaacatgggaatgtgtgaaaagaccaaacctacgtttgattggcgtacctgaaagtgacggggagtatgg

SEQ ID NO: 427 - DNA, 78 bp, Artificial Sequence
  Synthetic Polynucleotide
cctccaagaaatatgggactgtgtgaaaagaccaaacctacgtttgattggtatacctgaaagtgacagagagaatgg

SEQ ID NO: 428 - DNA, 78 bp, Artificial Sequence
  Synthetic Polynucleotide
ccattctccccttcactatcaggtacaccaatcaaacgtaggtttagtcttttcacatagtcccatatttcttggagg

SEQ ID NO: 429 - DNA, 78 bp, Artificial Sequence
  Synthetic Polynucleotide
ccattctccccgtcactttcagatacaccagtcaaacgtaggtttggtcttttcacatagtcccatatttcttggagg

SEQ ID NO: 430 - DNA, 78 bp, Artificial Sequence
  Synthetic Polynucleotide
ccatcttactttgtactacactgttctttagagaaagcttccttttggagaccaaccaggactccttagaagcagagg

SEQ ID NO: 431 - DNA, 78 bp, Artificial Sequence; identical to SEQ ID NO: 430
  Synthetic Polynucleotide

SEQ ID NO: 432 - DNA, 78 bp, Artificial Sequence
  Synthetic Polynucleotide
cctctgcttctaaggagtcctggttggtctccaaaaggaagctttctctaaagaacagtgtagtacaaagtaagatgg

SEQ ID NO: 433 - DNA, 78 bp, Artificial Sequence; identical to SEQ ID NO: 432
  Synthetic Polynucleotide

SEQ ID NO: 434 - DNA, 78 bp, Artificial Sequence; identical to SEQ ID NO: 432
  Synthetic Polynucleotide

SEQ ID NO: 435 - DNA, 77 bp, Artificial Sequence
  Synthetic Polynucleotide
ccaccactgtgcctggccattttcactattcttaaaggaagctttggtttacaaaggtttgctactgtacttccagg

SEQ ID NO: 436 - DNA, 78 bp, Artificial Sequence
  Synthetic Polynucleotide
ccattctccctgtcactttcaggtacaccattcaaacgtaggtttggtcttttctcatagtcccatatttcttggagg

SEQ ID NO: 437 - DNA, 78 bp, Artificial Sequence
  Synthetic Polynucleotide
cctccaagaaattcgggactatgtgaaaagacaaaacctacgtttaattggtgtgtggtgtacctgaaagtgacaagg

SEQ ID NO: 438 - DNA, 78 bp, Artificial Sequence
  Synthetic Polynucleotide
cctccaagaaatatgggactatgtgaaaagaccaaacctacgtttgattggtgtacctgaaagtgaccagaagaatgg

SEQ ID NO: 439 - DNA, 77 bp, Artificial Sequence
  Synthetic Polynucleotide
cctccaagaaatatgggactatgtgaaaagcccaaacctacgtttgactgatgtacctaaagtgacggggagaatgg

SEQ ID NO: 440 - DNA, 76 bp, Artificial Sequence
  Synthetic Polynucleotide
cccgcactgtgagcttggccgagtgctgtctgaaagcatcctttcccttcacctggagactggagcgccatagagg

SEQ ID NO: 441 - DNA, 78 bp, Artificial Sequence
  Synthetic Polynucleotide
cctgtctcccccattccatgcaaaataaaacacaaaccaagctttgctttaagtgctccctgatgcagttcagcgtgg

SEQ ID NO: 442 - DNA, 78 bp, Artificial Sequence
  Synthetic Polynucleotide
ccattcttcccgtcacattcaggtacaccaatcaaacgtaggtttggtcttttcccatagtcccatatttcttagagg

SEQ ID NO: 443 - DNA, 77 bp, Artificial Sequence
  Synthetic Polynucleotide
ccccctgctcagcttggggaagaaaaatacaaaaacgatgcttttaggcattttaaacaacttcactacattgaggg

SEQ ID NO: 444 - DNA, 76 bp, Artificial Sequence
  Synthetic Polynucleotide
ccccctgctcagcttggggaagaaaaatacaaaaacgatgcttttaggcattttaaacaacttcactacattgagg

SEQ ID NO: 445 - DNA, 78 bp, Artificial Sequence
  Synthetic Polynucleotide
cctttgtgttgtgtgtattcaactcacagagtgaaaccttcctttattcagagcagttttgaaacactctttttgtgg

SEQ ID NO: 446 - DNA, 78 bp, Artificial Sequence
  Synthetic Polynucleotide
cctttgtgttgtgtgtattcaactcacagagtgaaaccttcctttattcagagcagttttgaaaaacactttttgtgg

SEQ ID NO: 447 - DNA, 78 bp, Artificial Sequence
  Synthetic Polynucleotide
cctttgtgttgtgtgtattcaactcacagagtgaaaccttcctttattcagagcagttttgaaaaactctttttgtgg

SEQ ID NO: 448 - DNA, 78 bp, Artificial Sequence; identical to SEQ ID NO: 445
  Synthetic Polynucleotide

SEQ ID NO: 449 - DNA, 78 bp, Artificial Sequence
  Synthetic Polynucleotide
cctttgtgttgtgtgtattcaactcacagagtgaaaccttcctttattcagagcagttttgaaatactctttttgtgg

SEQ ID NO: 450 - DNA, 78 bp, Artificial Sequence; identical to SEQ ID NO: 445
  Synthetic Polynucleotide

SEQ ID NO: 451 - DNA, 78 bp, Artificial Sequence
  Synthetic Polynucleotide
ccattctccctgtcactttcaagtacaccaatcaaacctaggtttggtcttttcacatagttccatatttcttggagg

SEQ ID NO: 452 - DNA, 78 bp, Artificial Sequence; identical to SEQ ID NO: 176
  Synthetic Polynucleotide

SEQ ID NO: 453 - DNA, 77 bp, Artificial Sequence
  Synthetic Polynucleotide
cccctcccatcacaggccctgaggtttaagagaaaaccatggttttgtgggccaggcccatgacccttctcctctgg

SEQ ID NO: 454 - DNA, 77 bp, Artificial Sequence
  Synthetic Polynucleotide
ccctcccatcacaggccctgaggtttaagagaaaaccatggttttgtgggccaggcccatgacccttctcctctggg

SEQ ID NO: 455 - DNA, 76 bp, Artificial Sequence
  Synthetic Polynucleotide
ccctcccatcacaggccctgaggtttaagagaaaaccatggttttgtgggccaggcccatgacccttctcctctgg

SEQ ID NO: 456 - DNA, 78 bp, Artificial Sequence
  Synthetic Polynucleotide
ccattctccccatcactttcaggtacaccaatcaaacgtaggtttcatcttttcacatagtcccacggtttttggagg

SEQ ID NO: 457 - DNA, 78 bp, Artificial Sequence
  Synthetic Polynucleotide
cctccaagatatatgggactatgtgaaaagaccaaacctacgtttgattggtgtacctgaaattgatggggagaatgg

SEQ ID NO: 458 - DNA, 78 bp, Artificial Sequence
  Synthetic Polynucleotide
cctccaagaaatatgggactgtgtgaaaagaacaaacctacgtttgattggtgtacgtgaaagtgatggggagaatgg

SEQ ID NO: 459 - DNA, 78 bp, Artificial Sequence
  Synthetic Polynucleotide
ccattcctcccgtcactttcagatacaccaaaaaaacgtaggtttggtctcttcacatagtcccacatttcttggagg

SEQ ID NO: 460 - DNA, 78 bp, Artificial Sequence
  Synthetic Polynucleotide
cctccaagaaatgtgggactatgtgaagagaccaaacctacgtttttttggtgtatctgaaagtgacgggaggaatgg

SEQ ID NO: 461 - DNA, 77 bp, Artificial Sequence
  Synthetic Polynucleotide
cctccaaggggaatctgagttctctgaagacaaaaagcatggtttcttttcttctgtatttcttattgtttcctagg

SEQ ID NO: 462 - DNA, 78 bp, Artificial Sequence
  Synthetic Polynucleotide
ccattctccctatcactttccagtacaccaatcaaacgtaggtttggtcttttcacatagtcccatatttcttggagg

SEQ ID NO: 463 - DNA, 78 bp, Artificial Sequence
  Synthetic Polynucleotide
cctccaagaaatatgggactatgtgaaaagaccaaacctacgtttgattggtatacttgaaattgacaaggagaatgg

SEQ ID NO: 464 - DNA, 78 bp, Artificial Sequence
  Synthetic Polynucleotide
cctccaagaaatatgggactatgtggaaagaccaaacctacgtttgactggtgtacctgaaagtgatggggagaatgg

SEQ ID NO: 465 - DNA, 78 bp, Artificial Sequence
  Synthetic Polynucleotide
cctctaagaaatatgggactatgtgaagagatgaaacctacgtttgattggtgtacctgaaagtgacgaggagaatgg

SEQ ID NO: 466 - DNA, 77 bp, Artificial Sequence
  Synthetic Polynucleotide
ccctcgtatactacatgctatagtcaaagcagtaaaccttcctttccttaagcagaccacactctttcatgcctggg

SEQ ID NO: 467 - DNA, 76 bp, Artificial Sequence
  Synthetic Polynucleotide
cctcgtatactacatgctatagtcaaagcagtaaaccttcctttccttaagcagaccacactctttcatgcctggg

SEQ ID NO: 468 - DNA, 78 bp, Artificial Sequence
  Synthetic Polynucleotide
ccattctccccatcactttcaggtatactaatcaaaggtaggtttggtcttttcacatagtcccatatttcatggagg

SEQ ID NO: 469 - DNA, 77 bp, Artificial Sequence
  Synthetic Polynucleotide
ccattcccccgtcactttcaggtacaccaatcaaacgtaggtttggtcttttcacatagtcccatatttcttggagg

SEQ ID NO: 470 - DNA, 78 bp, Artificial Sequence
  Synthetic Polynucleotide
ccattctccccgtcactttcaggtacaccaatcaaacgtaggttttgtcttttcttatagtcccatatttcttggagg

SEQ ID NO: 471 - DNA, 78 bp, Artificial Sequence
  Synthetic Polynucleotide
ccactgcacctgaccaagatccttaatttttctaaacctacgtttatcatctataaaatgagccatcttttcacatgg

SEQ ID NO: 472 - DNA, 78 bp, Artificial Sequence
  Synthetic Polynucleotide
cctccgagaaatatgggactatgtgaaaagaccaaacctacgtttgattgttgtacctgaaagtgacagggagaatgg

SEQ ID NO: 473 - DNA, 78 bp, Artificial Sequence
  Synthetic Polynucleotide
ccattctccccatcacttttaggtacaccaatcaaacgtaggtttggtccttttgcatagacccatatttcttggagg

SEQ ID NO: 474 - DNA, 78 bp, Artificial Sequence
  Synthetic Polynucleotide
ccattttccccgtcagtttcatatacacctatcaaacgtaggtttactgttttcacatagtcccttatttcttggagg

SEQ ID NO: 475 - DNA, 78 bp, Artificial Sequence
  Synthetic Polynucleotide
cctccaagaaatatgggactatgtgaaaagaccaaacctacctttgattggtgtacctgaaagtgacgggcaggatgg

SEQ ID NO: 476 - DNA, 78 bp, Artificial Sequence
  Synthetic Polynucleotide
ccattcttctcgtcattttcaagtacaccaatcaaacgtaggtttggtcttttcgcatagtcccatatttcttggagg

SEQ ID NO: 477 - DNA, 78 bp, Artificial Sequence
  Synthetic Polynucleotide
ccattcttctcgtcactttcaagtacaccaatcaaacgtaggtttggtcttttcacatagtcccatatttcttggagg

SEQ ID NO: 478 - DNA, 78 bp, Artificial Sequence
  Synthetic Polynucleotide
cctccaagaaatataggactatgtgaaaagaccaaacctacgtttgattggtgtacttgaaagtgacagggagaatgg

SEQ ID NO: 479 - DNA, 78 bp, Artificial Sequence
  Synthetic Polynucleotide
cctccaagaaatgtggaactatgtgaaaagaccaaacctacgtttgattggtgtacctgaaagtgacagggagaatgg

SEQ ID NO: 480 - DNA, 76 bp, Artificial Sequence
  Synthetic Polynucleotide
ccctgacactgataaacggatatgaagagaaaaaagctaggttttcgctggaattcctaagcttgggctgcagtgg

SEQ ID NO: 481 - DNA, 78 bp, Artificial Sequence
  Synthetic Polynucleotide
cccttctcccagtcacttttaggtacaccaatgaaacgtaggtttggtcttttcacacagtcccatatttcttggagg

SEQ ID NO: 482 - DNA, 77 bp, Artificial Sequence
  Synthetic Polynucleotide
ccttctcccagtcacttttaggtacaccaatgaaacgtaggtttggtcttttcacacagtcccatatttcttggagg

SEQ ID NO: 483 - DNA, 76 bp, Artificial Sequence; identical to SEQ ID NO: 180
  Synthetic Polynucleotide

SEQ ID NO: 484 - DNA, 78 bp, Artificial Sequence
  Synthetic Polynucleotide
ccaaacccgcatcgcacaccctgtgagggggacaaaggaacctttccgttccaacatcaaggttgttttgacccaagg

SEQ ID NO: 485 - DNA, 78 bp, Artificial Sequence
  Synthetic Polynucleotide
ccattctttctgtcactttcaggtataccagtcaaacctaggtttggtcttttcacatagtcccatatttcttggagg

SEQ ID NO: 486 - DNA, 78 bp, Artificial Sequence; identical to SEQ ID NO: 367
  Synthetic Polynucleotide

SEQ ID NO: 487 - DNA, 77 bp, Artificial Sequence
  Synthetic Polynucleotide
ccacacggtagaggataaactaggtggattctcaaagcaacctttgaaataatctatgcagtttttctgggtactgg

SEQ ID NO: 488 - DNA, 78 bp, Artificial Sequence
  Synthetic Polynucleotide
ccaccaagaaacatgggactatgtgaaaagaccaaacctacgtttggttggtgtacctggaagtgacggggagagtgg

SEQ ID NO: 489 - DNA, 78 bp, Artificial Sequence
  Synthetic Polynucleotide
cctccaagaaatatgggaccatgtgaaaagaccaaacctacgtttgattggtgtacctgaaagtgacagggagaatgg

SEQ ID NO: 490 - DNA, 77 bp, Artificial Sequence
  Synthetic Polynucleotide
cctgtaaaaaggtcacatggtcaggtgtgcctaaacgatccttttatttatttatttatttatttttaagaaacagg

SEQ ID NO: 491 - DNA, 77 bp, Artificial Sequence
  Synthetic Polynucleotide
ccagccccaaaatgtcaggggcttagaacaacaaaggttccttttcatgtttatactacatgtttgtcatgggctgg

SEQ ID NO: 492 - DNA, 78 bp, Artificial Sequence
  Synthetic Polynucleotide
ccgttttccccatcactttcaggtacaccagtcaaacgtaggtttggtcttttcacatggtcccacatttcttggagg

SEQ ID NO: 493 - DNA, 78 bp, Artificial Sequence
  Synthetic Polynucleotide
cctggaatagctttcctgactgtctgacttcaaaaaccttggtttgaccacttcgtctatatcatgaggaaggactgg

SEQ ID NO: 494 - DNA, 77 bp, Artificial Sequence
  Synthetic Polynucleotide
ccctactctgaacctaccttgataaagcctagaaaaccaagctttgacaagatttgacaagagatggaatttggagg

SEQ ID NO: 495 - DNA, 76 bp, Artificial Sequence
  Synthetic Polynucleotide
cctactctgaacctaccttgataaagcctagaaaaccaagctttgacaagatttgacaagagatggaatttggagg

SEQ ID NO: 496 - DNA, 77 bp, Artificial Sequence
  Synthetic Polynucleotide
cccttataaaactgaaaactttaaccttttttaaagcatgcttttgaataaattcttttattacaaaaaagaccagg

SEQ ID NO: 497 - DNA, 78 bp, Artificial Sequence
  Synthetic Polynucleotide
ccattctccctgtcactttcaggtacaccaatcaaacgtaggtttggtcttttcacgtagtcccatatttcttggagg

SEQ ID NO: 498 - DNA, 77 bp, Artificial Sequence
  Synthetic Polynucleotide
ccctttattatccaagtggtttcctgctcttcaaaccttcctttcaaaattttgtctcctacttaaaacaagttagg

SEQ ID NO: 499 - DNA, 77 bp, Artificial Sequence
  Synthetic Polynucleotide
ccttctgttgagacctactgctaagaaaacaaaaaaggttcctttcaaatattattgtgaatcaataatgtacctgg

SEQ ID NO: 500 - DNA, 78 bp, Artificial Sequence
  Synthetic Polynucleotide
cctccaagaaatatgggactatgtgaaaagaccaaacctacgtttcattgatggacctgaaagtgatggggagaatgg

SEQ ID NO: 501 - DNA, 77 bp, Artificial Sequence
  Synthetic Polynucleotide
ccattctcccttcactttcagttacaccaatcaaacgtaggtttggtcttttcacatagtcccatatttcttggagg

SEQ ID NO: 502 - DNA, 77 bp, Artificial Sequence; identical to SEQ ID NO: 181
  Synthetic Polynucleotide

SEQ ID NO: 503 - DNA, 77 bp, Artificial Sequence; identical to SEQ ID NO: 501
  Synthetic Polynucleotide

SEQ ID NO: 504 - DNA, 78 bp, Artificial Sequence
  Synthetic Polynucleotide
cctccaagaaatatgggactatgtgaaaagactaaacctacgtttgattggtgtacctgaaagtgacagggagaatgg

SEQ ID NO: 505 - DNA, 78 bp, Artificial Sequence
  Synthetic Polynucleotide
ccattctccctgtcactttcaggtatgccagtcaaacgtaggtttggtcttttcacatagtcccatattccttggagg

SEQ ID NO: 506 - DNA, 78 bp, Artificial Sequence
  Synthetic Polynucleotide
cctccaagaaatatgggactatgtaaaaagacgaaacctacgtttgattggtgtacttaaaagtgacgaggagaatgg

SEQ ID NO: 507 - DNA, 78 bp, Artificial Sequence
  Synthetic Polynucleotide
cctccaagaaatatgggactatgtgaaaagaccaaacctacgtttgatttgtgtacctgaaagtgatggggagaatgg

SEQ ID NO: 508 - DNA, 78 bp, Artificial Sequence
  Synthetic Polynucleotide
ccattctccccgtcactttcaggcacaccaatcaaacgtaggtttagtcttttcacatagtcccatatttcttagagg

SEQ ID NO: 509 - DNA, 77 bp, Artificial Sequence
  Synthetic Polynucleotide
ccttaatgcattcatatttcatattttaaataaaaccatggtttcccacagagtgacttctactctaagaaatgggg

SEQ ID NO: 510 - DNA, 76 bp, Artificial Sequence
  Synthetic Polynucleotide
ccttaatgcattcatatttcatattttaaataaaaccatggtttcccacagagtgacttctactctaagaaatggg

SEQ ID NO: 511 - DNA, 78 bp, Artificial Sequence
  Synthetic Polynucleotide
ccgttctttccgtcactttcaggtacaccagtcaaacgtaggtttggtcttttcacatagtcccatatttcttggagg

SEQ ID NO: 512 - DNA, 77 bp, Artificial Sequence
  Synthetic Polynucleotide
ccattctccccatcactttcatgtacaccaatcaaacgtaggtttggtctttgttaacatagtcccatatttcttgg

SEQ ID NO: 513 - DNA, 77 bp, Artificial Sequence
  Synthetic Polynucleotide
ccctataaagcttagagaaacacagggctctttaaacgatcctttttctcttttctgttttaaatttcatcacttgg

SEQ ID NO: 514 - DNA, 76 bp, Artificial Sequence
  Synthetic Polynucleotide
cctataaagcttagagaaacacagggctctttaaacgatcctttttctcttttctgttttaaatttcatcacttgg

SEQ ID NO: 515 - DNA, 78 bp, Artificial Sequence
  Synthetic Polynucleotide
ccattctccccatcactttcaggtacactaatcaaaggtaggtttggtcttttcacatggtcctatatttcttggagg

SEQ ID NO: 516 - DNA, 78 bp, Artificial Sequence
  Synthetic Polynucleotide
ccccatagcacgatcacatgggacattcaggggaaagcaaccttttccaggaaggaaaacccaatgctgggacccagg

SEQ ID NO: 517 - DNA, 77 bp, Artificial Sequence
  Synthetic Polynucleotide
cccatagcacgatcacatgggacattcaggggaaagcaaccttttccaggaaggaaaacccaatgctgggacccagg

SEQ ID NO: 518 - DNA, 77 bp, Artificial Sequence
  Synthetic Polynucleotide
ccctttcagcgctcacaggctatggttttataaaaggaacctttgattttgttcatgtgaaactacaaaatgccagg

SEQ ID NO: 519 - DNA, 78 bp, Artificial Sequence; identical to SEQ ID NO: 516
  Synthetic Polynucleotide

SEQ ID NO: 520 - DNA, 77 bp, Artificial Sequence; identical to SEQ ID NO: 517
  Synthetic Polynucleotide

SEQ ID NO: 521 - DNA, 78 bp, Artificial Sequence
  Synthetic Polynucleotide
cctccaagaaatattggagtatgtgataagaccaaaccttcgtttgactggtgtacctgaaagtgatggggagaatgg

SEQ ID NO: 522 - DNA, 78 bp, Artificial Sequence
  Synthetic Polynucleotide
ccattctccccgtcactttcaggtacaccaatcaaacgtaggtttggtcttttcacatagtcccatatttcttggagg

SEQ ID NO: 523 - DNA, 78 bp, Artificial Sequence; identical to SEQ ID NO: 522
  Synthetic Polynucleotide

SEQ ID NO: 524 - DNA, 78 bp, Artificial Sequence
  Synthetic Polynucleotide
ccattctccccatcactttcaggtacaccagtcaaacgaaggtttggtcttatcacatactccaatatttcttggagg

SEQ ID NO: 525 - DNA, 78 bp, Artificial Sequence
  Synthetic Polynucleotide
cctccaagatatatgggactatgtgaaaaggccaaacctacctttgattgatacacctgaaaatgacagggagaatgg

SEQ ID NO: 526 - DNA, 78 bp, Artificial Sequence
  Synthetic Polynucleotide
cctccaagaaatatgcgactatgtgaaaagaccaaacctacgtttcattggtgtacctgaaagtgatggggagaatgg

SEQ ID NO: 527 - DNA, 77 bp, Artificial Sequence
  Synthetic Polynucleotide
cctccaagaaatatgggactatgtggaaagaccaaacctacgtttgtttggtgtacctgaaagtgaggggagaatgg

SEQ ID NO: 528 - DNA, 78 bp, Artificial Sequence
  Synthetic Polynucleotide
ccattctcctcatcactttcaagtacaccaatcaaacgtaggtttggtcttttcacatagtcttatatttcttggagg

SEQ ID NO: 529 - DNA, 78 bp, Artificial Sequence; identical to SEQ ID NO: 522
  Synthetic Polynucleotide

SEQ ID NO: 530 - DNA, 78 bp, Artificial Sequence; identical to SEQ ID NO: 524
  Synthetic Polynucleotide

SEQ ID NO: 531 - DNA, 78 bp, Artificial Sequence; identical to SEQ ID NO: 522
  Synthetic Polynucleotide

SEQ ID NO: 532 - DNA, 78 bp, Artificial Sequence
  Synthetic Polynucleotide
ccagcagaagaatctggggcacagtctgtgaaaaaaggtacctttcttaagcagggttcttatccttcatgggtctgg

SEQ ID NO: 533 - DNA, 78 bp, Artificial Sequence
  Synthetic Polynucleotide
cctccaagaaatatgggactatgtgaaaagaccaaacctacgtttgattgttgtacctgaaagtgagggggagaatgg

SEQ ID NO: 534 - DNA, 77 bp, Artificial Sequence
  Synthetic Polynucleotide
ccttgtgttgtgtgtattcaactcacagagttaaacgatcctttacacagagcagatttgaaacactgtttttctgg

SEQ ID NO: 535 - DNA, 77 bp, Artificial Sequence; identical to SEQ ID NO: 534
  Synthetic Polynucleotide

SEQ ID NO: 536 - DNA, 77 bp, Artificial Sequence; identical to SEQ ID NO: 534
  Synthetic Polynucleotide

SEQ ID NO: 537 - DNA, 77 bp, Artificial Sequence
  Synthetic Polynucleotide
ccttgtgttgtgtgtattcaactcacagagttaaacgatcctttacacacagcagatttgaaacactgtttttctgg

SEQ ID NO: 538 - DNA, 77 bp, Artificial Sequence; identical to SEQ ID NO: 534
  Synthetic Polynucleotide

SEQ ID NO: 539 - DNA, 77 bp, Artificial Sequence; identical to SEQ ID NO: 534
  Synthetic Polynucleotide

SEQ ID NO: 540 - DNA, 77 bp, Artificial Sequence; identical to SEQ ID NO: 534
  Synthetic Polynucleotide

SEQ ID NO: 541 - DNA, 77 bp, Artificial Sequence; identical to SEQ ID NO: 534
  Synthetic Polynucleotide

SEQ ID NO: 542 - DNA, 77 bp, Artificial Sequence; identical to SEQ ID NO: 534
  Synthetic Polynucleotide

SEQ ID NO: 543 - DNA, 77 bp, Artificial Sequence; identical to SEQ ID NO: 534
  Synthetic Polynucleotide

SEQ ID NO: 544 - DNA, 77 bp, Artificial Sequence; identical to SEQ ID NO: 534
  Synthetic Polynucleotide

SEQ ID NO: 545 - DNA, 77 bp, Artificial Sequence; identical to SEQ ID NO: 534
  Synthetic Polynucleotide

SEQ ID NO: 546 - DNA, 77 bp, Artificial Sequence; identical to SEQ ID NO: 534
  Synthetic Polynucleotide

SEQ ID NO: 547 - DNA, 77 bp, Artificial Sequence; identical to SEQ ID NO: 537
  Synthetic Polynucleotide

SEQ ID NO: 548 - DNA, 77 bp, Artificial Sequence; identical to SEQ ID NO: 534
  Synthetic Polynucleotide

SEQ ID NO: 549 - DNA, 77 bp, Artificial Sequence; identical to SEQ ID NO: 534
  Synthetic Polynucleotide

SEQ ID NO: 550 - DNA, 77 bp, Artificial Sequence; identical to SEQ ID NO: 534
  Synthetic Polynucleotide

SEQ ID NO: 551 - DNA, 77 bp, Artificial Sequence
  Synthetic Polynucleotide
ccttgtgttgtgtgtattcaactcaccgagttaaacgatcctttacacagagcagatttgaaacactgtttttctgg

SEQ ID NO: 552 - DNA, 77 bp, Artificial Sequence; identical to SEQ ID NO: 534
  Synthetic Polynucleotide

SEQ ID NO: 553 - DNA, 77 bp, Artificial Sequence; identical to SEQ ID NO: 534
  Synthetic Polynucleotide

SEQ ID NO: 554 - DNA, 77 bp, Artificial Sequence; identical to SEQ ID NO: 534
  Synthetic Polynucleotide

SEQ ID NO: 555 - DNA, 77 bp, Artificial Sequence; identical to SEQ ID NO: 534
  Synthetic Polynucleotide

SEQ ID NO: 556 - DNA, 77 bp, Artificial Sequence; identical to SEQ ID NO: 534
  Synthetic Polynucleotide

SEQ ID NO: 557 - DNA, 77 bp, Artificial Sequence; identical to SEQ ID NO: 534
  Synthetic Polynucleotide

SEQ ID NO: 558 - DNA, 77 bp, Artificial Sequence; identical to SEQ ID NO: 534
  Synthetic Polynucleotide

SEQ ID NO: 559 - DNA, 77 bp, Artificial Sequence; identical to SEQ ID NO: 537
  Synthetic Polynucleotide

SEQ ID NO: 560 - DNA, 77 bp, Artificial Sequence; identical to SEQ ID NO: 534
  Synthetic Polynucleotide

SEQ ID NO: 561 - DNA, 77 bp, Artificial Sequence; identical to SEQ ID NO: 534
  Synthetic Polynucleotide

SEQ ID NO: 562 - DNA, 77 bp, Artificial Sequence; identical to SEQ ID NO: 534
  Synthetic Polynucleotide

SEQ ID NO: 563 - DNA, 77 bp, Artificial Sequence; identical to SEQ ID NO: 534
  Synthetic Polynucleotide

SEQ ID NO: 564 - DNA, 77 bp, Artificial Sequence; identical to SEQ ID NO: 534
  Synthetic Polynucleotide

SEQ ID NO: 565 - DNA, 77 bp, Artificial Sequence; identical to SEQ ID NO: 534
  Synthetic Polynucleotide

SEQ ID NO: 566 - DNA, 77 bp, Artificial Sequence
  Synthetic Polynucleotide
ccttgtgttgtgtgtattcaactcacagagttaaacgatcctttacacagagcagatttgtaacactgtttttctgg

SEQ ID NO: 567 - DNA, 77 bp, Artificial Sequence; identical to SEQ ID NO: 534
  Synthetic Polynucleotide

SEQ ID NO: 568 - DNA, 77 bp, Artificial Sequence; identical to SEQ ID NO: 534
  Synthetic Polynucleotide

SEQ ID NO: 569 - DNA, 77 bp, Artificial Sequence; identical to SEQ ID NO: 534
  Synthetic Polynucleotide

SEQ ID NO: 570 - DNA, 77 bp, Artificial Sequence; identical to SEQ ID NO: 534
  Synthetic Polynucleotide

SEQ ID NO: 571 - DNA, 77 bp, Artificial Sequence; identical to SEQ ID NO: 534
  Synthetic Polynucleotide

SEQ ID NO: 572 - DNA, 77 bp, Artificial Sequence; identical to SEQ ID NO: 534
  Synthetic Polynucleotide

SEQ ID NO: 573 - DNA, 77 bp, Artificial Sequence; identical to SEQ ID NO: 534
  Synthetic Polynucleotide

SEQ ID NO: 574 - DNA, 77 bp, Artificial Sequence; identical to SEQ ID NO: 534
  Synthetic Polynucleotide

SEQ ID NO: 575 - DNA, 77 bp, Artificial Sequence
  Synthetic Polynucleotide
ccttgtgttgtgtgtattcaactcacagagttaaacgatcctttacacagagcagatttgaaacactgtttttgtgg

SEQ ID NO: 576 - DNA, 77 bp, Artificial Sequence; identical to SEQ ID NO: 534
  Synthetic Polynucleotide

SEQ ID NO: 577 - DNA, 77 bp, Artificial Sequence; identical to SEQ ID NO: 534
  Synthetic Polynucleotide

SEQ ID NO: 578 - DNA, 77 bp, Artificial Sequence; identical to SEQ ID NO: 534
  Synthetic Polynucleotide

SEQ ID NO: 579 - DNA, 77 bp, Artificial Sequence; identical to SEQ ID NO: 534
  Synthetic Polynucleotide

SEQ ID NO: 580 - DNA, 77 bp, Artificial Sequence; identical to SEQ ID NO: 534
  Synthetic Polynucleotide

SEQ ID NO: 581 - DNA, 77 bp, Artificial Sequence
  Synthetic Polynucleotide
ccttgtgttgtgtgtattcaactcacagagttaaacgatcctttccacagagcagatttgaaacactgtttttctgg

SEQ ID NO: 582 - DNA, 77 bp, Artificial Sequence; identical to SEQ ID NO: 534
  Synthetic Polynucleotide

SEQ ID NO: 583 - DNA, 77 bp, Artificial Sequence; identical to SEQ ID NO: 534
  Synthetic Polynucleotide

SEQ ID NO: 584 - DNA, 77 bp, Artificial Sequence; identical to SEQ ID NO: 534
  Synthetic Polynucleotide

SEQ ID NO: 585 - DNA, 77 bp, Artificial Sequence; identical to SEQ ID NO: 534
  Synthetic Polynucleotide

SEQ ID NO: 586 - DNA, 77 bp, Artificial Sequence; identical to SEQ ID NO: 534
  Synthetic Polynucleotide

SEQ ID NO: 587 - DNA, 77 bp, Artificial Sequence; identical to SEQ ID NO: 534
  Synthetic Polynucleotide

SEQ ID NO: 588 - DNA, 77 bp, Artificial Sequence; identical to SEQ ID NO: 534
  Synthetic Polynucleotide

SEQ ID NO: 589 - DNA, 77 bp, Artificial Sequence; identical to SEQ ID NO: 534
  Synthetic Polynucleotide

SEQ ID NO: 590 - DNA, 77 bp, Artificial Sequence; identical to SEQ ID NO: 534
  Synthetic Polynucleotide

SEQ ID NO: 591 - DNA, 77 bp, Artificial Sequence; identical to SEQ ID NO: 534
  Synthetic Polynucleotide

SEQ ID NO: 592 - DNA, 77 bp, Artificial Sequence; identical to SEQ ID NO: 551
  Synthetic Polynucleotide

SEQ ID NO: 593 - DNA, 77 bp, Artificial Sequence; identical to SEQ ID NO: 534
  Synthetic Polynucleotide

SEQ ID NO: 594 - DNA, 77 bp, Artificial Sequence; identical to SEQ ID NO: 534
  Synthetic Polynucleotide

SEQ ID NO: 595 - DNA, 77 bp, Artificial Sequence; identical to SEQ ID NO: 534
  Synthetic Polynucleotide

SEQ ID NO: 596 - DNA, 77 bp, Artificial Sequence; identical to SEQ ID NO: 534
  Synthetic Polynucleotide

SEQ ID NO: 597 - DNA, 77 bp, Artificial Sequence; identical to SEQ ID NO: 534
  Synthetic Polynucleotide

SEQ ID NO: 598 - DNA, 77 bp, Artificial Sequence
  Synthetic Polynucleotide
ccttgtgttgtgtgtattcaactcacagagttaaacgatcctttacacagagcagatttgaaaaactgtttttctgg

SEQ ID NO: 599 - DNA, 77 bp, Artificial Sequence
  Synthetic Polynucleotide
ccttgtgttgtgtgtattcaactcacagagtaaaacgatcctttacacagagcagatttgaaacactgtttttctgg

SEQ ID NO: 600 - DNA, 77 bp, Artificial Sequence; identical to SEQ ID NO: 575
  Synthetic Polynucleotide

SEQ ID NO: 601 - DNA, 77 bp, Artificial Sequence; identical to SEQ ID NO: 534
  Synthetic Polynucleotide

SEQ ID NO: 602 - DNA, 77 bp, Artificial Sequence
  Synthetic Polynucleotide
ccttgtgttgtgtgtatttaactcacagagttaaacgatcctttacacagagcagatttgaaacactgtttttctgg

SEQ ID NO: 603 - DNA, 77 bp, Artificial Sequence; identical to SEQ ID NO: 534
  Synthetic Polynucleotide

SEQ ID NO: 604 - DNA, 77 bp, Artificial Sequence; identical to SEQ ID NO: 534
  Synthetic Polynucleotide

SEQ ID NO: 605 - DNA, 77 bp, Artificial Sequence; identical to SEQ ID NO: 534
  Synthetic Polynucleotide

SEQ ID NO: 606 - DNA, 77 bp, Artificial Sequence; identical to SEQ ID NO: 534
  Synthetic Polynucleotide

SEQ ID NO: 607 - DNA, 77 bp, Artificial Sequence; identical to SEQ ID NO: 534
  Synthetic Polynucleotide

SEQ ID NO: 608 - DNA, 77 bp, Artificial Sequence; identical to SEQ ID NO: 534
  Synthetic Polynucleotide

SEQ ID NO: 609 - DNA, 77 bp, Artificial Sequence; identical to SEQ ID NO: 534
  Synthetic Polynucleotide

SEQ ID NO: 610 - DNA, 77 bp, Artificial Sequence; identical to SEQ ID NO: 534
  Synthetic Polynucleotide

SEQ ID NO: 611 - DNA, 77 bp, Artificial Sequence; identical to SEQ ID NO: 534
  Synthetic Polynucleotide

SEQ ID NO: 612 - DNA, 77 bp, Artificial Sequence; identical to SEQ ID NO: 534
  Synthetic Polynucleotide

SEQ ID NO: 613 - DNA, 77 bp, Artificial Sequence; identical to SEQ ID NO: 534
  Synthetic Polynucleotide

SEQ ID NO: 614 - DNA, 78 bp, Artificial Sequence
  Synthetic Polynucleotide
ccattctccctatcactttcaggtacaccaatcaaacgtaggtttggtcttttcacatagtcccatatttcttggagg

SEQ ID NO: 615 - DNA, 77 bp, Artificial Sequence
  Synthetic Polynucleotide
cctcgtcactgccagattttgtggctaccagcaaaggatcgttttaagctgcaactcaggaaattgagaaaatatgg

SEQ ID NO: 616 - DNA, 78 bp, Artificial Sequence
  Synthetic Polynucleotide
cctccaagaaatatgggactatgtgaaaaaaccaaacctacgtttgattggtgtacctgaaagtgacagggagaatgg

SEQ ID NO: 617 - DNA, 77 bp, Artificial Sequence
  Synthetic Polynucleotide
ccctgtgttcttttatactaaaacaagccagcaaaccaacctttgagatgtgttgccttaaacattactgaatgggg

SEQ ID NO: 618 - DNA, 76 bp, Artificial Sequence
  Synthetic Polynucleotide
ccctgtgttcttttatactaaaacaagccagcaaaccaacctttgagatgtgttgccttaaacattactgaatggg

SEQ ID NO: 619 - DNA, 77 bp, Artificial Sequence
  Synthetic Polynucleotide
ccgagaaacggctttagcaacaaataaatatcaaaaggatgctttctcttcagaataatctaaagtaagttgggagg

SEQ ID NO: 620 - DNA, 78 bp, Artificial Sequence
  Synthetic Polynucleotide
ccatgttactccggataaggacagcaaaggaggaaaggaaccttttctgggccaccagaaggatgagcttgggcttgg

SEQ ID NO: 621 - DNA, 78 bp, Artificial Sequence
  Synthetic Polynucleotide
cccagggatatgctggccacggggaggagccggaaaccaacctttgtgtcactgtgtagtgacaagtgcctttggagg

SEQ ID NO: 622 - DNA, 77 bp, Artificial Sequence
  Synthetic Polynucleotide
ccagggatatgctggccacggggaggagccggaaaccaacctttgtgtcactgtgtagtgacaagtgcctttggagg

SEQ ID NO: 623 - DNA, 78 bp, Artificial Sequence
  Synthetic Polynucleotide
ccttagggacccataatggccacaaccaggagaaaagcaagctttgatgcttaaacactacttacagacatgtacagg

SEQ ID NO: 624 - DNA, 78 bp, Artificial Sequence
  Synthetic Polynucleotide
cctgcctctgttcctccttcctgatggtggcggaaaggatgcttttgccagatcaacagtcacacacaacacaccagg

SEQ ID NO: 625 - DNA, 78 bp, Artificial Sequence
  Synthetic Polynucleotide
cctgactccagccctccttgacaaggtctccgtaaagcatgctttctcttagggaccctcagagggaggcttggtggg

SEQ ID NO: 626 - DNA, 77 bp, Artificial Sequence
  Synthetic Polynucleotide
cctgactccagccctccttgacaaggtctccgtaaagcatgctttctcttagggaccctcagagggaggcttggtgg

SEQ ID NO: 627 - DNA, 77 bp, Artificial Sequence
  Synthetic Polynucleotide
ccttatttggaatgtgacaagacccatttgtttaaaccttggtttttatgcagaaagaaaaggaaggctgcagtggg

SEQ ID NO: 628 - DNA, 78 bp, Artificial Sequence
  Synthetic Polynucleotide
ccattctccctgtcactttcaggtacactaatcaaacgtaggtttgctgtttttacataggctcatatttcttggagg

SEQ ID NO: 629 - DNA, 78 bp, Artificial Sequence
  Synthetic Polynucleotide
ccattctccccatcactttcaggtacaccagtcaaacgtaggtttggtcttttcacatagtcccatatttcttggagg

SEQ ID NO: 630 - DNA, 76 bp, Artificial Sequence
  Synthetic Polynucleotide
cctgtttgttattttagctaatgtcaaaaagaaaaccttgctttttctgaaccctttcagaggcagaaagtggggg

SEQ ID NO: 631 - DNA, 77 bp, Artificial Sequence
  Synthetic Polynucleotide
ccattttccccaccactttcacgtacagcaatcaaacgtaggtttggtcttttcactagtcccatatttcttggagg

SEQ ID NO: 632 - DNA, 77 bp, Artificial Sequence; identical to SEQ ID NO: 215
  Synthetic Polynucleotide

SEQ ID NO: 633 - DNA, 77 bp, Artificial Sequence; identical to SEQ ID NO: 216
  Synthetic Polynucleotide

SEQ ID NO: 634 - DNA, 77 bp, Artificial Sequence; identical to SEQ ID NO: 217
  Synthetic Polynucleotide

SEQ ID NO: 635 - DNA, 77 bp, Artificial Sequence; identical to SEQ ID NO: 218
  Synthetic Polynucleotide

SEQ ID NO: 636 - DNA, 77 bp, Artificial Sequence; identical to SEQ ID NO: 216
  Synthetic Polynucleotide

SEQ ID NO: 637 - DNA, 77 bp, Artificial Sequence; identical to SEQ ID NO: 220
  Synthetic Polynucleotide

SEQ ID NO: 638 - DNA, 77 bp, Artificial Sequence; identical to SEQ ID NO: 177
  Synthetic Polynucleotide

SEQ ID NO: 639 - DNA, 77 bp, Artificial Sequence; identical to SEQ ID NO: 222
  Synthetic Polynucleotide

SEQ ID NO: 640 - DNA, 77 bp, Artificial Sequence; identical to SEQ ID NO: 223
  Synthetic Polynucleotide

SEQ ID NO: 641 - DNA, 77 bp, Artificial Sequence; identical to SEQ ID NO: 217
  Synthetic Polynucleotide

SEQ ID NO: 642 - DNA, 77 bp, Artificial Sequence; identical to SEQ ID NO: 225
  Synthetic Polynucleotide

SEQ ID NO: 643 - DNA, 78 bp, Artificial Sequence
  Synthetic Polynucleotide
ccaggaaaaaatttaaactttcttaacttgataaaaggtagctttcaaaacctacaataaataacatacttagagtgg

SEQ ID NO: 644 - DNA, 78 bp, Artificial Sequence
  Synthetic Polynucleotide
ccattctcctcgtcactttcaggtacaccaaacaaacgtaggtttggtctttttacgtagtcccatatttcttggagg

SEQ ID NO: 645 - DNA, 78 bp, Artificial Sequence
  Synthetic Polynucleotide
ccctcttgaagttagggaagtagcatttaagggaaacgtagctttactattaagaatttcaaacagcacttgtcaggg

SEQ ID NO: 646 - DNA, 77 bp, Artificial Sequence
  Synthetic Polynucleotide
ccctcttgaagttagggaagtagcatttaagggaaacgtagctttactattaagaatttcaaacagcacttgtcagg

SEQ ID NO: 647 - DNA, 77 bp, Artificial Sequence
  Synthetic Polynucleotide
cctcttgaagttagggaagtagcatttaagggaaacgtagctttactattaagaatttcaaacagcacttgtcaggg

SEQ ID NO: 648 - DNA, 76 bp, Artificial Sequence
  Synthetic Polynucleotide
cctcttgaagttagggaagtagcatttaagggaaacgtagctttactattaagaatttcaaacagcacttgtcagg

SEQ ID NO: 649 - DNA, 78 bp, Artificial Sequence
  Synthetic Polynucleotide
ccattctccccgtcactttcaggtacaccaatcaaacgtaggtttggtcttttcacatattcccatatttcttggagg

SEQ ID NO: 650 - DNA, 77 bp, Artificial Sequence
  Synthetic Polynucleotide
ccattctcccttcactttcaggtacaccaatcaaacgtaggtttggtcttttcacatagtcccatattttttggagg

SEQ ID NO: 651 - DNA, 78 bp, Artificial Sequence
  Synthetic Polynucleotide
cctatagtctcagttacttgggaggctgaggtaaaaggatcgtttgagcccaggaggtggaggttgcagtgagccggg

SEQ ID NO: 652 - DNA, 77 bp, Artificial Sequence
  Synthetic Polynucleotide
cctatagtctcagttacttgggaggctgaggtaaaaggatcgtttgagcccaggaggtggaggttgcagtgagccgg

SEQ ID NO: 653 - DNA, 77 bp, Artificial Sequence
  Synthetic Polynucleotide
cctttcccaactctgctattgcccccacatcctaaaggaacctttctttttttatatattttattttaagttccagg

SEQ ID NO: 654 - DNA, 78 bp, Artificial Sequence
  Synthetic Polynucleotide
cctccaagaaatatggaactatgtgaaaagaccaaacctacgtttgattgacgtacctgaaagtgacagggagaatgg

SEQ ID NO: 655 - DNA, 76 bp, Artificial Sequence
  Synthetic Polynucleotide
cctcttctgaaagcattgataatcaacattttaaacgtagcttttccccatattgctaggaaggctcattcccggg

SEQ ID NO: 656 - DNA, 78 bp, Artificial Sequence
  Synthetic Polynucleotide
cctccaagaaatatgggactatgtgaaaaggccaaacctacgtttgattgctgtacccgagagtgacggggagaatgg

SEQ ID NO: 657 - DNA, 78 bp, Artificial Sequence; identical to SEQ ID NO: 333
  Synthetic Polynucleotide

SEQ ID NO: 658 - DNA, 77 bp, Artificial Sequence
  Synthetic Polynucleotide
cccggggcctgggtgcccagtgccagtggtcagaaaggttgctttggtgtttttcattgttagtgagacagagatgg

SEQ ID NO: 659 - DNA, 76 bp, Artificial Sequence
  Synthetic Polynucleotide
ccggggcctgggtgcccagtgccagtggtcagaaaggttgctttggtgtttttcattgttagtgagacagagatgg

SEQ ID NO: 660 - DNA, 78 bp, Artificial Sequence
  Synthetic Polynucleotide
ccattctccccatcattttcaggtacaccaatcaaacgtaggtttgatcttttcacatagccccatatttcttggagg

SEQ ID NO: 661 - DNA, 77 bp, Artificial Sequence
  Synthetic Polynucleotide
ccaccagcacttctgttagaagttgcagcagagaaaggatcctttaggcacatctcccagatccttgcgaagagggg

SEQ ID NO: 662 - DNA, 78 bp, Artificial Sequence
  Synthetic Polynucleotide
cctgtgccagggtccttccactgggactggcagaaacgtaggtttgcatggagtgagaagcaggggagaggttgaggg

SEQ ID NO: 663 - DNA, 77 bp, Artificial Sequence
  Synthetic Polynucleotide
cctgtgccagggtccttccactgggactggcagaaacgtaggtttgcatggagtgagaagcaggggagaggttgagg

SEQ ID NO: 664 - DNA, 78 bp, Artificial Sequence
  Synthetic Polynucleotide
ccctcagcctctcccctgcttctcactccatgcaaacctacgtttctgccagtcccagcagaaggaccctggcacggg

SEQ ID NO: 665 - DNA, 77 bp, Artificial Sequence
  Synthetic Polynucleotide
ccctcagcctctcccctgcttctcactccatgcaaacctacgtttctgccagtcccagcagaaggaccctggcacgg

SEQ ID NO: 666 - DNA, 77 bp, Artificial Sequence
  Synthetic Polynucleotide
cctcagcctctcccctgcttctcactccatgcaaacctacgtttctgccagtcccagcagaaggaccctggcacggg

SEQ ID NO: 667 - DNA, 76 bp, Artificial Sequence
  Synthetic Polynucleotide
cctcagcctctcccctgcttctcactccatgcaaacctacgtttctgccagtcccagcagaaggaccctggcacgg

SEQ ID NO: 668 - DNA, 78 bp, Artificial Sequence
  Synthetic Polynucleotide
cctccaagaaatatggggctatgtgaaaagaccaaacctacctttgattggtgtatctgaaagtgacggggagaatgg

SEQ ID NO: 669 - DNA, 78 bp, Artificial Sequence; identical to SEQ ID NO: 507
  Synthetic Polynucleotide

SEQ ID NO: 670 - DNA, 78 bp, Artificial Sequence
  Synthetic Polynucleotide
ccattctccccgtcactttcaggtacaccaatcaaacgtaggtttggtcttttctcattgtcccatatttcttggagg

SEQ ID NO: 671 - DNA, 76 bp, Artificial Sequence
  Synthetic Polynucleotide
cccatcaagagcggttgtgcatggcaacagtaaaaggatggtttgttacactagtacaaaaagaggtggccagagg

SEQ ID NO: 672 - DNA, 78 bp, Artificial Sequence; identical to SEQ ID NO: 291
  Synthetic Polynucleotide

SEQ ID NO: 673 - DNA, 78 bp, Artificial Sequence
  Synthetic Polynucleotide
cctccaagaaatacgggactatgtgaaaagaccaaacgtacgtttgattggtgtacctgaaagtgatagggagaatgg

SEQ ID NO: 674 - DNA, 78 bp, Artificial Sequence
  Synthetic Polynucleotide
cctccaagaaatatgggactatgtgaaaagaccaaacctacgtttgattggtgtacctgaaagtgactgggagaatgg

SEQ ID NO: 675 - DNA, 78 bp, Artificial Sequence
  Synthetic Polynucleotide
ccattctccctgtcactttcaggtacacgaatcaaacgtaggtttcatcttttcacatagtcccatatttcttagagg

SEQ ID NO: 676 - DNA, 77 bp, Artificial Sequence
  Synthetic Polynucleotide
ccattctctctgtcactttctggtacaccaatcaaacgtaggtttggtcttttcacatagtttcacatatttcttgg

SEQ ID NO: 677 - DNA, 78 bp, Artificial Sequence
  Synthetic Polynucleotide
cctccaagaaatatgggactatgtgaaaagaccaaacctacgtttgattggtgtacctgaaagtgacaaggaaaatgg

SEQ ID NO: 678 - DNA, 78 bp, Artificial Sequence
  Synthetic Polynucleotide
cctgaaaaacattgtttccaacctggtaaatcaaaaggaaggtttaactttgttagataagtccacatatcaccaagg

SEQ ID NO: 679 - DNA, 78 bp, Artificial Sequence
  Synthetic Polynucleotide
cctccaagaaatgtgggactatgggaaaagaccaaacctacctttgtttggtgtacctgaaagtgacggggagaaagg

SEQ ID NO: 680 - DNA, 78 bp, Artificial Sequence
  Synthetic Polynucleotide
cctccaagaaatatgggactatgtgaaaagaccaaacctacgtttcattggtgtacctgaaagtgatgggtagaatgg

SEQ ID NO: 681 - DNA, 78 bp, Artificial Sequence
  Synthetic Polynucleotide
cctacaagaaatatgggactatgggaaaagaccaaacctacgtttgattggtacactggaaagtgacagggataatgg

SEQ ID NO: 682 - DNA, 78 bp, Artificial Sequence
  Synthetic Polynucleotide
ccattctccctgtcactttctggtacaccaatcaaaggtaggtttggtcttttcacatagtcccatatttcttggagg

SEQ ID NO: 683 - DNA, 78 bp, Artificial Sequence; identical to SEQ ID NO: 333
  Synthetic Polynucleotide

SEQ ID NO: 684 - DNA, 78 bp, Artificial Sequence
  Synthetic Polynucleotide
ccattctctttgtcactttcaggtataccaatcaaacgttggtttggtctttttgcatagtcccatattttgtggagg

SEQ ID NO: 685 - DNA, 78 bp, Artificial Sequence
  Synthetic Polynucleotide
cctccaagaaatatgagactatgtgaaaagaccaaacctacgtttgattagtgtacctgaaaatgatggggagaatgg

SEQ ID NO: 686 - DNA, 78 bp, Artificial Sequence
  Synthetic Polynucleotide
ccattctttctgtcactttcaggtacaccaatcaaacgtaggtttggtcttttcacatagtcccatatttcttggagg

SEQ ID NO: 687 - DNA, 78 bp, Artificial Sequence
  Synthetic Polynucleotide
ccattctccctgtcactttcaggtacaccaatcaaacgtaggtttgttcttttcacatagtcccatatttcttggagg

SEQ ID NO: 688 - DNA, 78 bp, Artificial Sequence
  Synthetic Polynucleotide
ccattatccccatcactttcaggtacaccaatcaaacgtaggtttggttttttcacatagttcaatatttctttgagg

SEQ ID NO: 689 - DNA, 78 bp, Artificial Sequence
  Synthetic Polynucleotide
cctccaagaaatatgggactatctgaaaagatcaaacctacgtttgattggtgtacctgaaagtgacagggagaatgg

SEQ ID NO: 690 - DNA, 78 bp, Artificial Sequence
  Synthetic Polynucleotide
cctttctccccatcactttcaggtacaccaatcaaacgtaggtttggtcttttcatatagtcccatatttcttggagg

SEQ ID NO: 691 - DNA, 78 bp, Artificial Sequence
  Synthetic Polynucleotide
cctccaagaaatatgggactatgtgcaaagatcaaacctacgtttgattgctgtacctgaaagtgatggggagaatgg

SEQ ID NO: 692 - DNA, 78 bp, Artificial Sequence
  Synthetic Polynucleotide
ccattctccccatcactttcaggtacaccagtcaaacgtaggtttggtcttttcacataatcccatatttcttggagg

SEQ ID NO: 693 - DNA, 77 bp, Artificial Sequence
  Synthetic Polynucleotide
cctccaagaagtatgggaccatggaaaagatcaaacctacgtttgactggtgtacctgaaagtgactgggagaatgg

SEQ ID NO: 694 - DNA, 78 bp, Artificial Sequence
  Synthetic Polynucleotide
cctccaagaaatatgggactatgtgaaaagaccaaacctacgtttgattggagtacttgaaaatgacagggataatgg

SEQ ID NO: 695 - DNA, 77 bp, Artificial Sequence
  Synthetic Polynucleotide
cctttaaagacatgctctttgtgccagaaattcaaaggttgcttttatgtccagtggggtggagggaggaagctcgg

SEQ ID NO: 696 - DNA, 78 bp, Artificial Sequence
  Synthetic Polynucleotide
ccattctccccgtcactttcagggacctcaatcaaacgtaggttttgtcttttcacatagtcccatatttcttggagg

SEQ ID NO: 697 - DNA, 78 bp, Artificial Sequence
  Synthetic Polynucleotide
cctccaagaaatataggactatgtgaaaagaccaaacctacgtttgactggtgtacctgaaagtgacagggagaatgg

SEQ ID NO: 698 - DNA, 78 bp, Artificial Sequence
  Synthetic Polynucleotide
ccattctccccatcactttcaggtacaccaatcaaaggtaggtttggtcttttcacatagtccgatatttcctgcagg

SEQ ID NO: 699 - DNA, 12 bp, Artificial Sequence
  Synthetic Polynucleotide
  misc_feature (4)..(5): s is g or c
  misc_feature (6)..(7): w is a, t or u
  misc_feature (8)..(9): s is g or c
aaasswwssttt

SEQ ID NO: 700 - DNA, 20 bp, Artificial Sequence
  Synthetic Polynucleotide
ctgtaaaccgaggttttgga

SEQ ID NO: 701 - protein, 15 aa, Artificial Sequence
  Synthetic Polypeptide
GGSGGSGGSGGSGGS

SEQ ID NO: 702 - protein, 7 aa, Artificial Sequence
  Synthetic Polypeptide
PKKKRKV

SEQ ID NO: 703 - DNA, 20 bp, Artificial Sequence
  Synthetic Polynucleotide
tccaaaacctcggtttacag

SEQ ID NO: 704 - DNA, 78 bp, Artificial Sequence; identical to SEQ ID NO: 176
  Synthetic Polynucleotide

SEQ ID NO: 705 - DNA, 78 bp, Artificial Sequence
  Synthetic Polynucleotide
cccagaggagaagggtcatgggcctggcccacaaaaccatggttttctcttaaacctcagggcctgtgatgggagggg

SEQ ID NO: 706 - DNA, 76 bp, Artificial Sequence; identical to SEQ ID NO: 480
  Synthetic Polynucleotide

SEQ ID NO: 707 - DNA, 76 bp, Artificial Sequence
  Synthetic Polynucleotide
ccactgcagcccaagcttaggaattccagcgaaaacctagcttttttctcttcatatccgtttatcagagtcaggg

SEQ ID NO: 708 - DNA, 78 bp, Artificial Sequence; identical to SEQ ID NO: 481
  Synthetic Polunucleotide

SEQ ID NO: 709 - DNA, 78 bp, Artificial Sequence
  Synthetic Polynucleotide
cctccaagaaatatgggactgtgtgaaaagaccaaacctacgtttcattggtgtacctaaaagtgactgggagaaggg

SEQ ID NO: 710 - DNA, 77 bp, Artificial Sequence
  Synthetic Polynucleotide
ccctgacactgataaacggatatgaagagaaaaaagctaggtttggtcttttcacacagtcccatatttcttggagg

SEQ ID NO: 711 - DNA, 77 bp, Artificial Sequence
  Synthetic Polynucleotide
cctccaagaaatatgggactgtgtgaaaagaccaaacctagcttttttctcttcatatccgtttatcagagtcaggg

SEQ ID NO: 712 - protein, 1367 aa, Artificial Sequence
  Synthetic Polypeptide
DKKYSIGLAIGTNSVGWAVITDEYKVPSKKFKVLGNTDRHSIKKNLIGALLFDSGETAEATRLKRTARRRYTRRKNRICYLQEIFSNEMAKVDDSFFHRLEESFLVEEDKKHERHPIFGNIVDEVAYHEKYPTIYHLRKKLVDSTDKADLRLIYLALAHMIKFRGHFLIEGDLNPDNSDVDKLFIQLVQTYNQLFEENPINASGVDAKAILSARLSKSRRLENLIAQLPGEKKNGLFGNLIALSLGLTPNFKSNFDLAEDAKLQLSKDTYDDDLDNLLAQIGDQYADLFLAAKNLSDAILLSDILRVNTEITKAPLSASMIKRYDEHHQDLTLLKALVRQQLPEKYKEIFFDQSKNGYAGYIDGGASQEEFYKFIKPILEKMDGTEELLVKLNREDLLRKQRTFDNGSIPHQIHLGELHAILRRQEDFYPFLKDNREKIEKILTFRIPYYVGPLARGNSRFAWMTRKSEETITPWNFEEVVDKGASAQSFIERMTNFDKNLPNEKVLPKHSLLYEYFTVYNELTKVKYVTEGMRKPAFLSGEQKKAIVDLLFKTNRKVTVKQLKEDYFKKIECFDSVEISGVEDRFNASLGTYHDLLKIIKDKDFLDNEENEDILEDIVLTLTLFEDREMIEERLKTYAHLFDDKVMKQLKRRRYTGWGRLSRKLINGIRDKQSGKTILDFLKSDGFANRNFMQLIHDDSLTFKEDIQKAQVSGQGDSLHEHIANLAGSPAIKKGILQTVKVVDELVKVMGRHKPENIVIEMARENQTTQKGQKNSRERMKRIEEGIKELGSQILKEHPVENTQLQNEKLYLYYLQNGRDMYVDQELDINRLSDYDVDAIVPQSFLKDDSIDNKVLTRSDKNRGKSDNVPSEEVVKKMKNYWRQLLNAKLITQRKFDNLTKAERGGLSELDKAGFIKRQLVETRQITKHVAQILDSRMNTKYDENDKLIREVKVITLKSKLVSDFRKDFQFYKVREINNYHHAHDAYLNAVVGTALIKKYPKLESEFVYGDYKVYDVRKMIAKSEQEIGKATAKYFFYSNIMNFFKTEITLANGEIRKRPLIETNGETGEIVWDKGRDFATVRKVLSMPQVNIVKKTEVQTGGFSKESILPKRNSDKLIARKKDWDPKKYGGFDSPTVAYSVLVVAKVEKGKSKKLKSVKELLGITIMERSSFEKNPIDFLEAKGYKEVKKDLIIKLPKYSLFELENGRKRMLASAGELQKGNELALPSKYVNFLYLASHYEKLKGSPEDNEQKQLFVEQHKHYLDEIIEQISEFSKRVILADANLDKVLSAYNKHRDKPIREQAENIIHLFTLTNLGAPAAFKYFDTTIDRKRYTSTKEVLDATLIHQSITGLYETRIDLSQLGGD

SEQ ID NO: 713 - protein, 142 aa, Artificial Sequence
  Synthetic Polypeptide
MLIGYVRVSTNDQNTDLQRNALVCAGCEQIFEDKLSGTRTDRPGLKRALKRLQKGDTLVVWKLDRLGRSMKHLISLVGELRERGINFRSLTDSIDTSSPMGRFFFYVMGALAEMERELIIERTMAGLAAARNKGRRFGRPPK

SEQ ID NO: 714 - protein, 1300 aa, Francisella novicida
MSIYQEFVNKYSLSKTLRFELIPQGKTLENIKARGLILDDEKRAKDYKKAKQIIDKYHQFFIEEILSSVCISEDLLQNYSDVYFKLKKSDDDNLQKDFKSAKDTIKKQISEYIKDSEKFKNLFNQNLIDAKKGQESDLILWLKQSKDNGIELFKANSDITDIDEALEIIKSFKGWTTYFKGFHENRKNVYSSNDIPTSIIYRIVDDNLPKFLENKAKYESLKDKAPEAINYEQIKKDLAEELTFDIDYKTSEVNQRVFSLDEVFEIANFNNYLNQSGITKFNTIIGGKFVNGENTKRKGINEYINLYSQQINDKTLKKYKMSVLFKQILSDTESKSFVIDKLEDDSDVVTTMQSFYEQIAAFKTVEEKSIKETLSLLFDDLKAQKLDLSKIYFKNDKSLTDLSQQVFDDYSVIGTAVLEYITQQIAPKNLDNPSKKEQELIAKKTEKAKYLSLETIKLALEEFNKHRDIDKQCRFEEILANFAAIPMIFDEIAQNKDNLAQISIKYQNQGKKDLLQASAEDDVKAIKDLLDQTNNLLHKLKIFHISQSEDKANILDKDEHFYLVFEECYFELANIVPLYNKIRNYITQKPYSDEKFKLNFENSTLANGWDKNKEPDNTAILFIKDDKYYLGVMNKKNNKIFDDKAIKENKGEGYKKIVYKLLPGANKMLPKVFFSAKSIKFYNPSEDILRIRNHSTHTKNGSPQKGYEKFEFNIEDCRKFIDFYKQSISKHPEWKDFGFRFSDTQRYNSIDEFYREVENQGYKLTFENISESYIDSVVNQGKLYLFQIYNKDFSAYSKGRPNLHTLYWKALFDERNLQDVVYKLNGEAELFYRKQSIPKKITHPAKEAIANKNKDNPKKESVFEYDLIKDKRFTEDKFFFHCPITINFKSSGANKFNDEINLLLKEKANDVHILSIDRGERHLAYYTLVDGKGNIIKQDTFNIIGNDRMKTNYHDKLAAIEKDRDSARKDWKKINNIKEMKEGYLSQVVHEIAKLVIEYNAIVVFEDLNFGFKRGRFKVEKQVYQKLEKMLIEKLNYLVFKDNEFDKTGGVLRAYQLTAPFETFKKMGKQTGIIYYVPAGFTSKICPVTGFVNQLYPKYESVSKSQEFFSKFDKICYNLDKGYFEFSFDYKNFGDKAAKGKWTIASFGSRLINFRNSDKNHNWDTREVYPTKELEKLLKDYSIEYGHGECIKAAICGESDKKFFAKLTSVLNTILQMRNSKTGTELDYLISPVADVNGNFFDSRQAPKNMPQDADANGAYHIGLKGLMLLGRIKNNQEGKKLNLVIKNEEYFEFVQNRNN

SEQ ID NO: 715 - protein, 1300 aa, Francisella novicida
MSIYQEFVNKYSLSKTLRFELIPQGKTLENIKARGLILDDEKRAKDYKKAKQIIDKYHQFFIEEILSSVCISEDLLQNYSDVYFKLKKSDDDNLQKDFKSAKDTIKKQISEYIKDSEKFKNLFNQNLIDAKKGQESDLILWLKQSKDNGIELFKANSDITDIDEALEIIKSFKGWTTYFKGFHENRKNVYSSNDIPTSIIYRIVDDNLPKFLENKAKYESLKDKAPEAINYEQIKKDLAEELTFDIDYKTSEVNQRVFSLDEVFEIANFNNYLNQSGITKFNTIIGGKFVNGENTKRKGINEYINLYSQQINDKTLKKYKMSVLFKQILSDTESKSFVIDKLEDDSDVVTTMQSFYEQIAAFKTVEEKSIKETLSLLFDDLKAQKLDLSKIYFKNDKSLTDLSQQVFDDYSVIGTAVLEYITQQIAPKNLDNPSKKEQELIAKKTEKAKYLSLETIKLALEEFNKHRDIDKQCRFEEILANFAAIPMIFDEIAQNKDNLAQISIKYQNQGKKDLLQASAEDDVKAIKDLLDQTNNLLHKLKIFHISQSEDKANILDKDEHFYLVFEECYFELANIVPLYNKIRNYITQKPYSDEKFKLNFENSTLANGWDKNKEPDNTAILFIKDDKYYLGVMNKKNNKIFDDKAIKENKGEGYKKIVYKLLPGANKMLPKVFFSAKSIKFYNPSEDILRIRNHSTHTKNGSPQKGYEKFEFNIEDCRKFIDFYKQSISKHPEWKDFGFRFSDTQRYNSIDEFYREVENQGYKLTFENISESYIDSVVNQGKLYLFQIYNKDFSAYSKGRPNLHTLYWKALFDERNLQDVVYKLNGEAELFYRKQSIPKKITHPAKEAIANKNKDNPKKESVFEYDLIKDKRFTEDKFFFHCPITINFKSSGANKFNDEINLLLKEKANDVHILSIARGERHLAYYTLVDGKGNIIKQDTFNIIGNDRMKTNYHDKLAAIEKDRDSARKDWKKINNIKEMKEGYLSQVVHEIAKLVIEYNAIVVFEDLNFGFKRGRFKVEKQVYQKLEKMLIEKLNYLVFKDNEFDKTGGVLRAYQLTAPFETFKKMGKQTGIIYYVPAGFTSKICPVTGFVNQLYPKYESVSKSQEFFSKFDKICYNLDKGYFEFSFDYKNFGDKAAKGKWTIASFGSRLINFRNSDKNHNWDTREVYPTKELEKLLKDYSIEYGHGECIKAAICGESDKKFFAKLTSVLNTILQMRNSKTGTELDYLISPVADVNGNFFDSRQAPKNMPQDADANGAYHIGLKGLMLLGRIKNNQEGKKLNLVIKNEEYFEFVQNRNN

SEQ ID NO: 716 - protein, 1300 aa, Francisella novicida
MSIYQEFVNKYSLSKTLRFELIPQGKTLENIKARGLILDDEKRAKDYKKAKQIIDKYHQFFIEEILSSVCISEDLLQNYSDVYFKLKKSDDDNLQKDFKSAKDTIKKQISEYIKDSEKFKNLFNQNLIDAKKGQESDLILWLKQSKDNGIELFKANSDITDIDEALEIIKSFKGWTTYFKGFHENRKNVYSSNDIPTSIIYRIVDDNLPKFLENKAKYESLKDKAPEAINYEQIKKDLAEELTFDIDYKTSEVNQRVFSLDEVFEIANFNNYLNQSGITKFNTIIGGKFVNGENTKRKGINEYINLYSQQINDKTLKKYKMSVLFKQILSDTESKSFVIDKLEDDSDVVTTMQSFYEQIAAFKTVEEKSIKETLSLLFDDLKAQKLDLSKIYFKNDKSLTDLSQQVFDDYSVIGTAVLEYITQQIAPKNLDNPSKKEQELIAKKTEKAKYLSLETIKLALEEFNKHRDIDKQCRFEEILANFAAIPMIFDEIAQNKDNLAQISIKYQNQGKKDLLQASAEDDVKAIKDLLDQTNNLLHKLKIFHISQSEDKANILDKDEHFYLVFEECYFELANIVPLYNKIRNYITQKPYSDEKFKLNFENSTLANGWDKNKEPDNTAILFIKDDKYYLGVMNKKNNKIFDDKAIKENKGEGYKKIVYKLLPGANKMLPKVFFSAKSIKFYNPSEDILRIRNHSTHTKNGSPQKGYEKFEFNIEDCRKFIDFYKQSISKHPEWKDFGFRFSDTQRYNSIDEFYREVENQGYKLTFENISESYIDSVVNQGKLYLFQIYNKDFSAYSKGRPNLHTLYWKALFDERNLQDVVYKLNGEAELFYRKQSIPKKITHPAKEAIANKNKDNPKKESVFEYDLIKDKRFTEDKFFFHCPITINFKSSGANKFNDEINLLLKEKANDVHILSIDRGERHLAYYTLVDGKGNIIKQDTFNIIGNDRMKTNYHDKLAAIEKDRDSARKDWKKINNIKEMKEGYLSQVVHEIAKLVIEYNAIVVFADLNFGFKRGRFKVEKQVYQKLEKMLIEKLNYLVFKDNEFDKTGGVLRAYQLTAPFETFKKMGKQTGIIYYVPAGFTSKICPVTGFVNQLYPKYESVSKSQEFFSKFDKICYNLDKGYFEFSFDYKNFGDKAAKGKWTIASFGSRLINFRNSDKNHNWDTREVYPTKELEKLLKDYSIEYGHGECIKAAICGESDKKFFAKLTSVLNTILQMRNSKTGTELDYLISPVADVNGNFFDSRQAPKNMPQDADANGAYHIGLKGLMLLGRIKNNQEGKKLNLVIKNEEYFEFVQNRNN

SEQ ID NO: 717 - protein, 1300 aa, Francisella novicida
MSIYQEFVNKYSLSKTLRFELIPQGKTLENIKARGLILDDEKRAKDYKKAKQIIDKYHQFFIEEILSSVCISEDLLQNYSDVYFKLKKSDDDNLQKDFKSAKDTIKKQISEYIKDSEKFKNLFNQNLIDAKKGQESDLILWLKQSKDNGIELFKANSDITDIDEALEIIKSFKGWTTYFKGFHENRKNVYSSNDIPTSIIYRIVDDNLPKFLENKAKYESLKDKAPEAINYEQIKKDLAEELTFDIDYKTSEVNQRVFSLDEVFEIANFNNYLNQSGITKFNTIIGGKFVNGENTKRKGINEYINLYSQQINDKTLKKYKMSVLFKQILSDTESKSFVIDKLEDDSDVVTTMQSFYEQIAAFKTVEEKSIKETLSLLFDDLKAQKLDLSKIYFKNDKSLTDLSQQVFDDYSVIGTAVLEYITQQIAPKNLDNPSKKEQELIAKKTEKAKYLSLETIKLALEEFNKHRDIDKQCRFEEILANFAAIPMIFDEIAQNKDNLAQISIKYQNQGKKDLLQASAEDDVKAIKDLLDQTNNLLHKLKIFHISQSEDKANILDKDEHFYLVFEECYFELANIVPLYNKIRNYITQKPYSDEKFKLNFENSTLANGWDKNKEPDNTAILFIKDDKYYLGVMNKKNNKIFDDKAIKENKGEGYKKIVYKLLPGANKMLPKVFFSAKSIKFYNPSEDILRIRNHSTHTKNGSPQKGYEKFEFNIEDCRKFIDFYKQSISKHPEWKDFGFRFSDTQRYNSIDEFYREVENQGYKLTFENISESYIDSVVNQGKLYLFQIYNKDFSAYSKGRPNLHTLYWKALFDERNLQDVVYKLNGEAELFYRKQSIPKKITHPAKEAIANKNKDNPKKESVFEYDLIKDKRFTEDKFFFHCPITINFKSSGANKFNDEINLLLKEKANDVHILSIDRGERHLAYYTLVDGKGNIIKQDTFNIIGNDRMKTNYHDKLAAIEKDRDSARKDWKKINNIKEMKEGYLSQVVHEIAKLVIEYNAIVVFEDLNFGFKRGRFKVEKQVYQKLEKMLIEKLNYLVFKDNEFDKTGGVLRAYQLTAPFETFKKMGKQTGIIYYVPAGFTSKICPVTGFVNQLYPKYESVSKSQEFFSKFDKICYNLDKGYFEFSFDYKNFGDKAAKGKWTIASFGSRLINFRNSDKNHNWDTREVYPTKELEKLLKDYSIEYGHGECIKAAICGESDKKFFAKLTSVLNTILQMRNSKTGTELDYLISPVADVNGNFFDSRQAPKNMPQDAAANGAYHIGLKGLMLLGRIKNNQEGKKLNLVIKNEEYFEFVQNRNN

SEQ ID NO: 718 - protein, 887 aa, Natronobacterium gregoryi
MTVIDLDSTTTADELTSGHTYDISVTLTGVYDNTDEQHPRMSLAFEQDNGERRYITLWKNTTPKDVFTYDYATGSTYIFTNIDYEVKDGYENLTATYQTTVENATAQEVGTTDEDETFAGGEPLDHHLDDALNETPDDAETESDSGHVMTSFASRDQLPEWTLHTYTLTATDGAKTDTEYARRTLAYTVRQELYTDHDAAPVATDGLMLLTPEPLGETPLDLDCGVRVEADETRTLDYTTAKDRLLARELVEEGLKRSLWDDYLVRGIDEVLSKEPVLTCDEFDLHERYDLSVEVGHSGRAYLHINFRHRFVPKLTLADIDDDNIYPGLRVKTTYRPRRGHIVWGLRDECATDSLNTLGNQSVVAYHRNNQTPINTDLLDAIEAADRRVVETRRQGHGDDAVSFPQELLAVEPNTHQIKQFASDGFHQQARSKTRLSASRCSEKAQAFAERLDPVRLNGSTVEFSSEFFTGNNEQQLRLLYENGESVLTFRDGARGAHPDETFSKGIVNPPESFEVAVVLPEQQADTCKAQWDTMADLLNQAGAPPTRSETVQYDAFSSPESISLNVAGAIDPSEVDAAFVVLPPDQEGFADLASPTETYDELKKALANMGIYSQMAYFDRFRDAKIFYTRNVALGLLAAAGGVAFTTEHAMPGDADMFIGIDVSRSYPEDGASGQINIAATATAVYKDGTILGHSSTRPQLGEKLQSTDVRDIMKNAILGYQQVTGESPTHIVIHRDGFMNEDLDPATEFLNEQGVEYDIVEIRKQPQTRLLAVSDVQYDTPVKSIAAINQNEPRATVATFGAPEYLATRDGGGLPRPIQIERVAGETDIETLTRQVYLLSQSHIQVHNSTARLPITTAYADQASTHATKGYLVQTGAFESNVGFL

SEQ ID NO: 719 - protein, 1544 aa, Artificial Sequence
  Synthetic Polypeptide
MLIGYVRVSTNDQNTDLQRNALVCAGCEQIFEDKLSGTRTDRPGLKRALKRLQKGDTLVVWKLDRLGRSMKHLISLVGELRERGINFRSLTDSIDTSSPMGRFFFYVMGALAEMERELIIERTMAGLAAARNKGRRFGRPPKGGSGGSGGSGGSGGSGGSGGSGGSDKKYSIGLAIGTNSVGWAVITDEYKVPSKKFKVLGNTDRHSIKKNLIGALLFDSGETAEATRLKRTARRRYTRRKNRICYLQEIFSNEMAKVDDSFFHRLEESFLVEEDKKHERHPIFGNIVDEVAYHEKYPTIYHLRKKLVDSTDKADLRLIYLALAHMIKFRGHFLIEGDLNPDNSDVDKLFIQLVQTYNQLFEENPINASGVDAKAILSARLSKSRRLENLIAQLPGEKKNGLFGNLIALSLGLTPNFKSNFDLAEDAKLQLSKDTYDDDLDNLLAQIGDQYADLFLAAKNLSDAILLSDILRVNTEITKAPLSASMIKRYDEHHQDLTLLKALVRQQLPEKYKEIFFDQSKNGYAGYIDGGASQEEFYKFIKPILEKMDGTEELLVKLNREDLLRKQRTFDNGSIPHQIHLGELHAILRRQEDFYPFLKDNREKIEKILTFRIPYYVGPLARGNSRFAWMTRKSEETITPWNFEEVVDKGASAQSFIERMTNFDKNLPNEKVLPKHSLLYEYFTVYNELTKVKYVTEGMRKPAFLSGEQKKAIVDLLFKTNRKVTVKQLKEDYFKKIECFDSVEISGVEDRFNASLGTYHDLLKIIKDKDFLDNEENEDILEDIVLTLTLFEDREMIEERLKTYAHLFDDKVMKQLKRRRYTGWGRLSRKLINGIRDKQSGKTILDFLKSDGFANRNFMQLIHDDSLTFKEDIQKAQVSGQGDSLHEHIANLAGSPAIKKGILQTVKVVDELVKVMGRHKPENIVIEMARENQTTQKGQKNSRERMKRIEEGIKELGSQILKEHPVENTQLQNEKLYLYYLQNGRDMYVDQELDINRLSDYDVDAIVPQSFLKDDSIDNKVLTRSDKNRGKSDNVPSEEVVKKMKNYWRQLLNAKLITQRKFDNLTKAERGGLSELDKAGFIKRQLVETRQITKHVAQILDSRMNTKYDENDKLIREVKVITLKSKLVSDFRKDFQFYKVREINNYHHAHDAYLNAVVGTALIKKYPKLESEFVYGDYKVYDVRKMIAKSEQEIGKATAKYFFYSNIMNFFKTEITLANGEIRKRPLIETNGETGEIVWDKGRDFATVRKVLSMPQVNIVKKTEVQTGGFSKESILPKRNSDKLIARKKDWDPKKYGGFDSPTVAYSVLVVAKVEKGKSKKLKSVKELLGITIMERSSFEKNPIDFLEAKGYKEVKKDLIIKLPKYSLFELENGRKRMLASAGELQKGNELALPSKYVNFLYLASHYEKLKGSPEDNEQKQLFVEQHKHYLDEIIEQISEFSKRVILADANLDKVLSAYNKHRDKPIREQAENIIHLFTLTNLGAPAAFKYFDTTIDRKRYTSTKEVLDATLIHQSITGLYETRIDLSQLGGDGGSDYKDDDDK

SEQ ID NO: 720 - protein, 1367 aa, Artificial Sequence
  Synthetic polypeptide
DKKYSIGLAIGTNSVGWAVITDEYKVPSKKFKVLGNTDRHSIKKNLIGALLFDSGETAEATRLKRTARRRYTRRKNRICYLQEIFSNEMAKVDDSFFHRLEESFLVEEDKKHERHPIFGNIVDEVAYHEKYPTIYHLRKKLVDSTDKADLRLIYLALAHMIKFRGHFLIEGDLNPDNSDVDKLFIQLVQTYNQLFEENPINASGVDAKAILSARLSKSRRLENLIAQLPGEKKNGLFGNLIALSLGLTPNFKSNFDLAEDAKLQLSKDTYDDDLDNLLAQIGDQYADLFLAAKNLSDAILLSDILRVNTEITKAPLSASMIKRYDEHHQDLTLLKALVRQQLPEKYKEIFFDQSKNGYAGYIDGGASQEEFYKFIKPILEKMDGTEELLVKLNREDLLRKQRTFDNGSIPHQIHLGELHAILRRQEDFYPFLKDNREKIEKILTFRIPYYVGPLARGNSRFAWMTRKSEETITPWNFEEVVDKGASAQSFIERMTAFDKNLPNEKVLPKHSLLYEYFTVYNELTKVKYVTEGMRKPAFLSGEQKKAIVDLLFKTNRKVTVKQLKEDYFKKIECFDSVEISGVEDRFNASLGTYHDLLKIIKDKDFLDNEENEDILEDIVLTLTLFEDREMIEERLKTYAHLFDDKVMKQLKRRRYTGWGALSRKLINGIRDKQSGKTILDFLKSDGFANRNFMALIHDDSLTFKEDIQKAQVSGQGDSLHEHIANLAGSPAIKKGILQTVKVVDELVKVMGRHKPENIVIEMARENQTTQKGQKNSRERMKRIEEGIKELGSQILKEHPVENTQLQNEKLYLYYLQNGRDMYVDQELDINRLSDYDVDHIVPQSFLKDDSIDNKVLTRSDKNRGKSDNVPSEEVVKKMKNYWRQLLNAKLITQRKFDNLTKAERGGLSELDKAGFIKRQLVETRAITKHVAQILDSRMNTKYDENDKLIREVKVITLKSKLVSDFRKDFQFYKVREINNYHHAHDAYLNAVVGTALIKKYPKLESEFVYGDYKVYDVRKMIAKSEQEIGKATAKYFFYSNIMNFFKTEITLANGEIRKRPLIETNGETGEIVWDKGRDFATVRKVLSMPQVNIVKKTEVQTGGFSKESILPKRNSDKLIARKKDWDPKKYGGFDSPTVAYSVLVVAKVEKGKSKKLKSVKELLGITIMERSSFEKNPIDFLEAKGYKEVKKDLIIKLPKYSLFELENGRKRMLASAGELQKGNELALPSKYVNFLYLASHYEKLKGSPEDNEQKQLFVEQHKHYLDEIIEQISEFSKRVILADANLDKVLSAYNKHRDKPIREQAENIIHLFTLTNLGAPAAFKYFDTTIDRKRYTSTKEVLDATLIHQSITGLYETRIDLSQLGGD

SEQ ID NO: 721 - protein, 1612 aa, Artificial Sequence
  Synthetic polypeptide
MSSETGPVAVDPTLRRRIEPHEFEVFFDPRELRKETCLLYEINWGGRHSIWRHTSQNTNKHVEVNFIEKFTTERYFCPNTRCSITWFLSWSPCGECSRAITEFLSRYPHVTLFIYIARLYHHADPRNRQGLRDLISSGVTIQIMTEQESGYCWRNFVNYSPSNEAHWPRYPHLWVRLYVLELYCIILGLPPCLNILRRKQPQLTFFTIALQSCHYQRLPPHILWATGLKSGSETPGTSESATPESDKKYSIGLAIGTNSVGWAVITDEYKVPSKKFKVLGNTDRHSIKKNLIGALLFDSGETAEATRLKRTARRRYTRRKNRICYLQEIFSNEMAKVDDSFFHRLEESFLVEEDKKHERHPIFGNIVDEVAYHEKYPTIYHLRKKLVDSTDKADLRLIYLALAHMIKFRGHFLIEGDLNPDNSDVDKLFIQLVQTYNQLFEENPINASGVDAKAILSARLSKSRRLENLIAQLPGEKKNGLFGNLIALSLGLTPNFKSNFDLAEDAKLQLSKDTYDDDLDNLLAQIGDQYADLFLAAKNLSDAILLSDILRVNTEITKAPLSASMIKRYDEHHQDLTLLKALVRQQLPEKYKEIFFDQSKNGYAGYIDGGASQEEFYKFIKPILEKMDGTEELLVKLNREDLLRKQRTFDNGSIPHQIHLGELHAILRRQEDFYPFLKDNREKIEKILTFRIPYYVGPLARGNSRFAWMTRKSEETITPWNFEEVVDKGASAQSFIERMTAFDKNLPNEKVLPKHSLLYEYFTVYNELTKVKYVTEGMRKPAFLSGEQKKAIVDLLFKTNRKVTVKQLKEDYFKKIECFDSVEISGVEDRFNASLGTYHDLLKIIKDKDFLDNEENEDILEDIVLTLTLFEDREMIEERLKTYAHLFDDKVMKQLKRRRYTGWGALSRKLINGIRDKQSGKTILDFLKSDGFANRNFMALIHDDSLTFKEDIQKAQVSGQGDSLHEHIANLAGSPAIKKGILQTVKVVDELVKVMGRHKPENIVIEMARENQTTQKGQKNSRERMKRIEEGIKELGSQILKEHPVENTQLQNEKLYLYYLQNGRDMYVDQELDINRLSDYDVDHIVPQSFLKDDSIDNKVLTRSDKNRGKSDNVPSEEVVKKMKNYWRQLLNAKLITQRKFDNLTKAERGGLSELDKAGFIKRQLVETRAITKHVAQILDSRMNTKYDENDKLIREVKVITLKSKLVSDFRKDFQFYKVREINNYHHAHDAYLNAVVGTALIKKYPKLESEFVYGDYKVYDVRKMIAKSEQEIGKATAKYFFYSNIMNFFKTEITLANGEIRKRPLIETNGETGEIVWDKGRDFATVRKVLSMPQVNIVKKTEVQTGGFSKESILPKRNSDKLIARKKDWDPKKYGGFDSPTVAYSVLVVAKVEKGKSKKLKSVKELLGITIMERSSFEKNPIDFLEAKGYKEVKKDLIIKLPKYSLFELENGRKRMLASAGELQKGNELALPSKYVNFLYLASHYEKLKGSPEDNEQKQLFVEQHKHYLDEIIEQISEFSKRVILADANLDKVLSAYNKHRDKPIREQAENIIHLFTLTNLGAPAAFKYFDTTIDRKRYTSTKEVLDATLIHQSITGLYETRIDLSQLGGD

SEQ ID NO: 722 - protein, 5 aa, Artificial Sequence
  Synthetic polypeptide
GGGGS

SEQ ID NO: 723 - protein, 5 aa, Artificial Sequence
  Synthetic polypeptide
EAAAK

SEQ ID NO: 724 - protein, 16 aa, Artificial Sequence
  Synthetic polypeptide
SGSETPGTSESATPES

SEQ ID NO: 725 - protein, 343 aa, Artificial Sequence
  Synthetic polypeptide
MSNLLTVHQNLPALPVDATSDEVRKNLMDMFRDRQAFSEHTWKMLLSVCRSWAAWCKLNNRKWFPAEPEDVRDYLLYLQARGLAVKTIQQHLGQLNMLHRRSGLPRPSDSNAVSLVMRRIRKENVDAGERAKQALAFERTDFDQVRSLMENSDRCQDIRNLAFLGIAYNTLLRIAEIARIRVKDISRTDGGRMLIHIGRTKTLVSTAGVEKALSLGVTKLVERWISVSGVADDPNNYLFCRVRKNGVAAPSATSQLSTRALEGIFEATHRLIYGAKDDSGQRYLAWSGHSARVGAARDMARAGVSIPEIMQAGGWTNVNIVMNYIRNLDSETGAMVRLLEDGD

SEQ ID NO: 726 - protein, 423 aa, Artificial Sequence
  Synthetic polypeptide
MPQFGILCKTPPKVLVRQFVERFERPSGEKIALCAAELTYLCWMITHNGTAIKRATFMSYNTIISNSLSFDIVNKSLQFKYKTQKATILEASLKKLIPAWEFTIIPYYGQKHQSDITDIVSSLQLQFESSEEADKGNSHSKKMLKALLSEGESIWEITEKILNSFEYTSRFTKTKTLYQFLFLATFINCGRFSDIKNVDPKSFKLVQNKYLGVIIQCLVTETKTSVSRHIYFFSARGRIDPLVYLDEFLRNSEPVLKRVNRTGNSSSNKQEYQLLKDNLVRSYNKALKKNAPYSIFAIKNGPKSHIGRHLMTSFLSMKGLTELTNVVGNWSDKRASAVARTTYTHQITAIPDHYFALVSRYYAYDPISKEMIALKDETNPIEEWQHIEQLKGSAEGSIRYPAWNGIISQEVLDYLSSYINRRI

SEQ ID NO: 727 - protein, 144 aa, Artificial Sequence
  Synthetic polypeptide
MRLFGYARVSTSQQSLDIQVRALKDAGVKANRIFTDKASGSSSDRKGLDLLRMKVEEGDVILVKKLDRLGRDTADMIQLIKEFDAQGVSIRFIDDGISTDGEMGKMVVTILSAVAQAERQRILERTNEGRQEAMAKGVVFGRKR

SEQ ID NO: 728 - protein, 144 aa, Artificial Sequence; identical to SEQ ID NO: 727
  Synthetic polypeptide

SEQ ID NO: 729 - protein, 144 aa, Artificial Sequence
  Synthetic polypeptide
MRLFGYARVSTSQQSLDIQVRALKDAGVKANRIFTDKASGSSSDRKGLDLLRMKVEEGDVILVKKLDRLGRDTADMIQLIKEFDAQGVSIRFIDDGISTDGYMGKMVVTILSAVAQAERQRILQRTNEGRQEAMAKGVVFGRKR

SEQ ID NO: 730 - protein, 147 aa, Artificial Sequence
  Synthetic polypeptide
MAKIGYARVSSKEQNLDRQLQALQGVSKVFSDKLSGQSVERPQLQAMLNYIREGDIVVVTELDRLGRNNKELTELMNAIQQKGATLEVLDLPSMNGIEDENLRRLINNLVIELYKYQAESERKRIKERQAQGIEIAKSKGKFKGRQH

SEQ ID NO: 731 - protein, 147 aa, Artificial Sequence
  Synthetic polypeptide
MAKIGYARVSSKEQNLDRQLQALQGVSKVFSDKLSGQSVERPQLQAMLNYIREGDIVVVTELDRLGRNNKELTELMNAIQQKGATLEVLDLPSMDGIEDENLRRLINNLVIELYKYQAESERKRIKERQAQGIEIAKSKGKFKGRQH

SEQ ID NO: 732 - protein, 150 aa, Artificial Sequence
  Synthetic polypeptide
MIIGYARVSSLDQNLERQLENLKTFGAEKIFTEKQSGKSIENRPILQKALNFVRMGDRFIVESIDRLGRNYNEVIHTVNYLKDKEVQLMITSLPMMNEVIGNPLLDKFMKDLIIQILAMVSEQERNESKRRQAQGIQVAKEKGVYKGRPL

SEQ ID NO: 733 - protein, 150 aa, Artificial Sequence
  Synthetic polypeptide
MIIGYARVSSLDQNLERQLENLKTFGAEKIFTEKQSGKSIENRPILQKALNFVRMGDRFIVESIDRLGRNYNEVIHTVNYLKDKEVRLMITSLPMMNEVIGNPLLDKFMKDLIIRILAMVSEQERNESKRRQAQGIQVAKEKGVYKGRPL

SEQ ID NO: 734 - protein, 144 aa, Artificial Sequence
  Synthetic polypeptide
MRLFGYARVSTSQQSLDLQVRALKDAGVKANRIFTDKASGSSTDREGLDLLRMKVKEGDVILVKKLDRLGRDTADMLQLIKEFDAQGVAVRFIDDGISTDGDMGQMVVTILSAVAQAERRRILERTNEGRQEAKLKGIKFGRRR

SEQ ID NO: 735 - protein, 144 aa, Artificial Sequence
  Sythetic polypeptide
MRLFGYARVSTSQQSLDLQVRALKDAGVKANRIFTDKASGSSTDREGLDLLRMKVKEGDVILVKKLDRLSRDTADMLQLIKEFDAQGVAVRFIDDGISTDGYMGQMVVTILSAVAQAERRRILQRTNEGRQEAKLKGIKFGRRR

SEQ ID NO: 736 - protein, 142 aa, Artificial Sequence
  Synthetic polypeptide
MATIGYIRVSTIDQNIDLQRNALTSANCDRIFEDRISGKIANRPGLKRALKYVNKGDTLVVWKLDRLGRSVKNLVALISELHERGAHFHSLTDSIDTSSAMGRFFFHVMSALAEMERELIVERTLAGLAAARAQGRLGGRPV

SEQ ID NO: 737 - protein, 142 aa, Artificial Sequence
  Synthetic polypeptide
MATIGYIRVSTIDQNIDLQRNALTSANCDRIFEDRISGKIANRPGLKRALKYVNKGDTLVVWKLDRLGRSVKNLVALISELHERGAHFHSLTDSIDTSSAMGRFFFYVMSALAEMERELIVERTLAGLAAARAQGRLGGRPV

SEQ ID NO: 738 - protein, 608 aa, Artificial Sequence
  Synthetic polypeptide
MDTYAGAYDRQSRERENSSAASPATQRSANEDKAADLQREVERDGGRFRFVGHFSEAPGTSAFGTAERPEFERILNECRAGRLNMIIVYDVSRFSRLKVMDAIPIVSELLALGVTIVSTQEGVFRQGNVMDLIHLIMRLDASHKESSLKSAKILDTKNLQRELGGYVGGKAPYGFELVSETKEITRNGRMVNVVINKLAHSTTPLTGPFEFEPDVIRWWWREIKTHKHLPFKPGSQAAIHPGSITGLCKRMDADAVPTRGETIGKKTASSAWDPATVMRILRDPRIAGFAAEVIYKKKPDGTPTTKIEGYRIQRDPITLRPVELDCGPIIEPAEWYELQAWLDGRGRGKGLSRGQAILSAMDKLYCECGAVMTSKRGEESIKDSYRCRRRKVVDPSAPGQHEGTCNVSMAALDKFVAERIFNKIRHAEGDEETLALLWEAARRFGKLTEAPEKSGERANLVAERADALNALEELYEDRAAGAYDGPVGRKHFRKQQAALTLRQQGAEERLAELEAAEAPKLPLDQWFPEDADADPTGPKSWWGRASVDDKRVFVGLFVDKIVVTKSTTGRGQGTPIEKRASITWAKPPTDDDEDDAQDGTEDVAATGA

SEQ ID NO: 739 - DNA, 34 bp, Artificial Sequence
  Synthetic polynucleotide
ataacttcgtatagcatacattatacgaagttat

SEQ ID NO: 740 - DNA, 34 bp, Artificial Sequence
  Synthetic polynucleotide
gaagttcctattctctagaaagtataggaacttc

SEQ ID NO: 741 - protein, 4 aa, Artificial Sequence
  Synthetic polypeptide
NGAN

SEQ ID NO: 742 - protein, 4 aa, Artificial Sequence
  Synthetic polypeptide
NGNG

SEQ ID NO: 743 - protein, 4 aa, Artificial Sequence
  Synthetic polypeptide
NGAG

SEQ ID NO: 744 - protein, 4 aa, Artificial Sequence
  Synthetic polypeptide
NGCG

SEQ ID NO: 745 - protein, 6 aa, Artificial Sequence
  Synthetic polypeptide
NNGRRT

SEQ ID NO: 746 - protein, 5 aa, Artificial Sequence
  Synthetic polypeptide
NGRRN

SEQ ID NO: 747 - protein, 6 aa, Artificial Sequence
  Synthetic polypeptide
NNNRRT

SEQ ID NO: 748 - protein, 7 aa, Artificial Sequence
  Synthetic polypeptide
NNNGATT

SEQ ID NO: 749 - protein, 7 aa, Artificial Sequence
  Synthetic polypeptide
NNAGAAW

SEQ ID NO: 750 - protein, 5 aa, Artificial Sequence
  Synthetic polypeptide
NAAAC

SEQ ID NO: 751 - protein, 4 aa, Artificial Sequence
  Synthetic polypeptide
TTTN

SEQ ID NO: 752 - protein, 1367 aa, Artificial Sequence; identical to SEQ ID NO: 712
  Synthetic Polypeptide

SEQ ID NO: 753 - protein, 1367 aa, Artificial Sequence
  Synthetic Polypeptide
DKKYSIGLAIGTNSVGWAVITDEYKVPSKKFKVLGNTDRHSIKKNLIGALLFDSGETAEATRLKRTARRRYTRRKNRICYLQEIFSNEMAKVDDSFFHRLEESFLVEEDKKHERHPIFGNIVDEVAYHEKYPTIYHLRKKLVDSTDKADLRLIYLALAHMIKFRGHFLIEGDLNPDNSDVDKLFIQLVQTYNQLFEENPINASGVDAKAILSARLSKSRRLENLIAQLPGEKKNGLFGNLIALSLGLTPNFKSNFDLAEDAKLQLSKDTYDDDLDNLLAQIGDQYADLFLAAKNLSDAILLSDILRVNTEITKAPLSASMIKRYDEHHQDLTLLKALVRQQLPEKYKEIFFDQSKNGYAGYIDGGASQEEFYKFIKPILEKMDGTEELLVKLNREDLLRKQRTFDNGSIPHQIHLGELHAILRRQEDFYPFLKDNREKIEKILTFRIPYYVGPLARGNSRFAWMTRKSEETITPWNFEEVVDKGASAQSFIERMTNFDKNLPNEKVLPKHSLLYEYFTVYNELTKVKYVTEGMRKPAFLSGEQKKAIVDLLFKTNRKVTVKQLKEDYFKKIECFDSVEISGVEDRFNASLGTYHDLLKIIKDKDFLDNEENEDILEDIVLTLTLFEDREMIEERLKTYAHLFDDKVMKQLKRRRYTGWGRLSRKLINGIRDKQSGKTILDFLKSDGFANRNFMQLIHDDSLTFKEDIQKAQVSGQGDSLHEHIANLAGSPAIKKGILQTVKVVDELVKVMGRHKPENIVIEMARENQTTQKGQKNSRERMKRIEEGIKELGSQILKEHPVENTQLQNEKLYLYYLQNGRDMYVDQELDINRLSDYDVDHIVPQSFLKDDSIDNKVLTRSDKNRGKSDNVPSEEVVKKMKNYWRQLLNAKLITQRKFDNLTKAERGGLSELDKAGFIKRQLVETRQITKHVAQILDSRMNTKYDENDKLIREVKVITLKSKLVSDFRKDFQFYKVREINNYHHAHDAYLNAVVGTALIKKYPKLESEFVYGDYKVYDVRKMIAKSEQEIGKATAKYFFYSNIMNFFKTEITLANGEIRKRPLIETNGETGEIVWDKGRDFATVRKVLSMPQVNIVKKTEVQTGGFSKESILPKRNSDKLIARKKDWDPKKYGGFDSPTVAYSVLVVAKVEKGKSKKLKSVKELLGITIMERSSFEKNPIDFLEAKGYKEVKKDLIIKLPKYSLFELENGRKRMLASAGELQKGNELALPSKYVNFLYLASHYEKLKGSPEDNEQKQLFVEQHKHYLDEIIEQISEFSKRVILADANLDKVLSAYNKHRDKPIREQAENIIHLFTLTNLGAPAAFKYFDTTIDRKRYTSTKEVLDATLIHQSITGLYETRIDLSQLGGD

SEQ ID NO: 754 - protein, 1367 aa, Artificial Sequence
  Synthetic Polypeptide
DKKYSIGLDIGTNSVGWAVITDEYKVPSKKFKVLGNTDRHSIKKNLIGALLFDSGETAEATRLKRTARRRYTRRKNRICYLQEIFSNEMAKVDDSFFHRLEESFLVEEDKKHERHPIFGNIVDEVAYHEKYPTIYHLRKKLVDSTDKADLRLIYLALAHMIKFRGHFLIEGDLNPDNSDVDKLFIQLVQTYNQLFEENPINASGVDAKAILSARLSKSRRLENLIAQLPGEKKNGLFGNLIALSLGLTPNFKSNFDLAEDAKLQLSKDTYDDDLDNLLAQIGDQYADLFLAAKNLSDAILLSDILRVNTEITKAPLSASMIKRYDEHHQDLTLLKALVRQQLPEKYKEIFFDQSKNGYAGYIDGGASQEEFYKFIKPILEKMDGTEELLVKLNREDLLRKQRTFDNGSIPHQIHLGELHAILRRQEDFYPFLKDNREKIEKILTFRIPYYVGPLARGNSRFAWMTRKSEETITPWNFEEVVDKGASAQSFIERMTNFDKNLPNEKVLPKHSLLYEYFTVYNELTKVKYVTEGMRKPAFLSGEQKKAIVDLLFKTNRKVTVKQLKEDYFKKIECFDSVEISGVEDRFNASLGTYHDLLKIIKDKDFLDNEENEDILEDIVLTLTLFEDREMIEERLKTYAHLFDDKVMKQLKRRRYTGWGRLSRKLINGIRDKQSGKTILDFLKSDGFANRNFMQLIHDDSLTFKEDIQKAQVSGQGDSLHEHIANLAGSPAIKKGILQTVKVVDELVKVMGRHKPENIVIEMARENQTTQKGQKNSRERMKRIEEGIKELGSQILKEHPVENTQLQNEKLYLYYLQNGRDMYVDQELDINRLSDYDVDHIVPQSFLKDDSIDNKVLTRSDKNRGKSDNVPSEEVVKKMKNYWRQLLNAKLITQRKFDNLTKAERGGLSELDKAGFIKRQLVETRQITKHVAQILDSRMNTKYDENDKLIREVKVITLKSKLVSDFRKDFQFYKVREINNYHHAHDAYLNAVVGTALIKKYPKLESEFVYGDYKVYDVRKMIAKSEQEIGKATAKYFFYSNIMNFFKTEITLANGEIRKRPLIETNGETGEIVWDKGRDFATVRKVLSMPQVNIVKKTEVQTGGFSKESILPKRNSDKLIARKKDWDPKKYGGFDSPTVAYSVLVVAKVEKGKSKKLKSVKELLGITIMERSSFEKNPIDFLEAKGYKEVKKDLIIKLPKYSLFELENGRKRMLASAGELQKGNELALPSKYVNFLYLASHYEKLKGSPEDNEQKQLFVEQHKHYLDEIIEQISEFSKRVILADANLDKVLSAYNKHRDKPIREQAENIIHLFTLTNLGAPAAFKYFDTTIDRKRYTSTKEVLDATLIHQSITGLYETRIDLSQLGGD

SEQ ID NO: 755 - protein, 345 aa, Sulfolobus islandicus
MEVPLYNIFGDNYIIQVATEAENSTIYNNKVEIDDEELRNVLNLAYKIAKNNEDAAAERRGKAKKKKGEEGETTTSNIILPLSGNDKNPWTETLKCYNFPTTVALSEVFKNFSQVKECEEVSAPSFVKPEFYEFGRSPGMVERTRRVKLEVEPHYLIIAAAGWVLTRLGKAKVSEGDYVGVNVFTPTRGILYSLIQNVNGIVPGIKPETAFGLWIARKVVSSVTNPNVSVVRIYTISDAVGQNPTTINGGFSIDLTKLLEKRYLLSERLEAIARNALSISSNMRERYIVLANYIYEYLTGSKRLEDLLYFANRDLIMNLNSDDGKVRDLKLISAYVNGELIRGEG

SEQ ID NO: 756 - protein, 345 aa, Sulfolobus islandicus
MEVPLYNIFGDNYIIQVATEAENSTIYNNKVEIDDEELRNVLNLAYKIAKNNEDAAAERRGKAKKKKGEEGETTTSNIILPLSGNDKNPWTETLKCYNFPTTVALSEVFKNFSQVKECEEVSAPSFVKPEFYKFGRSPGMVERTRRVKLEVEPHYLIMAAAGWVLTRLGKAKVSEGDYVGVNVFTPTRGILYSLIQNVNGIVPGIKPETAFGLWIARKVVSSVTNPNVSVVSIYTISDAVGQNPTTINGGFSIDLTKLLEKRDLLSERLEAIARNALSISSNMRERYIVLANYIYEYLTGSKRLEDLLYFANRDLIMNLNSDDGKVRDLKLISAYVNGELIRGEG

SEQ ID NO: 757 - protein, 1210 aa, Parcubacteria
MSKRHPRISGVKGYRLHAQRLEYTGKSGAMRTIKYPLYSSPSGGRTVPREIVSAINDDYVGLYGLSNFDDLYNAEKRNEEKVYSVLDFWYDCVQYGAVFSYTAPGLLKNVAEVRGGSYELTKTLKGSHLYDELQIDKVIKFLNKKEISRANGSLDKLKKDIIDCFKAEYRERHKDQCNKLADDIKNAKKDAGASLGERQKKLFRDFFGISEQSENDKPSFTNPLNLTCCLLPFDTVNNNRNRGEVLFNKLKEYAQKLDKNEGSLEMWEYIGIGNSGTAFSNFLGEGFLGRLRENKITELKKAMMDITDAWRGQEQEEELEKRLRILAALTIKLREPKFDNHWGGYRSDINGKLSSWLQNYINQTVKIKEDLKGHKKDLKKAKEMINRFGESDTKEEAVVSSLLESIEKIVPDDSADDEKPDIPAIAIYRRFLSDGRLTLNRFVQREDVQEALIKERLEAEKKKKPKKRKKKSDAEDEKETIDFKELFPHLAKPLKLVPNFYGDSKRELYKKYKNAAIYTDALWKAVEKIYKSAFSSSLKNSFFDTDFDKDFFIKRLQKIFSVYRRFNTDKWKPIVKNSFAPYCDIVSLAENEVLYKPKQSRSRKSAAIDKNRVRLPSTENIAKAGIALARELSVAGFDWKDLLKKEEHEEYIDLIELHKTALALLLAVTETQLDISALDFVENGTVKDFMKTRDGNLVLEGRFLEMFSQSIVFSELRGLAGLMSRKEFITRSAIQTMNGKQAELLYIPHEFQSAKITTPKEMSRAFLDLAPAEFATSLEPESLSEKSLLKLKQMRYYPHYFGYELTRTGQGIDGGVAENALRLEKSPVKKREIKCKQYKTLGRGQNKIVLYVRSSYYQTQFLEWFLHRPKNVQTDVAVSGSFLIDEKKVKTRWNYDALTVALEPVSGSERVFVSQPFTIFPEKSAEEEGQRYLGIDIGEYGIAYTALEITGDSAKILDQNFISDPQLKTLREEVKGLKLDQRRGTFAMPSTKIARIRESLVHSLRNRIHHLALKHKAKIVYELEVSRFEEGKQKIKKVYATLKKADVYSEIDADKNLQTTVWGKLAVASEISASYTSQFCGACKKLWRAEMQVDETITTQELIGTVRVIKGGTLIDAIKDFMRPPIFDENDTPFPKYRDFCDKHHISKKMRGNSCLFICPFCRANADADIQASQTIALLRYVKEEKKVEDYFERFRKLKNIKVLGQMKKI

SEQ ID NO: 758 - protein, 4 aa, Artificial Sequence
  Synthetic Polypeptide
SGGS

SEQ ID NO: 759 - protein, 4 aa, Artificial Sequence
  Synthetic Polypeptide
GGGS

SEQ ID NO: 760 - DNA, 91 bp, Artificial Sequence
  Synthetic Polynucleotide
cctagggaagtgatcatagctgagtttctatctcatggtttatgctaaactatatgttgacatgttgaggagacttaagtccaaaacctgg

SEQ ID NO: 761 - protein, 30 aa, Artificial Sequence
  Synthetic Polypeptide
MDSLLMNRRKFLYQFKNVRWAKGRRETYLC

SEQ ID NO: 762 - protein, 1129 aa, Alicyclobacillus acidoterrestris
MAVKSIKVKLRLDDMPEIRAGLWKLHKEVNAGVRYYTEWLSLLRQENLYRRSPNGDGEQECDKTAEECKAELLERLRARQVENGHRGPAGSDDELLQLARQLYELLVPQAIGAKGDAQQIARKFLSPLADKDAVGGLGIAKAGNKPRWVRMREAGEPGWEEEKEKAETRKSADRTADVLRALADFGLKPLMRVYTDSEMSSVEWKPLRKGQAVRTWDRDMFQQAIERMMSWESWNQRVGQEYAKLVEQKNRFEQKNFVGQEHLVHLVNQLQQDMKEASPGLESKEQTAHYVTGRALRGSDKVFEKWGKLAPDAPFDLYDAEIKNVQRRNTRRFGSHDLFAKLAEPEYQALWREDASFLTRYAVYNSILRKLNHAKMFATFTLPDATAHPIWTRFDKLGGNLHQYTFLFNEFGERRHAIRFHKLLKVENGVAREVDDVTVPISMSEQLDNLLPRDPNEPIALYFRDYGAEQHFTGEFGGAKIQCRRDQLAHMHRRRGARDVYLNVSVRVQSQSEARGERRPPYAAVFRLVGDNHRAFVHFDKLSDYLAEHPDDGKLGSEGLLSGLRVMSVDLGLRTSASISVFRVARKDELKPNSKGRVPFFFPIKGNDNLVAVHERSQLLKLPGETESKDLRAIREERQRTLRQLRTQLAYLRLLVRCGSEDVGRRERSWAKLIEQPVDAANHMTPDWREAFENELQKLKSLHGICSDKEWMDAVYESVRRVWRHMGKQVRDWRKDVRSGERPKIRGYAKDVVGGNSIEQIEYLERQYKFLKSWSFFGKVSGQVIRAEKGSRFAITLREHIDHAKEDRLKKLADRIIMEALGYVYALDERGKGKWVAKYPPCQLILLEELSEYQFNNDRPPSENNQLMQWSHRGVFQELINQAQVHDLLVGTMYAAFSSRFDARTGAPGIRCRRVPARCTQEHNPEPFPWWLNKFVVEHTLDACPLRADDLIPTGEGEIFVSPFSAEEGDFHQIHADLNAAQNLQQRLWSDFDISQIRLRCDWGEVDGELVLIPRLTGKRTADSYSNKVFYTNTGVTYYERERGKKRRKVFAQEKLSEEEAELLVEADEAREKSVVLMRDPSGIINRGNWTRQKEFWSMVNQRIEGYLVKQIRSRVPLQDSACENTGDI

SEQ ID NO: 763 - protein, 5 aa, Artificial Sequence
  Synthetic Polypeptide
NGGNG

SEQ ID NO: 764 - protein, 1389 aa, Leptotrichia shahii
MGNLFGHKRWYEVRDKKDFKIKRKVKVKRNYDGNKYILNINENNNKEKIDNNKFIRKYINYKKNDNILKEFTRKFHAGNILFKLKGKEGIIRIENNDDFLETEEVVLYIEAYGKSEKLKALGITKKKIIDEAIRQGITKDDKKIEIKRQENEEEIEIDIRDEYTNKTLNDCSIILRIIENDELETKKSIYEIFKNINMSLYKIIEKIIENETEKVFENRYYEEHLREKLLKDDKIDVILTNFMEIREKIKSNLEILGFVKFYLNVGGDKKKSKNKKMLVEKILNINVDLTVEDIADFVIKELEFWNITKRIEKVKKVNNEFLEKRRNRTYIKSYVLLDKHEKFKIERENKKDKIVKFFVENIKNNSIKEKIEKILAEFKIDELIKKLEKELKKGNCDTEIFGIFKKHYKVNFDSKKFSKKSDEEKELYKIIYRYLKGRIEKILVNEQKVRLKKMEKIEIEKILNESILSEKILKRVKQYTLEHIMYLGKLRHNDIDMTTVNTDDFSRLHAKEELDLELITFFASTNMELNKIFSRENINNDENIDFFGGDREKNYVLDKKILNSKIKIIRDLDFIDNKNNITNNFIRKFTKIGTNERNRILHAISKERDLQGTQDDYNKVINIIQNLKISDEEVSKALNLDVVFKDKKNIITKINDIKISEENNNDIKYLPSFSKVLPEILNLYRNNPKNEPFDTIETEKIVLNALIYVNKELYKKLILEDDLEENESKNIFLQELKKTLGNIDEIDENIIENYYKNAQISASKGNNKAIKKYQKKVIECYIGYLRKNYEELFDFSDFKMNIQEIKKQIKDINDNKTYERITVKTSDKTIVINDDFEYIISIFALLNSNAVINKIRNRFFATSVWLNTSEYQNIIDILDEIMQLNTLRNECITENWNLNLEEFIQKMKEIEKDFDDFKIQTKKEIFNNYYEDIKNNILTEFKDDINGCDVLEKKLEKIVIFDDETKFEIDKKSNILQDEQRKLSNINKKDLKKKVDQYIKDKDQEIKSKILCRIIFNSDFLKKYKKEIDNLIEDMESENENKFQEIYYPKERKNELYIYKKNLFLNIGNPNFDKIYGLISNDIKMADAKFLFNIDGKNIRKNKISEIDAILKNLNDKLNGYSKEYKEKYIKKLKENDDFFAKNIQNKNYKSFEKDYNRVSEYKKIRDLVEFNYLNKIESYLIDINWKLAIQMARFERDMHYIVNGLRELGIIKLSGYNTGISRAYPKRNGSDGFYTTTAYYKFFDEESYKKFEKICYGFGIDLSENSEINKPENESIRNYISHFYIVRNPFADYSIAEQIDRVSNLLSYSTRYNNSTYASVFEVFKKDVNLDYDELKKKFKLIGNNDILERLMKPKKVSVLELESYNSDYIKNLIIELLTKIENTNDTL

SEQ ID NO: 765 - DNA, 5268 bp, Artificial Sequence
  Synthetic Polynucleotide
atgtccaacctccttaccgtccaccagaatctccctgcccttccggtggatgccacctctgatgaagtgcgaaaaaacctgatggatatgtttcgcgataggcaagctttttctgaacacacgtggaagatgctcctgtcagtgtgtagaagctgggcagcttggtgcaagttgaacaaccgaaaatggtttcctgccgaacccgaagatgtgagagactacctcctctacctgcaggctcgagggctcgccgtgaaaacaatccaacaacacttgggtcagctcaacatgctgcacaggagatctgggctgccccggccgagtgactctaatgccgttagtctcgtaatgcggcgcattcgcaaagagaatgtggatgctggagaacgggcgaaacaggcactggcttttgaacggaccgacttcgatcaggtgcggagtcttatggagaatagtgacagatgccaggacattcggaaccttgcattcctgggtatcgcgtataataccctgctgagaatcgctgagatcgccagaatcagggtaaaggatatttctcgaacggacgggggacggatgttgattcatatcggtcgcactaaaacacttgtgagtaccgccggggtagagaaagccctgagccttggagttactaaactggtggagcggtggattagcgtgtccggcgtggcggatgacccaaacaattacttgttttgtagggtgcggaaaaatggtgtagccgctccatccgctacctcacagttgagtacacgcgcgttggaggggattttcgaagccacacatcgcttgatctacggcgccaaggacgattcaggccagcgatatcttgcctggagcgggcatagtgcccgggtgggtgccgcccgagacatggcaagggctggcgtgtcaattcctgaaatcatgcaggccggcgggtggaccaacgtgaacattgtgatgaactatatccggaacctggatagcgagaccggagcaatggtcagactgcttgaggatggcgacggtggatccggagggtccggaggtagtggcggcagcggtggttcaggtggcagcggagggtcaggaggctctgataaaaagtattctattggtttagctatcggcactaattccgttggatgggctgtcataaccgatgaatacaaagtaccttcaaagaaatttaaggtgttggggaacacagaccgtcattcgattaaaaagaatcttatcggtgccctcctattcgatagtggcgaaacggcagaggcgactcgcctgaaacgaaccgctcggagaaggtatacacgtcgcaagaaccgaatatgttacttacaagaaatttttagcaatgagatggccaaagttgacgattctttctttcaccgtttggaagagtccttccttgtcgaagaggacaagaaacatgaacggcaccccatctttggaaacatagtagatgaggtggcatatcatgaaaagtacccaacgatttatcacctcagaaaaaagctagttgactcaactgataaagcggacctgaggttaatctacttggctcttgcccatatgataaagttccgtgggcactttctcattgagggtgatctaaatccggacaactcggatgtcgacaaactgttcatccagttagtacaaacctataatcagttgtttgaagagaaccctataaatgcaagtggcgtggatgcgaaggctattcttagcgcccgcctctctaaatcccgacggctagaaaacctgatcgcacaattacccggagagaagaaaaatgggttgttcggtaaccttatagcgctctcactaggcctgacaccaaattttaagtcgaacttcgacttagctgaagatgccaaattgcagcttagtaaggacacgtacgatgacgatctcgacaatctactggcacaaattggagatcagtatgcggacttatttttggctgccaaaaaccttagcgatgcaatcctcctatctgacatactgagagttaatactgagattaccaaggcgccgttatccgcttcaatgatcaaaaggtacgatgaacatcaccaagacttgacacttctcaaggccctagtccgtcagcaactgcctgagaaatataaggaaatattctttgatcagtcgaaaaacgggtacgcaggttatattgacggcggagcgagtcaagaggaattctacaagtttatcaaacccatattagagaagatggatgggacggaagagttgcttgtaaaactcaatcgcgaagatctactgcgaaagcagcggactttcgacaacggtagcattccacatcaaatccacttaggcgaattgcatgctatacttagaaggcaggaggatttttatccgttcctcaaagacaatcgtgaaaagattgagaaaatcctaacctttcgcataccttactatgtgggacccctggcccgagggaactctcggttcgcatggatgacaagaaagtccgaagaaacgattactccatggaattttgaggaagttgtcgataaaggtgcgtcagctcaatcgttcatcgagaggatgaccaactttgacaagaatttaccgaacgaaaaagtattgcctaagcacagtttactttacgagtatttcacagtgtacaatgaactcacgaaagttaagtatgtcactgagggcatgcgtaaacccgcctttctaagcggagaacagaagaaagcaatagtagatctgttattcaagaccaaccgcaaagtgacagttaagcaattgaaagaggactactttaagaaaattgaatgcttcgattctgtcgagatctccggggtagaagatcgatttaatgcgtcacttggtacgtatcatgacctcctaaagataattaaagataaggacttcctggataacgaagagaatgaagatatcttagaagatatagtgttgactcttaccctctttgaagatcgggaaatgattgaggaaagactaaaaacatacgctcacctgttcgacgataaggttatgaaacagttaaagaggcgtcgctatacgggctggggacgattgtcgcggaaacttatcaacgggataagagacaagcaaagtggtaaaactattctcgattttctaaagagcgacggcttcgccaataggaactttatgcagctgatccatgatgactctttaaccttcaaagaggatatacaaaaggcacaggtttccggacaaggggactcattgcacgaacatattgcgaatcttgctggttcgccagccatcaaaaagggcatactccagacagtcaaagtagtggatgagctagttaaggtcatgggacgtcacaaaccggaaaacattgtaatcgagatggcacgcgaaaatcaaacgactcagaaggggcaaaaaaacagtcgagagcggatgaagagaatagaagagggtattaaagaactgggcagccagatcttaaaggagcatcctgtggaaaatacccaattgcagaacgagaaactttacctctattacctacaaaatggaagggacatgtatgttgatcaggaactggacataaaccgtttatctgattacgacgtcgatgccattgtaccccaatcctttttgaaggacgattcaatcgacaataaagtgcttacacgctcggataagaaccgagggaaaagtgacaatgttccaagcgaggaagtcgtaaagaaaatgaagaactattggcggcagctcctaaatgcgaaactgataacgcaaagaaagttcgataacttaactaaagctgagaggggtggcttgtctgaacttgacaaggccggatttattaaacgtcagctcgtggaaacccgccaaatcacaaagcatgttgcacagatactagattcccgaatgaatacgaaatacgacgagaacgataagctgattcgggaagtcaaagtaatcactttaaagtcaaaattggtgtcggacttcagaaaggattttcaattctataaagttagggagataaataactaccaccatgcgcacgacgcttatcttaatgccgtcgtagggaccgcactcattaagaaatacccgaagctagaaagtgagtttgtgtatggtgattacaaagtttatgacgtccgtaagatgatcgcgaaaagcgaacaggagataggcaaggctacagccaaatacttcttttattctaacattatgaatttctttaagacggaaatcactctggcaaacggagagatacgcaaacgacctttaattgaaaccaatggggagacaggtgaaatcgtatgggataagggccgggacttcgcgacggtgagaaaagttttgtccatgccccaagtcaacatagtaaagaaaactgaggtgcagaccggagggttttcaaaggaatcgattcttccaaaaaggaatagtgataagctcatcgctcgtaaaaaggactgggacccgaaaaagtacggtggcttcgatagccctacagttgcctattctgtcctagtagtggcaaaagttgagaagggaaaatccaagaaactgaagtcagtcaaagaattattggggataacgattatggagcgctcgtcttttgaaaagaaccccatcgacttccttgaggcgaaaggttacaaggaagtaaaaaaggatctcataattaaactaccaaagtatagtctgtttgagttagaaaatggccgaaaacggatgttggctagcgccggagagcttcaaaaggggaacgaactcgcactaccgtctaaatacgtgaatttcctgtatttagcgtcccattacgagaagttgaaaggttcacctgaagataacgaacagaagcaactttttgttgagcagcacaaacattatctcgacgaaatcatagagcaaatttcggaattcagtaagagagtcatcctagctgatgccaatctggacaaagtattaagcgcatacaacaagcacagggataaacccatacgtgagcaggcggaaaatattatccatttgtttactcttaccaacctcggcgctccagccgcattcaagtattttgacacaacgatagatcgcaaacgatacacttctaccaaggaggtgctagacgcgacactgattcaccaatccatcacgggattatatgaaactcggatagatttgtcacagcttgggggtgacggtggctccgattataaggatgatgacgacaagggaggttccccaaagaagaaaaggaaggtctga

SEQ ID NO: 766 - protein, 1755 aa, Artificial Sequence
  Synthetic Polypeptide
MSNLLTVHQNLPALPVDATSDEVRKNLMDMFRDRQAFSEHTWKMLLSVCRSWAAWCKLNNRKWFPAEPEDVRDYLLYLQARGLAVKTIQQHLGQLNMLHRRSGLPRPSDSNAVSLVMRRIRKENVDAGERAKQALAFERTDFDQVRSLMENSDRCQDIRNLAFLGIAYNTLLRIAEIARIRVKDISRTDGGRMLIHIGRTKTLVSTAGVEKALSLGVTKLVERWISVSGVADDPNNYLFCRVRKNGVAAPSATSQLSTRALEGIFEATHRLIYGAKDDSGQRYLAWSGHSARVGAARDMARAGVSIPEIMQAGGWTNVNIVMNYIRNLDSETGAMVRLLEDGDGGSGGSGGSGGSGGSGGSGGSGGSDKKYSIGLAIGTNSVGWAVITDEYKVPSKKFKVLGNTDRHSIKKNLIGALLFDSGETAEATRLKRTARRRYTRRKNRICYLQEIFSNEMAKVDDSFFHRLEESFLVEEDKKHERHPIFGNIVDEVAYHEKYPTIYHLRKKLVDSTDKADLRLIYLALAHMIKFRGHFLIEGDLNPDNSDVDKLFIQLVQTYNQLFEENPINASGVDAKAILSARLSKSRRLENLIAQLPGEKKNGLFGNLIALSLGLTPNFKSNFDLAEDAKLQLSKDTYDDDLDNLLAQIGDQYADLFLAAKNLSDAILLSDILRVNTEITKAPLSASMIKRYDEHHQDLTLLKALVRQQLPEKYKEIFFDQSKNGYAGYIDGGASQEEFYKFIKPILEKMDGTEELLVKLNREDLLRKQRTFDNGSIPHQIHLGELHAILRRQEDFYPFLKDNREKIEKILTFRIPYYVGPLARGNSRFAWMTRKSEETITPWNFEEVVDKGASAQSFIERMTNFDKNLPNEKVLPKHSLLYEYFTVYNELTKVKYVTEGMRKPAFLSGEQKKAIVDLLFKTNRKVTVKQLKEDYFKKIECFDSVEISGVEDRFNASLGTYHDLLKIIKDKDFLDNEENEDILEDIVLTLTLFEDREMIEERLKTYAHLFDDKVMKQLKRRRYTGWGRLSRKLINGIRDKQSGKTILDFLKSDGFANRNFMQLIHDDSLTFKEDIQKAQVSGQGDSLHEHIANLAGSPAIKKGILQTVKVVDELVKVMGRHKPENIVIEMARENQTTQKGQKNSRERMKRIEEGIKELGSQILKEHPVENTQLQNEKLYLYYLQNGRDMYVDQELDINRLSDYDVDAIVPQSFLKDDSIDNKVLTRSDKNRGKSDNVPSEEVVKKMKNYWRQLLNAKLITQRKFDNLTKAERGGLSELDKAGFIKRQLVETRQITKHVAQILDSRMNTKYDENDKLIREVKVITLKSKLVSDFRKDFQFYKVREINNYHHAHDAYLNAVVGTALIKKYPKLESEFVYGDYKVYDVRKMIAKSEQEIGKATAKYFFYSNIMNFFKTEITLANGEIRKRPLIETNGETGEIVWDKGRDFATVRKVLSMPQVNIVKKTEVQTGGFSKESILPKRNSDKLIARKKDWDPKKYGGFDSPTVAYSVLVVAKVEKGKSKKLKSVKELLGITIMERSSFEKNPIDFLEAKGYKEVKKDLIIKLPKYSLFELENGRKRMLASAGELQKGNELALPSKYVNFLYLASHYEKLKGSPEDNEQKQLFVEQHKHYLDEIIEQISEFSKRVILADANLDKVLSAYNKHRDKPIREQAENIIHLFTLTNLGAPAAFKYFDTTIDRKRYTSTKEVLDATLIHQSITGLYETRIDLSQLGGDGGSDYKDDDDKGGSPKKKRKV

SEQ ID NO: 767 - DNA, 95 bp, Artificial Sequence
  Synthetic Polynucleotide
cctgaaataatgcaagtgtagaataactttttaaaatctcatggtttatgctaaactatatgttgacataagagtggtgataaggcaacagtagg

SEQ ID NO: 768 - DNA, 91 bp, Artificial Sequence; identical to SEQ ID NO: 760
  Synthetic Polynucleotide

SEQ ID NO: 769 - DNA, 105 bp, Artificial Sequence
  Synthetic Polynucleotide
atgtcctgaaataatgcaagtgtagaataactttttaaaatctcatggtttatgctaaactatatgttgacataagagtggtgataaggcaacagtaggtaaaag

SEQ ID NO: 770 - protein, 35 aa, Artificial Sequence
  Synthetic Polypeptide
  MISC_FEATURE (3)..(3): Xaa is a stop codon
  MISC_FEATURE (10)..(10): Xaa is a stop codon
  MISC_FEATURE (25)..(25): Xaa is a stop codon
  MISC_FEATURE (28)..(29): Xaa is a stop codon
  MISC_FEATURE (34)..(34): Xaa is a stop codon
MSXNNASVEXLFKISWFMLNYMLTXEWXXGNSRXK

SEQ ID NO: 771 - protein, 4 aa, Artificial Sequence
  Synthetic Polypeptide
NAAR

SEQ ID NO: 772 - protein, 4 aa, Artificial Sequence
  Synthetic Polypeptide
AGVF

SEQ ID NO: 773 - protein, 4 aa, Artificial Sequence
  Synthetic Polypeptide
GFLG

SEQ ID NO: 774 - protein, 4 aa, Artificial Sequence
  Synthetic Polypeptide
ALAL

SEQ ID NO: 775 - protein, 5 aa, Artificial Sequence
  Synthetic Polypeptide
ALALA